European Patent Application EP 4 227 408 A1, published August 16, 2023. Title: An engineered guide RNA including a U-rich tail for the optimized CRISPR/Cas12f1 system and use thereof. Applicant: Genkore. The sequence listing filed with the application follows.

SEQUENCE LISTING (649 sequences)

SEQ ID NO: 1 - RNA, 140 nt, Artificial Sequence
  mature form of Cas12f1 tracrRNA
cuucacugauaaaguggagaaccgcuucaccaaaagcugucccuuaggggauuagaacuugagugaaggugggcugcuugcaucagccuaaugucgagaagugcuuucuucggaaaguaacccucgaaacaaauucauuu

SEQ ID NO: 2 - RNA, 161 nt, Artificial Sequence
  wild-type of Cas12f1 tracrRNA
cuucacugauaaaguggagaaccgcuucaccaaaagcugucccuuaggggauuagaacuugagugaaggugggcugcuugcaucagccuaaugucgagaagugcuuucuucggaaaguaacccucgaaacaaauucauuuuuccucuccaauucugcacaa

SEQ ID NO: 3 - RNA, 17 nt, Artificial Sequence
  mature form of Cas12f1 crRNA repeat
gaaugaaggaaugcaac

SEQ ID NO: 4 - RNA, 37 nt, Artificial Sequence
  wild-type of Cas12f1 crRNA repeat
guugcagaacccgaauagacgaaugaaggaaugcaac

SEQ ID NO: 5 - RNA, 37 nt, Artificial Sequence
  mature form of Cas12f1 crRNA
gaaugaaggaaugcaacnnnnnnnnnnnnnnnnnnnn

SEQ ID NO: 6 - RNA, 57 nt, Artificial Sequence
  wild-type of Cas12f1 crRNA
guugcagaacccgaauagacgaaugaaggaaugcaacnnnnnnnnnnnnnnnnnnnn

SEQ ID NO: 7 - RNA, 161 nt, Artificial Sequence
  mature form of Cas12f1 tracrRNA + GAAA + mature form of Cas12f1 crRNA repeat crRNA repeat
cuucacugauaaaguggagaaccgcuucaccaaaagcugucccuuaggggauuagaacuugagugaaggugggcugcuugcaucagccuaaugucgagaagugcuuucuucggaaaguaacccucgaaacaaauucauuugaaagaaugaaggaaugcaac

SEQ ID NO: 8 - RNA, 181 nt, Artificial Sequence
  mature form of Cas12f1 tracrRNA + GAAA + mature form of Cas12f1 crRNA crRNA
cuucacugauaaaguggagaaccgcuucaccaaaagcugucccuuaggggauuagaacuugagugaaggugggcugcuugcaucagccuaaugucgagaagugcuuucuucggaaaguaacccucgaaacaaauucauuugaaagaaugaaggaaugcaacnnnnnnnnnnnnnnnnnnnn

SEQ ID NO: 9 - RNA, 190 nt, Artificial Sequence
  mature form of Cas12f1 tracrRNA - GAAA - mature form of Cas12f1 crRNA - U-rich tail crRNA - U-rich tail
cuucacugauaaaguggagaaccgcuucaccaaaagcugucccuuaggggauuagaacuugagugaaggugggcugcuugcaucagccuaaugucgagaagugcuuucuucggaaaguaacccucgaaacaaauucauuugaaagaaugaaggaaugcaacnnnnnnnnnnnnnnnnnnnnuuuuauuuu

SEQ ID NO: 10 - RNA, 21 nt, Artificial Sequence
  1st region of Cas12f1 guide RNA
cuucacugauaaaguggagaa

SEQ ID NO: 11 - RNA, 50 nt, Artificial Sequence
  2nd region of Cas12f1 guide RNA
ccgcuucaccaaaagcugucccuuaggggauuagaacuugagugaaggug

SEQ ID NO: 12 - RNA, 56 nt, Artificial Sequence
  3rd region of Cas12f1 guide RNA
ggcugcuugcaucagccuaaugucgagaagugcuuucuucggaaaguaacccucga

SEQ ID NO: 13 - RNA, 13 nt, Artificial Sequence
  4th region of Cas12f1 guide RNA (Mature form)
aacaaauucauuu

SEQ ID NO: 14 - RNA, 34 nt, Artificial Sequence
  4th region of Cas12f1 guide RNA (Wild-type)
aacaaauucauuuuuccucuccaauucugcacaa

SEQ ID NO: 15 - RNA, 10 nt, Artificial Sequence
  5th region of Cas12f1 guide RNA (Mature form)
gaaugaagga

SEQ ID NO: 16 - RNA, 30 nt, Artificial Sequence
  5th region of Cas12f1 guide RNA (Wild-type)
guugcagaacccgaauagacgaaugaagga

SEQ ID NO: 17 - RNA, 10 nt, Artificial Sequence
  first region, 11nt deletion
aaguggagaa

SEQ ID NO: 18 - RNA, 11 nt, Artificial Sequence
  first region, 10nt deletion
aaaguggagaa

SEQ ID NO: 19 - RNA, 12 nt, Artificial Sequence
  first region, 9nt deletion
uaaaguggagaa

SEQ ID NO: 20 - RNA, 13 nt, Artificial Sequence
  first region, 8nt deletion
auaaaguggagaa

SEQ ID NO: 21 - RNA, 14 nt, Artificial Sequence
  first region, 7nt deletion
gauaaaguggagaa

SEQ ID NO: 22 - RNA, 15 nt, Artificial Sequence
  first region, 6nt deletion
ugauaaaguggagaa

SEQ ID NO: 23 - RNA, 16 nt, Artificial Sequence
  first region, 5nt deletion
cugauaaaguggagaa

SEQ ID NO: 24 - RNA, 17 nt, Artificial Sequence
  first region, 4nt deletion
acugauaaaguggagaa

SEQ ID NO: 25 - RNA, 18 nt, Artificial Sequence
  first region, 3nt deletion
cacugauaaaguggagaa

SEQ ID NO: 26 - RNA, 19 nt, Artificial Sequence
  first region, 2nt deletion
ucacugauaaaguggagaa

SEQ ID NO: 27 - RNA, 20 nt, Artificial Sequence
  first region, 1nt deletion
uucacugauaaaguggagaa

SEQ ID NO: 28 - RNA, 10 nt, Artificial Sequence
  deleted part of the first region, 10nt
aaaguggaga

SEQ ID NO: 29 - RNA, 11 nt, Artificial Sequence
  deleted part of the first region, 11nt
uaaaguggaga

SEQ ID NO: 30 - RNA, 12 nt, Artificial Sequence
  deleted part of the first region, 12nt
auaaaguggaga

SEQ ID NO: 31 - RNA, 13 nt, Artificial Sequence
  deleted part of the first region, 13nt
gauaaaguggaga

SEQ ID NO: 32 - RNA, 14 nt, Artificial Sequence
  deleted part of the first region, 14nt
ugauaaaguggaga

SEQ ID NO: 33 - RNA, 15 nt, Artificial Sequence
  deleted part of the first region, 15nt
cugauaaaguggaga

SEQ ID NO: 34 - RNA, 16 nt, Artificial Sequence
  deleted part of the first region, 16nt
acugauaaaguggaga

SEQ ID NO: 35 - RNA, 17 nt, Artificial Sequence
  deleted part of the first region, 17nt
cacugauaaaguggaga

SEQ ID NO: 36 - RNA, 18 nt, Artificial Sequence
  deleted part of the first region, 18nt
ucacugauaaaguggaga

SEQ ID NO: 37 - RNA, 19 nt, Artificial Sequence
  deleted part of the first region, 19nt
uucacugauaaaguggaga

SEQ ID NO: 38 - RNA, 20 nt, Artificial Sequence
  deleted part of the first region, 20nt
cuucacugauaaaguggaga

SEQ ID NO: 39 - RNA, 28 nt, Artificial Sequence
  second region, 11bp deletion
ccgcuucaccauuagugagugaaggugg

SEQ ID NO: 40 - RNA, 30 nt, Artificial Sequence
  second region, 10bp deletion
ccgcuucaccaauuaguugagugaaggugg

SEQ ID NO: 41 - RNA, 32 nt, Artificial Sequence
  second region, 9bp deletion
ccgcuucaccaaauuagcuugagugaaggugg

SEQ ID NO: 42 - RNA, 34 nt, Artificial Sequence
  second region, 8bp deletion
ccgcuucaccaaaauuagacuugagugaaggugg

SEQ ID NO: 43 - RNA, 36 nt, Artificial Sequence
  second region, 7bp deletion
ccgcuucaccaaaaguuagaacuugagugaaggugg

SEQ ID NO: 44 - RNA, 38 nt, Artificial Sequence
  second region, 6bp deletion
ccgcuucaccaaaagcuuaggaacuugagugaaggugg

SEQ ID NO: 45 - RNA, 40 nt, Artificial Sequence
  second region, 5bp deletion
ccgcuucaccaaaagcuuuagagaacuugagugaaggugg

SEQ ID NO: 46 - RNA, 43 nt, Artificial Sequence
  second region, 4bp deletion
ccgcuucaccaaaagcuguuaguuagaacuugagugaaggugg

SEQ ID NO: 47 - RNA, 42 nt, Artificial Sequence
  second region, 4bp+1nt deletion
ccgcuucaccaaaagcuguuaguagaacuugagugaaggugg

SEQ ID NO: 48 - RNA, 45 nt, Artificial Sequence
  second region, 3bp deletion
ccgcuucaccaaaagcuguuuagauuagaacuugagugaaggugg

SEQ ID NO: 49 - RNA, 47 nt, Artificial Sequence
  second region, 2bp deletion
ccgcuucaccaaaagcugucuuaggauuagaacuugagugaaggugg

SEQ ID NO: 50 - RNA, 49 nt, Artificial Sequence
  second region, 1bp deletion
ccgcuucaccaaaagcuguccuuagggauuagaacuugagugaaggugg

SEQ ID NO: 51 - RNA, 11 nt, Artificial Sequence
  second region, 5' remains
ccgcuucacca

SEQ ID NO: 52 - RNA, 13 nt, Artificial Sequence
  second region, 3' remains
ugagugaaggugg

SEQ ID NO: 53 - RNA, 10 nt, Artificial Sequence
  upper-deleted part of the second region, 10nt
aaagcugucc

SEQ ID NO: 54 - RNA, 11 nt, Artificial Sequence
  upper-deleted part of the second region, 11nt
aaagcuguccc

SEQ ID NO: 55 - RNA, 10 nt, Artificial Sequence
  lower-deleted part of the second region, 10nt
gauuagaacu

SEQ ID NO: 56 - RNA, 11 nt, Artificial Sequence
  lower-deleted part of the second region, 11nt
ggauuagaacu

SEQ ID NO: 57 - RNA, 12 nt, Artificial Sequence
  lower-deleted part of the second region, 12nt
gggauuagaacu

SEQ ID NO: 58 - RNA, 10 nt, Artificial Sequence
  intermediate sequence of the second region, 10nt
aaauuagacu

SEQ ID NO: 59 - RNA, 12 nt, Artificial Sequence
  intermediate sequence of the second region, 11nt
aaaguuagaacu

SEQ ID NO: 60 - RNA, 14 nt, Artificial Sequence
  intermediate sequence of the second region, 12nt
aaagcuuaggaacu

SEQ ID NO: 61 - RNA, 16 nt, Artificial Sequence
  intermediate sequence of the second region, 13nt
aaagcuuuagagaacu

SEQ ID NO: 62 - RNA, 18 nt, Artificial Sequence
  intermediate sequence of the second region, 14nt
aaagcuguuaguagaacu

SEQ ID NO: 63 - RNA, 19 nt, Artificial Sequence
  intermediate sequence of the second region, 15nt
aaagcuguuaguuagaacu

SEQ ID NO: 64 - RNA, 21 nt, Artificial Sequence
  intermediate sequence of the second region, 16nt
aaagcuguuuagauuagaacu

SEQ ID NO: 65 - RNA, 23 nt, Artificial Sequence
  intermediate sequence of the second region, 17nt
aaagcugucuuaggauuagaacu

SEQ ID NO: 66 - RNA, 25 nt, Artificial Sequence
  intermediate sequence of the second region, 18nt
aaagcuguccuuagggauuagaacu

SEQ ID NO: 67 - RNA, 10 nt, Artificial Sequence
  fourth region of the tracrRNA(mature form), delete 3nt
aacaaauuca

SEQ ID NO: 68 - RNA, 11 nt, Artificial Sequence
  fourth region of the tracrRNA(mature form), delete 4nt
aacaaauucau

SEQ ID NO: 69 - RNA, 12 nt, Artificial Sequence
  fourth region of the tracrRNA(mature form), delete 5nt
aacaaauucauu

SEQ ID NO: 70 - RNA, 13 nt, Artificial Sequence
  fourth region of the tracrRNA(wild-type), 21nt deletion
aacaaauucauuu

SEQ ID NO: 71 - RNA, 14 nt, Artificial Sequence
  fourth region of the tracrRNA(wild-type), 20nt deletion
aacaaauucauuuu

SEQ ID NO: 72 - RNA, 15 nt, Artificial Sequence
  fourth region of the tracrRNA(wild-type), 19nt deletion
aacaaauucauuuuu

SEQ ID NO: 73 - RNA, 16 nt, Artificial Sequence
  fourth region of the tracrRNA(wild-type), 18nt deletion
aacaaauucauuuuuc

SEQ ID NO: 74 - RNA, 17 nt, Artificial Sequence
  fourth region of the tracrRNA(wild-type), 17nt deletion
aacaaauucauuuuucc

SEQ ID NO: 75 - RNA, 18 nt, Artificial Sequence
  fourth region of the tracrRNA(wild-type), 16nt deletion
aacaaauucauuuuuccu

SEQ ID NO: 76 - RNA, 19 nt, Artificial Sequence
  fourth region of the tracrRNA(wild-type), 15nt deletion
aacaaauucauuuuuccuc

SEQ ID NO: 77 - RNA, 20 nt, Artificial Sequence
  fourth region of the tracrRNA(wild-type), 14nt deletion
aacaaauucauuuuuccucu

SEQ ID NO: 78 - RNA, 21 nt, Artificial Sequence
  fourth region of the tracrRNA(wild-type), 13nt deletion
aacaaauucauuuuuccucuc

SEQ ID NO: 79 - RNA, 22 nt, Artificial Sequence
  fourth region of the tracrRNA(wild-type), 12nt deletion
aacaaauucauuuuuccucucc

SEQ ID NO: 80 - RNA, 23 nt, Artificial Sequence
  fourth region of the tracrRNA(wild-type), 11nt deletion
aacaaauucauuuuuccucucca

SEQ ID NO: 81 - RNA, 24 nt, Artificial Sequence
  fourth region of the tracrRNA(wild-type), 10nt deletion
aacaaauucauuuuuccucuccaa

SEQ ID NO: 82 - RNA, 25 nt, Artificial Sequence
  fourth region of the tracrRNA(wild-type), 9nt deletion
aacaaauucauuuuuccucuccaau

SEQ ID NO: 83 - RNA, 26 nt, Artificial Sequence
  fourth region of the tracrRNA(wild-type), 8nt deletion
aacaaauucauuuuuccucuccaauu

SEQ ID NO: 84 - RNA, 27 nt, Artificial Sequence
  fourth region of the tracrRNA(wild-type), 7nt deletion
aacaaauucauuuuuccucuccaauuc

SEQ ID NO: 85 - RNA, 28 nt, Artificial Sequence
  fourth region of the tracrRNA(wild-type), 6nt deletion
aacaaauucauuuuuccucuccaauucu

SEQ ID NO: 86 - RNA, 29 nt, Artificial Sequence
  fourth region of the tracrRNA(wild-type), 5nt deletion
aacaaauucauuuuuccucuccaauucug

SEQ ID NO: 87 - RNA, 30 nt, Artificial Sequence
  fourth region of the tracrRNA(wild-type), 4nt deletion
aacaaauucauuuuuccucuccaauucugc

SEQ ID NO: 88 - RNA, 31 nt, Artificial Sequence
  fourth region of the tracrRNA(wild-type), 3nt deletion
aacaaauucauuuuuccucuccaauucugca

SEQ ID NO: 89 - RNA, 32 nt, Artificial Sequence
  fourth region of the tracrRNA(wild-type), 2nt deletion
aacaaauucauuuuuccucuccaauucugcac

SEQ ID NO: 90 - RNA, 33 nt, Artificial Sequence
  fourth region of the tracrRNA(wild-type), 1nt deletion
aacaaauucauuuuuccucuccaauucugcaca

SEQ ID NO: 91 - RNA, 10 nt, Artificial Sequence
  fifth region of the crRNA(wild-type), 20nt deletion
gaaugaagga

SEQ ID NO: 92 - RNA, 11 nt, Artificial Sequence
  fifth region of the crRNA(wild-type), 19nt deletion
cgaaugaagga

SEQ ID NO: 93 - RNA, 12 nt, Artificial Sequence
  fifth region of the crRNA(wild-type), 18nt deletion
acgaaugaagga

SEQ ID NO: 94 - RNA, 13 nt, Artificial Sequence
  fifth region of the crRNA(wild-type), 17nt deletion
gacgaaugaagga

SEQ ID NO: 95 - RNA, 14 nt, Artificial Sequence
  fifth region of the crRNA(wild-type), 16nt deletion
agacgaaugaagga

SEQ ID NO: 96 - RNA, 15 nt, Artificial Sequence
  fifth region of the crRNA(wild-type), 15nt deletion
uagacgaaugaagga

SEQ ID NO: 97 - RNA, 16 nt, Artificial Sequence
  fifth region of the crRNA(wild-type), 14nt deletion
auagacgaaugaagga

SEQ ID NO: 98 - RNA, 17 nt, Artificial Sequence
  fifth region of the crRNA(wild-type), 13nt deletion
aauagacgaaugaagga

SEQ ID NO: 99 - RNA, 18 nt, Artificial Sequence
  fifth region of the crRNA(wild-type), 12nt deletion
gaauagacgaaugaagga

SEQ ID NO: 100 - RNA, 19 nt, Artificial Sequence
  fifth region of the crRNA(wild-type), 11nt deletion
cgaauagacgaaugaagga

SEQ ID NO: 101 - RNA, 20 nt, Artificial Sequence
  fifth region of the crRNA(wild-type), 10nt deletion
ccgaauagacgaaugaagga

SEQ ID NO: 102 - RNA, 21 nt, Artificial Sequence
  fifth region of the crRNA(wild-type), 9nt deletion
cccgaauagacgaaugaagga

SEQ ID NO: 103 - RNA, 22 nt, Artificial Sequence
  fifth region of the crRNA(wild-type), 8nt deletion
acccgaauagacgaaugaagga

SEQ ID NO: 104 - RNA, 23 nt, Artificial Sequence
  fifth region of the crRNA(wild-type), 7nt deletion
aacccgaauagacgaaugaagga

SEQ ID NO: 105 - RNA, 24 nt, Artificial Sequence
  fifth region of the crRNA(wild-type), 6nt deletion
gaacccgaauagacgaaugaagga

SEQ ID NO: 106 - RNA, 25 nt, Artificial Sequence
  fifth region of the crRNA(wild-type), 5nt deletion
agaacccgaauagacgaaugaagga

SEQ ID NO: 107 - RNA, 26 nt, Artificial Sequence
  fifth region of the crRNA(wild-type), 4nt deletion
cagaacccgaauagacgaaugaagga

SEQ ID NO: 108 - RNA, 27 nt, Artificial Sequence
  fifth region of the crRNA(wild-type), 3nt deletion
gcagaacccgaauagacgaaugaagga

SEQ ID NO: 109 - RNA, 28 nt, Artificial Sequence
  fifth region of the crRNA(wild-type), 2nt deletion
ugcagaacccgaauagacgaaugaagga

SEQ ID NO: 110 - RNA, 29 nt, Artificial Sequence
  fifth region of the crRNA(wild-type), 1nt deletion
uugcagaacccgaauagacgaaugaagga

SEQ ID NO: 111 - RNA, 13 nt, Artificial Sequence
  fourth region + Linker + fifth region, 7bp deletion (mature form)
aacaaagaaagga

SEQ ID NO: 112 - RNA, 15 nt, Artificial Sequence
  fourth region + Linker + fifth region, 6bp deletion (mature form)
aacaaaugaaaagga

SEQ ID NO: 113 - RNA, 17 nt, Artificial Sequence
  fourth region + Linker + fifth region, 5bp deletion (mature form)
aacaaauugaaaaagga

SEQ ID NO: 114 - RNA, 19 nt, Artificial Sequence
  fourth region + Linker + fifth region, 4bp deletion (mature form)
aacaaauucgaaagaagga

SEQ ID NO: 115 - RNA, 21 nt, Artificial Sequence
  fourth region + Linker + fifth region, 3bp deletion (mature form)
aacaaauucagaaaugaagga

SEQ ID NO: 116 - RNA, 23 nt, Artificial Sequence
  fourth region + Linker + fifth region, 2bp deletion (mature form)
aacaaauucaugaaaaugaagga

SEQ ID NO: 117 - RNA, 25 nt, Artificial Sequence
  fourth region + Linker + fifth region, 1bp deletion (mature form)
aacaaauucauugaaaaaugaagga

SEQ ID NO: 118 - RNA, 27 nt, Artificial Sequence
  fourth region + Linker + fifth region (mature form)
aacaaauucauuugaaagaaugaagga

SEQ ID NO: 119 - RNA, 120 nt, Artificial Sequence
  engineered tracrRNA(mature form, 20nt deletion in the first region)
accgcuucaccaaaagcugucccuuaggggauuagaacuugagugaaggugggcugcuugcaucagccuaaugucgagaagugcuuucuucggaaaguaacccucgaaacaaauucauuu

SEQ ID NO: 120 - RNA, 121 nt, Artificial Sequence
  engineered tracrRNA(mature form, 19nt deletion in the first region)
aaccgcuucaccaaaagcugucccuuaggggauuagaacuugagugaaggugggcugcuugcaucagccuaaugucgagaagugcuuucuucggaaaguaacccucgaaacaaauucauuu

SEQ ID NO: 121 - RNA, 122 nt, Artificial Sequence
  engineered tracrRNA(mature form, 18nt deletion in the first region)
gaaccgcuucaccaaaagcugucccuuaggggauuagaacuugagugaaggugggcugcuugcaucagccuaaugucgagaagugcuuucuucggaaaguaacccucgaaacaaauucauuu

SEQ ID NO: 122 - RNA, 123 nt, Artificial Sequence
  engineered tracrRNA(mature form, 17nt deletion in the first region)
agaaccgcuucaccaaaagcugucccuuaggggauuagaacuugagugaaggugggcugcuugcaucagccuaaugucgagaagugcuuucuucggaaaguaacccucgaaacaaauucauuu

SEQ ID NO: 123 - RNA, 124 nt, Artificial Sequence
  engineered tracrRNA(mature form, 16nt deletion in the first region)
gagaaccgcuucaccaaaagcugucccuuaggggauuagaacuugagugaaggugggcugcuugcaucagccuaaugucgagaagugcuuucuucggaaaguaacccucgaaacaaauucauuu

SEQ ID NO: 124 - RNA, 125 nt, Artificial Sequence
  engineered tracrRNA(mature form, 15nt deletion in the first region)
ggagaaccgcuucaccaaaagcugucccuuaggggauuagaacuugagugaaggugggcugcuugcaucagccuaaugucgagaagugcuuucuucggaaaguaacccucgaaacaaauucauuu

SEQ ID NO: 125 - RNA, 126 nt, Artificial Sequence
  engineered tracrRNA(mature form, 14nt deletion in the first region)
uggagaaccgcuucaccaaaagcugucccuuaggggauuagaacuugagugaaggugggcugcuugcaucagccuaaugucgagaagugcuuucuucggaaaguaacccucgaaacaaauucauuu

SEQ ID NO: 126 - RNA, 127 nt, Artificial Sequence
  engineered tracrRNA(mature form, 13nt deletion in the first region)
guggagaaccgcuucaccaaaagcugucccuuaggggauuagaacuugagugaaggugggcugcuugcaucagccuaaugucgagaagugcuuucuucggaaaguaacccucgaaacaaauucauuu

SEQ ID NO: 127 - RNA, 128 nt, Artificial Sequence
  engineered tracrRNA(mature form, 12nt deletion in the first region)
aguggagaaccgcuucaccaaaagcugucccuuaggggauuagaacuugagugaaggugggcugcuugcaucagccuaaugucgagaagugcuuucuucggaaaguaacccucgaaacaaauucauuu

SEQ ID NO: 128 - RNA, 129 nt, Artificial Sequence
  engineered tracrRNA(mature form, 11nt deletion in the first region)
aaguggagaaccgcuucaccaaaagcugucccuuaggggauuagaacuugagugaaggugggcugcuugcaucagccuaaugucgagaagugcuuucuucggaaaguaacccucgaaacaaauucauuu

SEQ ID NO: 129 - RNA, 130 nt, Artificial Sequence
  engineered tracrRNA(mature form, 10nt deletion in the first region)
aaaguggagaaccgcuucaccaaaagcugucccuuaggggauuagaacuugagugaaggugggcugcuugcaucagccuaaugucgagaagugcuuucuucggaaaguaacccucgaaacaaauucauuu

SEQ ID NO: 130 - RNA, 131 nt, Artificial Sequence
  engineered tracrRNA(mature form, 9nt deletion in the first region)
uaaaguggagaaccgcuucaccaaaagcugucccuuaggggauuagaacuugagugaaggugggcugcuugcaucagccuaaugucgagaagugcuuucuucggaaaguaacccucgaaacaaauucauuu

SEQ ID NO: 131 - RNA, 132 nt, Artificial Sequence
  engineered tracrRNA(mature form, 8nt deletion in the first region)
auaaaguggagaaccgcuucaccaaaagcugucccuuaggggauuagaacuugagugaaggugggcugcuugcaucagccuaaugucgagaagugcuuucuucggaaaguaacccucgaaacaaauucauuu

SEQ ID NO: 132 - RNA, 133 nt, Artificial Sequence
  engineered tracrRNA(mature form, 7nt deletion in the first region)
gauaaaguggagaaccgcuucaccaaaagcugucccuuaggggauuagaacuugagugaaggugggcugcuugcaucagccuaaugucgagaagugcuuucuucggaaaguaacccucgaaacaaauucauuu

SEQ ID NO: 133 - RNA, 134 nt, Artificial Sequence
  engineered tracrRNA(mature form, 6nt deletion in the first region)
ugauaaaguggagaaccgcuucaccaaaagcugucccuuaggggauuagaacuugagugaaggugggcugcuugcaucagccuaaugucgagaagugcuuucuucggaaaguaacccucgaaacaaauucauuu

SEQ ID NO: 134 - RNA, 135 nt, Artificial Sequence
  engineered tracrRNA(mature form, 5nt deletion in the first region)
cugauaaaguggagaaccgcuucaccaaaagcugucccuuaggggauuagaacuugagugaaggugggcugcuugcaucagccuaaugucgagaagugcuuucuucggaaaguaacccucgaaacaaauucauuu

SEQ ID NO: 135 - RNA, 136 nt, Artificial Sequence
  engineered tracrRNA(mature form, 4nt deletion in the first region)
acugauaaaguggagaaccgcuucaccaaaagcugucccuuaggggauuagaacuugagugaaggugggcugcuugcaucagccuaaugucgagaagugcuuucuucggaaaguaacccucgaaacaaauucauuu

SEQ ID NO: 136 - RNA, 137 nt, Artificial Sequence
  engineered tracrRNA(mature form, 3nt deletion in the first region)
cacugauaaaguggagaaccgcuucaccaaaagcugucccuuaggggauuagaacuugagugaaggugggcugcuugcaucagccuaaugucgagaagugcuuucuucggaaaguaacccucgaaacaaauucauuu

SEQ ID NO: 137 - RNA, 138 nt, Artificial Sequence
  engineered tracrRNA(mature form, 2nt deletion in the first region)
ucacugauaaaguggagaaccgcuucaccaaaagcugucccuuaggggauuagaacuugagugaaggugggcugcuugcaucagccuaaugucgagaagugcuuucuucggaaaguaacccucgaaacaaauucauuu

SEQ ID NO: 138 - RNA, 139 nt, Artificial Sequence
  engineered tracrRNA(mature form, 1nt deletion in the first region)
uucacugauaaaguggagaaccgcuucaccaaaagcugucccuuaggggauuagaacuugagugaaggugggcugcuugcaucagccuaaugucgagaagugcuuucuucggaaaguaacccucgaaacaaauucauuu

SEQ ID NO: 139 - RNA, 117 nt, Artificial Sequence
  engineered tracrRNA(mature form, 10bp deletion in the second region)
cuucacugauaaaguggagaaccgcuucaccauuagugagugaaggugggcugcuugcaucagccuaaugucgagaagugcuuucuucggaaaguaacccucgaaacaaauucauuu

SEQ ID NO: 140 - RNA, 119 nt, Artificial Sequence
  engineered tracrRNA(mature form, 9bp deletion in the second region)
cuucacugauaaaguggagaaccgcuucaccaauuaguugagugaaggugggcugcuugcaucagccuaaugucgagaagugcuuucuucggaaaguaacccucgaaacaaauucauuu

SEQ ID NO: 141 - RNA, 122 nt, Artificial Sequence
  engineered tracrRNA(mature form, 8bp deletion in the second region)
cuucacugauaaaguggagaaccgcuucaccaaauuagacuugagugaaggugggcugcuugcaucagccuaaugucgagaagugcuuucuucggaaaguaacccucgaaacaaauucauuu

SEQ ID NO: 142 - RNA, 125 nt, Artificial Sequence
  engineered tracrRNA(mature form, 7bp deletion in the second region)
cuucacugauaaaguggagaaccgcuucaccaaaaguuagaacuugagugaaggugggcugcuugcaucagccuaaugucgagaagugcuuucuucggaaaguaacccucgaaacaaauucauuu

SEQ ID NO: 143 - RNA, 127 nt, Artificial Sequence
  engineered tracrRNA(mature form, 6bp deletion in the second region)
cuucacugauaaaguggagaaccgcuucaccaaaagcuuaggaacuugagugaaggugggcugcuugcaucagccuaaugucgagaagugcuuucuucggaaaguaacccucgaaacaaauucauuu

SEQ ID NO: 144 - RNA, 129 nt, Artificial Sequence
  engineered tracrRNA(mature form, 5bp deletion in the second region)
cuucacugauaaaguggagaaccgcuucaccaaaagcuuuagagaacuugagugaaggugggcugcuugcaucagccuaaugucgagaagugcuuucuucggaaaguaacccucgaaacaaauucauuu

SEQ ID NO: 145 - RNA, 132 nt, Artificial Sequence
  engineered tracrRNA(mature form, 4bp deletion in the second region)
cuucacugauaaaguggagaaccgcuucaccaaaagcuguuaguuagaacuugagugaaggugggcugcuugcaucagccuaaugucgagaagugcuuucuucggaaaguaacccucgaaacaaauucauuu

SEQ ID NO: 146 - RNA, 131 nt, Artificial Sequence
  engineered tracrRNA(mature form, 4bp+1nt deletion in the second region)
cuucacugauaaaguggagaaccgcuucaccaaaagcuguuaguagaacuugagugaaggugggcugcuugcaucagccuaaugucgagaagugcuuucuucggaaaguaacccucgaaacaaauucauuu

SEQ ID NO: 147 - RNA, 134 nt, Artificial Sequence
  engineered tracrRNA(mature form, 3bp deletion in the second region)
cuucacugauaaaguggagaaccgcuucaccaaaagcuguuuagauuagaacuugagugaaggugggcugcuugcaucagccuaaugucgagaagugcuuucuucggaaaguaacccucgaaacaaauucauuu

SEQ ID NO: 148 - RNA, 136 nt, Artificial Sequence
  engineered tracrRNA(mature form, 2bp deletion in the second region)
cuucacugauaaaguggagaaccgcuucaccaaaagcugucuuaggauuagaacuugagugaaggugggcugcuugcaucagccuaaugucgagaagugcuuucuucggaaaguaacccucgaaacaaauucauuu

SEQ ID NO: 149 - RNA, 138 nt, Artificial Sequence
  engineered tracrRNA(mature form, 1bp deletion in the second region)
cuucacugauaaaguggagaaccgcuucaccaaaagcuguccuuagggauuagaacuugagugaaggugggcugcuugcaucagccuaaugucgagaagugcuuucuucggaaaguaacccucgaaacaaauucauuu

SEQ ID NO: 150 - RNA, 133 nt, Artificial Sequence
  engineered tracrRNA(mature form, 7nt deletion in the fourth region)
cuucacugauaaaguggagaaccgcuucaccaaaagcugucccuuaggggauuagaacuugagugaaggugggcugcuugcaucagccuaaugucgagaagugcuuucuucggaaaguaacccucgaaacaaa

SEQ ID NO: 151 - RNA, 134 nt, Artificial Sequence
  engineered tracrRNA(mature form, 6nt deletion in the fourth region)
cuucacugauaaaguggagaaccgcuucaccaaaagcugucccuuaggggauuagaacuugagugaaggugggcugcuugcaucagccuaaugucgagaagugcuuucuucggaaaguaacccucgaaacaaau

SEQ ID NO: 152 - RNA, 135 nt, Artificial Sequence
  engineered tracrRNA(mature form, 5nt deletion in the fourth region)
cuucacugauaaaguggagaaccgcuucaccaaaagcugucccuuaggggauuagaacuugagugaaggugggcugcuugcaucagccuaaugucgagaagugcuuucuucggaaaguaacccucgaaacaaauu

SEQ ID NO: 153 - RNA, 136 nt, Artificial Sequence
  engineered tracrRNA(mature form, 4nt deletion in the fourth region)
cuucacugauaaaguggagaaccgcuucaccaaaagcugucccuuaggggauuagaacuugagugaaggugggcugcuugcaucagccuaaugucgagaagugcuuucuucggaaaguaacccucgaaacaaauuc

SEQ ID NO: 154 - RNA, 137 nt, Artificial Sequence
  engineered tracrRNA(mature form, 3nt deletion in the fourth region)
cuucacugauaaaguggagaaccgcuucaccaaaagcugucccuuaggggauuagaacuugagugaaggugggcugcuugcaucagccuaaugucgagaagugcuuucuucggaaaguaacccucgaaacaaauuca

SEQ ID NO: 155 - RNA, 138 nt, Artificial Sequence
  engineered tracrRNA(mature form, 2nt deletion in the fourth region)
cuucacugauaaaguggagaaccgcuucaccaaaagcugucccuuaggggauuagaacuugagugaaggugggcugcuugcaucagccuaaugucgagaagugcuuucuucggaaaguaacccucgaaacaaauucau

SEQ ID NO: 156 - RNA, 139 nt, Artificial Sequence
  engineered tracrRNA(mature form, 1nt deletion in the fourth region)
cuucacugauaaaguggagaaccgcuucaccaaaagcugucccuuaggggauuagaacuugagugaaggugggcugcuugcaucagccuaaugucgagaagugcuuucuucggaaaguaacccucgaaacaaauucauu

SEQ ID NO: 157 - RNA, 97 nt, Artificial Sequence
  engineered tracrRNA(mature form, modified first region and modified second region)
accgcuucaccauuagugagugaaggugggcugcuugcaucagccuaaugucgagaagugcuuucuucggaaaguaacccucgaaacaaauucauuu

SEQ ID NO: 158 - RNA, 113 nt, Artificial Sequence
  engineered tracrRNA(mature form, modified first region and modified fourth and fifth region)
accgcuucaccaaaagcugucccuuaggggauuagaacuugagugaaggugggcugcuugcaucagccuaaugucgagaagugcuuucuucggaaaguaacccucgaaacaaa

SEQ ID NO: 159 - RNA, 110 nt, Artificial Sequence
  engineered tracrRNA(mature form, modified second region and modified fourth and fifth region)
cuucacugauaaaguggagaaccgcuucaccauuagugagugaaggugggcugcuugcaucagccuaaugucgagaagugcuuucuucggaaaguaacccucgaaacaaa

SEQ ID NO: 160 - RNA, 90 nt, Artificial Sequence
  engineered tracrRNA(mature form, modified first region, modified second region, modified fourth and fifth region)
accgcuucaccauuagugagugaaggugggcugcuugcaucagccuaaugucgagaagugcuuucuucggaaaguaacccucgaaacaaa

SEQ ID NO: 161 - RNA, 10 nt, Artificial Sequence
  engineered crRNA repeat(mature form, 7nt deletion in the fifth region)
ggaaugcaac

SEQ ID NO: 162 - RNA, 11 nt, Artificial Sequence
  engineered crRNA repeat(mature form, 6nt deletion in the fifth region)
aggaaugcaac

SEQ ID NO: 163 - RNA, 12 nt, Artificial Sequence
  engineered crRNA repeat(mature form, 5nt deletion in the fifth region)
aaggaaugcaac

SEQ ID NO: 164 - RNA, 13 nt, Artificial Sequence
  engineered crRNA repeat(mature form, 4nt deletion in the fifth region)
gaaggaaugcaac

SEQ ID NO: 165 - RNA, 14 nt, Artificial Sequence
  engineered crRNA repeat(mature form, 3nt deletion in the fifth region)
ugaaggaaugcaac

SEQ ID NO: 166 - RNA, 15 nt, Artificial Sequence
  engineered crRNA repeat(mature form, 2nt deletion in the fifth region)
augaaggaaugcaac

SEQ ID NO: 167 - RNA, 16 nt, Artificial Sequence
  engineered crRNA repeat(mature form, 1nt deletion in the fifth region)
aaugaaggaaugcaac

SEQ ID NO: 168 - RNA, 141 nt, Artificial Sequence
  engineered scaffold(mature form, 20nt deletion in the first region)
accgcuucaccaaaagcugucccuuaggggauuagaacuugagugaaggugggcugcuugcaucagccuaaugucgagaagugcuuucuucggaaaguaacccucgaaacaaauucauuugaaagaaugaaggaaugcaac

SEQ ID NO: 169 - RNA, 142 nt, Artificial Sequence
  engineered scaffold(mature form, 19nt deletion in the first region)
aaccgcuucaccaaaagcugucccuuaggggauuagaacuugagugaaggugggcugcuugcaucagccuaaugucgagaagugcuuucuucggaaaguaacccucgaaacaaauucauuugaaagaaugaaggaaugcaac

SEQ ID NO: 170 - RNA, 143 nt, Artificial Sequence
  engineered scaffold(mature form, 18nt deletion in the first region)
gaaccgcuucaccaaaagcugucccuuaggggauuagaacuugagugaaggugggcugcuugcaucagccuaaugucgagaagugcuuucuucggaaaguaacccucgaaacaaauucauuugaaagaaugaaggaaugcaac

SEQ ID NO: 171 - RNA, 144 nt, Artificial Sequence
  engineered scaffold(mature form, 17nt deletion in the first region)
agaaccgcuucaccaaaagcugucccuuaggggauuagaacuugagugaaggugggcugcuugcaucagccuaaugucgagaagugcuuucuucggaaaguaacccucgaaacaaauucauuugaaagaaugaaggaaugcaac

SEQ ID NO: 172 - RNA, 145 nt, Artificial Sequence
  engineered scaffold(mature form, 16nt deletion in the first region)
gagaaccgcuucaccaaaagcugucccuuaggggauuagaacuugagugaaggugggcugcuugcaucagccuaaugucgagaagugcuuucuucggaaaguaacccucgaaacaaauucauuugaaagaaugaaggaaugcaac

SEQ ID NO: 173 - RNA, 146 nt, Artificial Sequence
  engineered scaffold(mature form, 15nt deletion in the first region)
ggagaaccgcuucaccaaaagcugucccuuaggggauuagaacuugagugaaggugggcugcuugcaucagccuaaugucgagaagugcuuucuucggaaaguaacccucgaaacaaauucauuugaaagaaugaaggaaugcaac

SEQ ID NO: 174 - RNA, 147 nt, Artificial Sequence
  engineered scaffold(mature form, 14nt deletion in the first region)
uggagaaccgcuucaccaaaagcugucccuuaggggauuagaacuugagugaaggugggcugcuugcaucagccuaaugucgagaagugcuuucuucggaaaguaacccucgaaacaaauucauuugaaagaaugaaggaaugcaac

SEQ ID NO: 175 - RNA, 148 nt, Artificial Sequence
  engineered scaffold(mature form, 13nt deletion in the first region)
guggagaaccgcuucaccaaaagcugucccuuaggggauuagaacuugagugaaggugggcugcuugcaucagccuaaugucgagaagugcuuucuucggaaaguaacccucgaaacaaauucauuugaaagaaugaaggaaugcaac

SEQ ID NO: 176 - RNA, 149 nt, Artificial Sequence
  engineered scaffold(mature form, 12nt deletion in the first region)
aguggagaaccgcuucaccaaaagcugucccuuaggggauuagaacuugagugaaggugggcugcuugcaucagccuaaugucgagaagugcuuucuucggaaaguaacccucgaaacaaauucauuugaaagaaugaaggaaugcaac

SEQ ID NO: 177 - RNA, 150 nt, Artificial Sequence
  engineered scaffold(mature form, 11nt deletion in the first region)
aaguggagaaccgcuucaccaaaagcugucccuuaggggauuagaacuugagugaaggugggcugcuugcaucagccuaaugucgagaagugcuuucuucggaaaguaacccucgaaacaaauucauuugaaagaaugaaggaaugcaac

SEQ ID NO: 178 - RNA, 151 nt, Artificial Sequence
  engineered scaffold(mature form, 10nt deletion in the first region)
aaaguggagaaccgcuucaccaaaagcugucccuuaggggauuagaacuugagugaaggugggcugcuugcaucagccuaaugucgagaagugcuuucuucggaaaguaacccucgaaacaaauucauuugaaagaaugaaggaaugcaac

SEQ ID NO: 179 - RNA, 152 nt, Artificial Sequence
  engineered scaffold(mature form, 9nt deletion in the first region)
uaaaguggagaaccgcuucaccaaaagcugucccuuaggggauuagaacuugagugaaggugggcugcuugcaucagccuaaugucgagaagugcuuucuucggaaaguaacccucgaaacaaauucauuugaaagaaugaaggaaugcaac

SEQ ID NO: 180 - RNA, 153 nt, Artificial Sequence
  engineered scaffold(mature form, 8nt deletion in the first region)
auaaaguggagaaccgcuucaccaaaagcugucccuuaggggauuagaacuugagugaaggugggcugcuugcaucagccuaaugucgagaagugcuuucuucggaaaguaacccucgaaacaaauucauuugaaagaaugaaggaaugcaac

SEQ ID NO: 181 - RNA, 154 nt, Artificial Sequence
  engineered scaffold(mature form, 7nt deletion in the first region)
gauaaaguggagaaccgcuucaccaaaagcugucccuuaggggauuagaacuugagugaaggugggcugcuugcaucagccuaaugucgagaagugcuuucuucggaaaguaacccucgaaacaaauucauuugaaagaaugaaggaaugcaac

SEQ ID NO: 182 - RNA, 155 nt, Artificial Sequence
  engineered scaffold(mature form, 6nt deletion in the first region)
ugauaaaguggagaaccgcuucaccaaaagcugucccuuaggggauuagaacuugagugaaggugggcugcuugcaucagccuaaugucgagaagugcuuucuucggaaaguaacccucgaaacaaauucauuugaaagaaugaaggaaugcaac

SEQ ID NO: 183 - RNA, 156 nt, Artificial Sequence
  engineered scaffold(mature form, 5nt deletion in the first region)
cugauaaaguggagaaccgcuucaccaaaagcugucccuuaggggauuagaacuugagugaaggugggcugcuugcaucagccuaaugucgagaagugcuuucuucggaaaguaacccucgaaacaaauucauuugaaagaaugaaggaaugcaac

SEQ ID NO: 184 - RNA, 157 nt, Artificial Sequence
  engineered scaffold(mature form, 4nt deletion in the first region)
acugauaaaguggagaaccgcuucaccaaaagcugucccuuaggggauuagaacuugagugaaggugggcugcuugcaucagccuaaugucgagaagugcuuucuucggaaaguaacccucgaaacaaauucauuugaaagaaugaaggaaugcaac

SEQ ID NO: 185 - RNA, 158 nt, Artificial Sequence
  engineered scaffold(mature form, 3nt deletion in the first region)
cacugauaaaguggagaaccgcuucaccaaaagcugucccuuaggggauuagaacuugagugaaggugggcugcuugcaucagccuaaugucgagaagugcuuucuucggaaaguaacccucgaaacaaauucauuugaaagaaugaaggaaugcaac

SEQ ID NO: 186 - RNA, 159 nt, Artificial Sequence
  engineered scaffold(mature form, 2nt deletion in the first region)
ucacugauaaaguggagaaccgcuucaccaaaagcugucccuuaggggauuagaacuugagugaaggugggcugcuugcaucagccuaaugucgagaagugcuuucuucggaaaguaacccucgaaacaaauucauuugaaagaaugaaggaaugcaac

SEQ ID NO: 187 - RNA, 160 nt, Artificial Sequence
  engineered scaffold(mature form, 1nt deletion in the first region)
uucacugauaaaguggagaaccgcuucaccaaaagcugucccuuaggggauuagaacuugagugaaggugggcugcuugcaucagccuaaugucgagaagugcuuucuucggaaaguaacccucgaaacaaauucauuugaaagaaugaaggaaugcaac

SEQ ID NO: 188 - RNA, 138 nt, Artificial Sequence
  engineered scaffold(mature form, 11bp deletion in the second region)
cuucacugauaaaguggagaaccgcuucaccauuagugagugaaggugggcugcuugcaucagccuaaugucgagaagugcuuucuucggaaaguaacccucgaaacaaauucauuugaaagaaugaaggaaugcaac

SEQ ID NO: 189 - RNA, 140 nt, Artificial Sequence
  engineered scaffold(mature form, 10bp deletion in the second region)
cuucacugauaaaguggagaaccgcuucaccaauuaguugagugaaggugggcugcuugcaucagccuaaugucgagaagugcuuucuucggaaaguaacccucgaaacaaauucauuugaaagaaugaaggaaugcaac

SEQ ID NO: 190 - RNA, 142 nt, Artificial Sequence
  engineered scaffold(mature form, 9bp deletion in the second region)
cuucacugauaaaguggagaaccgcuucaccaaauuagcuugagugaaggugggcugcuugcaucagccuaaugucgagaagugcuuucuucggaaaguaacccucgaaacaaauucauuugaaagaaugaaggaaugcaac

SEQ ID NO: 191 - RNA, 144 nt, Artificial Sequence
  engineered scaffold(mature form, 8bp deletion in the second region)
cuucacugauaaaguggagaaccgcuucaccaaaauuagacuugagugaaggugggcugcuugcaucagccuaaugucgagaagugcuuucuucggaaaguaacccucgaaacaaauucauuugaaagaaugaaggaaugcaac

SEQ ID NO: 192 - RNA, 146 nt, Artificial Sequence
  engineered scaffold(mature form, 7bp deletion in the second region)
cuucacugauaaaguggagaaccgcuucaccaaaaguuagaacuugagugaaggugggcugcuugcaucagccuaaugucgagaagugcuuucuucggaaaguaacccucgaaacaaauucauuugaaagaaugaaggaaugcaac

SEQ ID NO: 193 - RNA, 148 nt, Artificial Sequence
  engineered scaffold(mature form, 6bp deletion in the second region)
cuucacugauaaaguggagaaccgcuucaccaaaagcuuaggaacuugagugaaggugggcugcuugcaucagccuaaugucgagaagugcuuucuucggaaaguaacccucgaaacaaauucauuugaaagaaugaaggaaugcaac

SEQ ID NO: 194 - RNA, 150 nt, Artificial Sequence
  engineered scaffold(mature form, 5bp deletion in the second region)
cuucacugauaaaguggagaaccgcuucaccaaaagcuuuagagaacuugagugaaggugggcugcuugcaucagccuaaugucgagaagugcuuucuucggaaaguaacccucgaaacaaauucauuugaaagaaugaaggaaugcaac

SEQ ID NO: 195 - RNA, 152 nt, Artificial Sequence
  engineered scaffold(mature form, 4bp deletion in the second region)
cuucacugauaaaguggagaaccgcuucaccaaaagcuguuaguagaacuugagugaaggugggcugcuugcaucagccuaaugucgagaagugcuuucuucggaaaguaacccucgaaacaaauucauuugaaagaaugaaggaaugcaac

SEQ ID NO: 196 - RNA, 153 nt, Artificial Sequence
  engineered scaffold(mature form, 4bp+1nt deletion in the second region)
cuucacugauaaaguggagaaccgcuucaccaaaagcuguuaguuagaacuugagugaaggugggcugcuugcaucagccuaaugucgagaagugcuuucuucggaaaguaacccucgaaacaaauucauuugaaagaaugaaggaaugcaac

SEQ ID NO: 197 - RNA, 155 nt, Artificial Sequence
  engineered scaffold(mature form, 3bp deletion in the second region)
cuucacugauaaaguggagaaccgcuucaccaaaagcuguuuagauuagaacuugagugaaggugggcugcuugcaucagccuaaugucgagaagugcuuucuucggaaaguaacccucgaaacaaauucauuugaaagaaugaaggaaugcaac

SEQ ID NO: 198 - RNA, 157 nt, Artificial Sequence
  engineered scaffold(mature form, 2bp deletion in the second region)
cuucacugauaaaguggagaaccgcuucaccaaaagcugucuuaggauuagaacuugagugaaggugggcugcuugcaucagccuaaugucgagaagugcuuucuucggaaaguaacccucgaaacaaauucauuugaaagaaugaaggaaugcaac

SEQ ID NO: 199 - RNA, 159 nt, Artificial Sequence
  engineered scaffold(mature form, 1bp deletion in the second region)
cuucacugauaaaguggagaaccgcuucaccaaaagcuguccuuagggauuagaacuugagugaaggugggcugcuugcaucagccuaaugucgagaagugcuuucuucggaaaguaacccucgaaacaaauucauuugaaagaaugaaggaaugcaac

SEQ ID NO: 200 - RNA, 147 nt, Artificial Sequence
  engineered scaffold(mature form, 7bp deletion in the fourth and fifth region)
cuucacugauaaaguggagaaccgcuucaccaaaagcugucccuuaggggauuagaacuugagugaaggugggcugcuugcaucagccuaaugucgagaagugcuuucuucggaaaguaacccucgaaacaaagaaaggaaugcaac

SEQ ID NO: 201 - RNA, 149 nt, Artificial Sequence
  engineered scaffold(mature form, 6bp deletion in the fourth and fifth region)
cuucacugauaaaguggagaaccgcuucaccaaaagcugucccuuaggggauuagaacuugagugaaggugggcugcuugcaucagccuaaugucgagaagugcuuucuucggaaaguaacccucgaaacaaaugaaaaggaaugcaac

SEQ ID NO: 202 - RNA, 151 nt, Artificial Sequence
  engineered scaffold(mature form, 5bp deletion in the fourth and fifth region)
cuucacugauaaaguggagaaccgcuucaccaaaagcugucccuuaggggauuagaacuugagugaaggugggcugcuugcaucagccuaaugucgagaagugcuuucuucggaaaguaacccucgaaacaaauugaaaaaggaaugcaac

SEQ ID NO: 203 - RNA, 153 nt, Artificial Sequence
  engineered scaffold(mature form, 4bp deletion in the fourth and fifth region)
cuucacugauaaaguggagaaccgcuucaccaaaagcugucccuuaggggauuagaacuugagugaaggugggcugcuugcaucagccuaaugucgagaagugcuuucuucggaaaguaacccucgaaacaaauucgaaagaaggaaugcaac

SEQ ID NO: 204 - RNA, 155 nt, Artificial Sequence
  engineered scaffold(mature form, 3bp deletion in the fourth and fifth region)
cuucacugauaaaguggagaaccgcuucaccaaaagcugucccuuaggggauuagaacuugagugaaggugggcugcuugcaucagccuaaugucgagaagugcuuucuucggaaaguaacccucgaaacaaauucagaaaugaaggaaugcaac

SEQ ID NO: 205 - RNA, 157 nt, Artificial Sequence
  engineered scaffold(mature form, 2bp deletion in the fourth and fifth region)
cuucacugauaaaguggagaaccgcuucaccaaaagcugucccuuaggggauuagaacuugagugaaggugggcugcuugcaucagccuaaugucgagaagugcuuucuucggaaaguaacccucgaaacaaauucaugaaaaugaaggaaugcaac

SEQ ID NO: 206 - RNA, 159 nt, Artificial Sequence
  engineered scaffold(mature form, 1bp deletion in the fourth and fifth region)
cuucacugauaaaguggagaaccgcuucaccaaaagcugucccuuaggggauuagaacuugagugaaggugggcugcuugcaucagccuaaugucgagaagugcuuucuucggaaaguaacccucgaaacaaauucauugaaaaaugaaggaaugcaac

SEQ ID NO: 207 - RNA, 118 nt, Artificial Sequence
  engineered scaffold(mature form, modified first and second region)
accgcuucaccauuagugagugaaggugggcugcuugcaucagccuaaugucgagaagugcuuucuucggaaaguaacccucgaaacaaauucauuugaaagaaugaaggaaugcaac

SEQ ID NO: 208 - RNA, 127 nt, Artificial Sequence
  engineered scaffold(mature form, modified first, fourth and fifth region)
accgcuucaccaaaagcugucccuuaggggauuagaacuugagugaaggugggcugcuugcaucagccuaaugucgagaagugcuuucuucggaaaguaacccucgaaacaaagaaaggaaugcaac

SEQ ID NO: 209 - RNA, 121 nt, Artificial Sequence
  engineered scaffold(mature form, modified second, fourth and fifth region)
cuucacugauaaaguggagaaccgcuucacuuagagugaagguggggcugcuugcaucagccuaaugucgagaagugcuuucuucggaaaguaacccucgaaacaaagaaaggaaugcaac

SEQ ID NO: 210 - RNA, 101 nt, Artificial Sequence
  engineered scaffold(mature form, modified first, second, fourth and fifth region)
accgcuucacuuagagugaagguggggcugcuugcaucagccuaaugucgagaagugcuuucuucggaaaguaacccucgaaacaaagaaaggaaugcaac

SEQ ID NO: 211 - RNA, 189 nt, Artificial Sequence
  sgRNA(mature form, 1nt deletion in the first region)
uucacugauaaaguggagaaccgcuucaccaaaagcugucccuuaggggauuagaacuugagugaaggugggcugcuugcaucagccuaaugucgagaagugcuuucuucggaaaguaacccucgaaacaaauucauuugaaagaaugaaggaaugcaacnnnnnnnnnnnnnnnnnnnnuuuuauuuu

SEQ ID NO: 212 - RNA, 188 nt, Artificial Sequence
  sgRNA(mature form, 2nt deletion in the first region)
ucacugauaaaguggagaaccgcuucaccaaaagcugucccuuaggggauuagaacuugagugaaggugggcugcuugcaucagccuaaugucgagaagugcuuucuucggaaaguaacccucgaaacaaauucauuugaaagaaugaaggaaugcaacnnnnnnnnnnnnnnnnnnnnuuuuauuuu

SEQ ID NO: 213 - RNA, 187 nt, Artificial Sequence
  sgRNA(mature form, 3nt deletion in the first region)
cacugauaaaguggagaaccgcuucaccaaaagcugucccuuaggggauuagaacuugagugaaggugggcugcuugcaucagccuaaugucgagaagugcuuucuucggaaaguaacccucgaaacaaauucauuugaaagaaugaaggaaugcaacnnnnnnnnnnnnnnnnnnnnuuuuauuuu

SEQ ID NO: 214 - RNA, 186 nt, Artificial Sequence
  sgRNA(mature form, 4nt deletion in the first region)
acugauaaaguggagaaccgcuucaccaaaagcugucccuuaggggauuagaacuugagugaaggugggcugcuugcaucagccuaaugucgagaagugcuuucuucggaaaguaacccucgaaacaaauucauuugaaagaaugaaggaaugcaacnnnnnnnnnnnnnnnnnnnnuuuuauuuu

SEQ ID NO: 215 - RNA, 185 nt, Artificial Sequence
  sgRNA(mature form, 5nt deletion in the first region)
cugauaaaguggagaaccgcuucaccaaaagcugucccuuaggggauuagaacuugagugaaggugggcugcuugcaucagccuaaugucgagaagugcuuucuucggaaaguaacccucgaaacaaauucauuugaaagaaugaaggaaugcaacnnnnnnnnnnnnnnnnnnnnuuuuauuuu

SEQ ID NO: 216 - RNA, 184 nt, Artificial Sequence
  sgRNA(mature form, 6nt deletion in the first region)
ugauaaaguggagaaccgcuucaccaaaagcugucccuuaggggauuagaacuugagugaaggugggcugcuugcaucagccuaaugucgagaagugcuuucuucggaaaguaacccucgaaacaaauucauuugaaagaaugaaggaaugcaacnnnnnnnnnnnnnnnnnnnnuuuuauuuu

SEQ ID NO: 217 - RNA, 183 nt, Artificial Sequence
  sgRNA(mature form, 7nt deletion in the first region)
gauaaaguggagaaccgcuucaccaaaagcugucccuuaggggauuagaacuugagugaaggugggcugcuugcaucagccuaaugucgagaagugcuuucuucggaaaguaacccucgaaacaaauucauuugaaagaaugaaggaaugcaacnnnnnnnnnnnnnnnnnnnnuuuuauuuu

SEQ ID NO: 218 - RNA, 182 nt, Artificial Sequence
  sgRNA(mature form, 8nt deletion in the first region)
auaaaguggagaaccgcuucaccaaaagcugucccuuaggggauuagaacuugagugaaggugggcugcuugcaucagccuaaugucgagaagugcuuucuucggaaaguaacccucgaaacaaauucauuugaaagaaugaaggaaugcaacnnnnnnnnnnnnnnnnnnnnuuuuauuuu

SEQ ID NO: 219 - RNA, 181 nt, Artificial Sequence
  sgRNA(mature form, 9nt deletion in the first region)
uaaaguggagaaccgcuucaccaaaagcugucccuuaggggauuagaacuugagugaaggugggcugcuugcaucagccuaaugucgagaagugcuuucuucggaaaguaacccucgaaacaaauucauuugaaagaaugaaggaaugcaacnnnnnnnnnnnnnnnnnnnnuuuuauuuu

SEQ ID NO: 220 - RNA, 180 nt, Artificial Sequence
  sgRNA(mature form, 10nt deletion in the first region)
aaaguggagaaccgcuucaccaaaagcugucccuuaggggauuagaacuugagugaaggugggcugcuugcaucagccuaaugucgagaagugcuuucuucggaaaguaacccucgaaacaaauucauuugaaagaaugaaggaaugcaacnnnnnnnnnnnnnnnnnnnnuuuuauuuu

SEQ ID NO: 221 - RNA, 179 nt, Artificial Sequence
  sgRNA(mature form, 11nt deletion in the first region)
aaguggagaaccgcuucaccaaaagcugucccuuaggggauuagaacuugagugaaggugggcugcuugcaucagccuaaugucgagaagugcuuucuucggaaaguaacccucgaaacaaauucauuugaaagaaugaaggaaugcaacnnnnnnnnnnnnnnnnnnnnuuuuauuuu

SEQ ID NO: 222 - RNA, 178 nt, Artificial Sequence
  sgRNA(mature form, 12nt deletion in the first region)
aguggagaaccgcuucaccaaaagcugucccuuaggggauuagaacuugagugaaggugggcugcuugcaucagccuaaugucgagaagugcuuucuucggaaaguaacccucgaaacaaauucauuugaaagaaugaaggaaugcaacnnnnnnnnnnnnnnnnnnnnuuuuauuuu

SEQ ID NO: 223 - RNA, 177 nt, Artificial Sequence
  sgRNA(mature form, 13nt deletion in the first region)
guggagaaccgcuucaccaaaagcugucccuuaggggauuagaacuugagugaaggugggcugcuugcaucagccuaaugucgagaagugcuuucuucggaaaguaacccucgaaacaaauucauuugaaagaaugaaggaaugcaacnnnnnnnnnnnnnnnnnnnnuuuuauuuu

SEQ ID NO: 224 - RNA, 176 nt, Artificial Sequence
  sgRNA(mature form, 14nt deletion in the first region)
uggagaaccgcuucaccaaaagcugucccuuaggggauuagaacuugagugaaggugggcugcuugcaucagccuaaugucgagaagugcuuucuucggaaaguaacccucgaaacaaauucauuugaaagaaugaaggaaugcaacnnnnnnnnnnnnnnnnnnnnuuuuauuuu

SEQ ID NO: 225 - RNA, 175 nt, Artificial Sequence
  sgRNA(mature form, 15nt deletion in the first region)
ggagaaccgcuucaccaaaagcugucccuuaggggauuagaacuugagugaaggugggcugcuugcaucagccuaaugucgagaagugcuuucuucggaaaguaacccucgaaacaaauucauuugaaagaaugaaggaaugcaacnnnnnnnnnnnnnnnnnnnnuuuuauuuu

SEQ ID NO: 226 - RNA, 174 nt, Artificial Sequence
  sgRNA(mature form, 16nt deletion in the first region)
gagaaccgcuucaccaaaagcugucccuuaggggauuagaacuugagugaaggugggcugcuugcaucagccuaaugucgagaagugcuuucuucggaaaguaacccucgaaacaaauucauuugaaagaaugaaggaaugcaacnnnnnnnnnnnnnnnnnnnnuuuuauuuu

SEQ ID NO: 227 - RNA, 173 nt, Artificial Sequence
  sgRNA(mature form, 17nt deletion in the first region)
agaaccgcuucaccaaaagcugucccuuaggggauuagaacuugagugaaggugggcugcuugcaucagccuaaugucgagaagugcuuucuucggaaaguaacccucgaaacaaauucauuugaaagaaugaaggaaugcaacnnnnnnnnnnnnnnnnnnnnuuuuauuuu

SEQ ID NO: 228 - RNA, 172 nt, Artificial Sequence
  sgRNA(mature form, 18nt deletion in the first region)
gaaccgcuucaccaaaagcugucccuuaggggauuagaacuugagugaaggugggcugcuugcaucagccuaaugucgagaagugcuuucuucggaaaguaacccucgaaacaaauucauuugaaagaaugaaggaaugcaacnnnnnnnnnnnnnnnnnnnnuuuuauuuu

SEQ ID NO: 229 - RNA, 171 nt, Artificial Sequence
  sgRNA(mature form, 19nt deletion in the first region)
aaccgcuucaccaaaagcugucccuuaggggauuagaacuugagugaaggugggcugcuugcaucagccuaaugucgagaagugcuuucuucggaaaguaacccucgaaacaaauucauuugaaagaaugaaggaaugcaacnnnnnnnnnnnnnnnnnnnnuuuuauuuu

SEQ ID NO: 230 - RNA, 170 nt, Artificial Sequence
  sgRNA(mature form, 20nt deletion in the first region)
accgcuucaccaaaagcugucccuuaggggauuagaacuugagugaaggugggcugcuugcaucagccuaaugucgagaagugcuuucuucggaaaguaacccucgaaacaaauucauuugaaagaaugaaggaaugcaacnnnnnnnnnnnnnnnnnnnnuuuuauuuu

SEQ ID NO: 231 - RNA, 188 nt, Artificial Sequence
  sgRNA(mature form, 1bp deletion in the second region)
cuucacugauaaaguggagaaccgcuucaccaaaagcuguccuuagggauuagaacuugagugaaggugggcugcuugcaucagccuaaugucgagaagugcuuucuucggaaaguaacccucgaaacaaauucauuugaaagaaugaaggaaugcaacnnnnnnnnnnnnnnnnnnnnuuuuauuuu

SEQ ID NO: 232 - RNA, 186 nt, Artificial Sequence
  sgRNA(mature form, 2bp deletion in the second region)
cuucacugauaaaguggagaaccgcuucaccaaaagcugucuuaggauuagaacuugagugaaggugggcugcuugcaucagccuaaugucgagaagugcuuucuucggaaaguaacccucgaaacaaauucauuugaaagaaugaaggaaugcaacnnnnnnnnnnnnnnnnnnnnuuuuauuuu

SEQ ID NO: 233 - RNA, 184 nt, Artificial Sequence
  sgRNA(mature form, 3bp deletion in the second region)
cuucacugauaaaguggagaaccgcuucaccaaaagcuguuuagauuagaacuugagugaaggugggcugcuugcaucagccuaaugucgagaagugcuuucuucggaaaguaacccucgaaacaaauucauuugaaagaaugaaggaaugcaacnnnnnnnnnnnnnnnnnnnnuuuuauuuu

SEQ ID NO: 234 - RNA, 182 nt, Artificial Sequence
  sgRNA(mature form, 4bp+1nt deletion in the second region)
cuucacugauaaaguggagaaccgcuucaccaaaagcuguuaguuagaacuugagugaaggugggcugcuugcaucagccuaaugucgagaagugcuuucuucggaaaguaacccucgaaacaaauucauuugaaagaaugaaggaaugcaacnnnnnnnnnnnnnnnnnnnnuuuuauuuu

SEQ ID NO: 235 - RNA, 181 nt, Artificial Sequence
  sgRNA(mature form, 4bp deletion in the second region)
cuucacugauaaaguggagaaccgcuucaccaaaagcuguuaguagaacuugagugaaggugggcugcuugcaucagccuaaugucgagaagugcuuucuucggaaaguaacccucgaaacaaauucauuugaaagaaugaaggaaugcaacnnnnnnnnnnnnnnnnnnnnuuuuauuuu

SEQ ID NO: 236 - RNA, 179 nt, Artificial Sequence
  sgRNA(mature form, 5bp deletion in the second region)
cuucacugauaaaguggagaaccgcuucaccaaaagcuuuagagaacuugagugaaggugggcugcuugcaucagccuaaugucgagaagugcuuucuucggaaaguaacccucgaaacaaauucauuugaaagaaugaaggaaugcaacnnnnnnnnnnnnnnnnnnnnuuuuauuuu

SEQ ID NO: 237 - RNA, 177 nt, Artificial Sequence
  sgRNA(mature form, 6bp deletion in the second region)
cuucacugauaaaguggagaaccgcuucaccaaaagcuuaggaacuugagugaaggugggcugcuugcaucagccuaaugucgagaagugcuuucuucggaaaguaacccucgaaacaaauucauuugaaagaaugaaggaaugcaacnnnnnnnnnnnnnnnnnnnnuuuuauuuu

SEQ ID NO: 238 - RNA, 175 nt, Artificial Sequence
  sgRNA(mature form, 7bp deletion in the second region)
cuucacugauaaaguggagaaccgcuucaccaaaaguuagaacuugagugaaggugggcugcuugcaucagccuaaugucgagaagugcuuucuucggaaaguaacccucgaaacaaauucauuugaaagaaugaaggaaugcaacnnnnnnnnnnnnnnnnnnnnuuuuauuuu

SEQ ID NO: 239 - RNA, 173 nt, Artificial Sequence
  sgRNA(mature form, 8bp deletion in the second region)
cuucacugauaaaguggagaaccgcuucaccaaaauuagacuugagugaaggugggcugcuugcaucagccuaaugucgagaagugcuuucuucggaaaguaacccucgaaacaaauucauuugaaagaaugaaggaaugcaacnnnnnnnnnnnnnnnnnnnnuuuuauuuu

SEQ ID NO: 240 - RNA, 171 nt, Artificial Sequence
  sgRNA(mature form, 9bp deletion in the second region)
cuucacugauaaaguggagaaccgcuucaccaaauuagcuugagugaaggugggcugcuugcaucagccuaaugucgagaagugcuuucuucggaaaguaacccucgaaacaaauucauuugaaagaaugaaggaaugcaacnnnnnnnnnnnnnnnnnnnnuuuuauuuu

SEQ ID NO: 241 - RNA, 169 nt, Artificial Sequence
  sgRNA(mature form, 10bp deletion in the second region)
cuucacugauaaaguggagaaccgcuucaccaauuaguugagugaaggugggcugcuugcaucagccuaaugucgagaagugcuuucuucggaaaguaacccucgaaacaaauucauuugaaagaaugaaggaaugcaacnnnnnnnnnnnnnnnnnnnnuuuuauuuu

SEQ ID NO: 242 - RNA, 167 nt, Artificial Sequence
  sgRNA(mature form, 11bp deletion in the second region)
cuucacugauaaaguggagaaccgcuucaccauuagugagugaaggugggcugcuugcaucagccuaaugucgagaagugcuuucuucggaaaguaacccucgaaacaaauucauuugaaagaaugaaggaaugcaacnnnnnnnnnnnnnnnnnnnnuuuuauuuu

SEQ ID NO: 243 - RNA, 188 nt, Artificial Sequence
  sgRNA(mature form, 1bp deletion in the fourth and fifth region)
cuucacugauaaaguggagaaccgcuucaccaaaagcugucccuuaggggauuagaacuugagugaaggugggcugcuugcaucagccuaaugucgagaagugcuuucuucggaaaguaacccucgaaacaaauucauugaaaaaugaaggaaugcaacnnnnnnnnnnnnnnnnnnnnuuuuauuuu

SEQ ID NO: 244 - RNA, 186 nt, Artificial Sequence
  sgRNA(mature form, 2bp deletion in the fourth and fifth region)
cuucacugauaaaguggagaaccgcuucaccaaaagcugucccuuaggggauuagaacuugagugaaggugggcugcuugcaucagccuaaugucgagaagugcuuucuucggaaaguaacccucgaaacaaauucaugaaaaugaaggaaugcaacnnnnnnnnnnnnnnnnnnnnuuuuauuuu

SEQ ID NO: 245 - RNA, 184 nt, Artificial Sequence
  sgRNA(mature form, 3bp deletion in the fourth and fifth region)
cuucacugauaaaguggagaaccgcuucaccaaaagcugucccuuaggggauuagaacuugagugaaggugggcugcuugcaucagccuaaugucgagaagugcuuucuucggaaaguaacccucgaaacaaauucagaaaugaaggaaugcaacnnnnnnnnnnnnnnnnnnnnuuuuauuuu

SEQ ID NO: 246 - RNA, 182 nt, Artificial Sequence
  sgRNA(mature form, 4bp deletion in the fourth and fifth region)
cuucacugauaaaguggagaaccgcuucaccaaaagcugucccuuaggggauuagaacuugagugaaggugggcugcuugcaucagccuaaugucgagaagugcuuucuucggaaaguaacccucgaaacaaauucgaaagaaggaaugcaacnnnnnnnnnnnnnnnnnnnnuuuuauuuu

SEQ ID NO: 247 - RNA, 180 nt, Artificial Sequence
  sgRNA(mature form, 5bp deletion in the fourth and fifth region)
cuucacugauaaaguggagaaccgcuucaccaaaagcugucccuuaggggauuagaacuugagugaaggugggcugcuugcaucagccuaaugucgagaagugcuuucuucggaaaguaacccucgaaacaaauugaaaaaggaaugcaacnnnnnnnnnnnnnnnnnnnnuuuuauuuu

SEQ ID NO: 248 - RNA, 178 nt, Artificial Sequence
  sgRNA(mature form, 6bp deletion in the fourth and fifth region)
cuucacugauaaaguggagaaccgcuucaccaaaagcugucccuuaggggauuagaacuugagugaaggugggcugcuugcaucagccuaaugucgagaagugcuuucuucggaaaguaacccucgaaacaaaugaaaaggaaugcaacnnnnnnnnnnnnnnnnnnnnuuuuauuuu

SEQ ID NO: 249 - RNA, 176 nt, Artificial Sequence
  sgRNA(mature form, 7bp deletion in the fourth and fifth region)
cuucacugauaaaguggagaaccgcuucaccaaaagcugucccuuaggggauuagaacuugagugaaggugggcugcuugcaucagccuaaugucgagaagugcuuucuucggaaaguaacccucgaaacaaagaaaggaaugcaacnnnnnnnnnnnnnnnnnnnnuuuuauuuu

SEQ ID NO: 250 - RNA, 147 nt, Artificial Sequence
  sgRNA(mature form, modified first and second region)
accgcuucaccauuagugagugaaggugggcugcuugcaucagccuaaugucgagaagugcuuucuucggaaaguaacccucgaaacaaauucauuugaaagaaugaaggaaugcaacnnnnnnnnnnnnnnnnnnnnuuuuauuuu

SEQ ID NO: 251 - RNA, 156 nt, Artificial Sequence
  sgRNA(mature form, modified first, fourth and fifth region)
accgcuucaccaaaagcugucccuuaggggauuagaacuugagugaaggugggcugcuugcaucagccuaaugucgagaagugcuuucuucggaaaguaacccucgaaacaaagaaaggaaugcaacnnnnnnnnnnnnnnnnnnnnuuuuauuuu

SEQ ID NO: 252 - RNA, 153 nt, Artificial Sequence
  sgRNA(mature form, modified second, fourth and fifth region)
cuucacugauaaaguggagaaccgcuucaccauuagugagugaaggugggcugcuugcaucagccuaaugucgagaagugcuuucuucggaaaguaacccucgaaacaaagaaaggaaugcaacnnnnnnnnnnnnnnnnnnnnuuuuauuuu

SEQ ID NO: 253 - RNA, 130 nt, Artificial Sequence
  sgRNA(mature form, modified first, second, fourth and fifth region)
accgcuucacuuagagugaagguggggcugcuugcaucagccuaaugucgagaagugcuuucuucggaaaguaacccucgaaacaaagaaaggaaugcaacnnnnnnnnnnnnnnnnnnnnuuuuauuuu

SEQ ID NO: 254 - RNA, 11 nt, Artificial Sequence
  U-rich tail sequence
uuuauuuauuu

SEQ ID NO: 255 - RNA, 10 nt, Artificial Sequence
  U-rich tail sequence
uuuuauuuuu

SEQ ID NO: 256 - RNA, 11 nt, Artificial Sequence
  U-rich tail sequence
uuuuauuuuuu

SEQ ID NO: 257 - RNA, 11 nt, Artificial Sequence
  U-rich tail sequence
uuuguuuguuu

SEQ ID NO: 258 - RNA, 10 nt, Artificial Sequence
  U-rich tail sequence
uuuuguuuuu

SEQ ID NO: 259 - RNA, 11 nt, Artificial Sequence
  U-rich tail sequence
uuuuguuuuuu

SEQ ID NO: 260 - protein, 529 aa, Artificial Sequence
  Cas14a1 amino acid sequence
MAKNTITKTLKLRIVRPYNSAEVEKIVADEKNNREKIALEKNKDKVKEACSKHLKVAAYCTTQVERNACLFCKARKLDDKFYQKLRGQFPDAVFWQEISEIFRQLQKQAAEIYNQSLIELYYEIFIKGKGIANASSVEHYLSDVCYTRAAELFKNAAIASGLRSKIKSNFRLKELKNMKSGLPTTKSDNFPIPLVKQKGGQYTGFEISNHNSDFIIKIPFGRWQVKKEIDKYRPWEKFDFEQVQKSPKPISLLLSTQRRKRNKGWSKDEGTEAEIKKVMNGDYQTSYIEVKRGSKIGEKSAWMLNLSIDVPKIDKGVDPSIIGGIDVGVKSPLVCAINNAFSRYSISDNDLFHFNKKMFARRRILLKKNRHKRAGHGAKNKLKPITILTEKSERFRKKLIERWACEIADFFIKNKVGTVQMENLESMKRKEDSYFNIRLRGFWPYAEMQNKIEFKLKQYGIEIRKVAPNNTSKTCSKCGHLNNYFNFEYRKKNKFPHFKCEKCNFKENADYNAALNISNPKLKSTKEEP

SEQ ID NO: 261 - protein, 536 aa, Artificial Sequence
  N-terminal NLS + Cas14a1 amino acid sequence
MPKKKRKVAKNTITKTLKLRIVRPYNSAEVEKIVADEKNNREKIALEKNKDKVKEACSKHLKVAAYCTTQVERNACLFCKARKLDDKFYQKLRGQFPDAVFWQEISEIFRQLQKQAAEIYNQSLIELYYEIFIKGKGIANASSVEHYLSDVCYTRAAELFKNAAIASGLRSKIKSNFRLKELKNMKSGLPTTKSDNFPIPLVKQKGGQYTGFEISNHNSDFIIKIPFGRWQVKKEIDKYRPWEKFDFEQVQKSPKPISLLLSTQRRKRNKGWSKDEGTEAEIKKVMNGDYQTSYIEVKRGSKIGEKSAWMLNLSIDVPKIDKGVDPSIIGGIDVGVKSPLVCAINNAFSRYSISDNDLFHFNKKMFARRRILLKKNRHKRAGHGAKNKLKPITILTEKSERFRKKLIERWACEIADFFIKNKVGTVQMENLESMKRKEDSYFNIRLRGFWPYAEMQNKIEFKLKQYGIEIRKVAPNNTSKTCSKCGHLNNYFNFEYRKKNKFPHFKCEKCNFKENADYNAALNISNPKLKSTKEEP

SEQ ID NO: 262 - protein, 536 aa, Artificial Sequence
  C-terminal NLS + Cas14a1 amino acid sequence
MAKNTITKTLKLRIVRPYNSAEVEKIVADEKNNREKIALEKNKDKVKEACSKHLKVAAYCTTQVERNACLFCKARKLDDKFYQKLRGQFPDAVFWQEISEIFRQLQKQAAEIYNQSLIELYYEIFIKGKGIANASSVEHYLSDVCYTRAAELFKNAAIASGLRSKIKSNFRLKELKNMKSGLPTTKSDNFPIPLVKQKGGQYTGFEISNHNSDFIIKIPFGRWQVKKEIDKYRPWEKFDFEQVQKSPKPISLLLSTQRRKRNKGWSKDEGTEAEIKKVMNGDYQTSYIEVKRGSKIGEKSAWMLNLSIDVPKIDKGVDPSIIGGIDVGVKSPLVCAINNAFSRYSISDNDLFHFNKKMFARRRILLKKNRHKRAGHGAKNKLKPITILTEKSERFRKKLIERWACEIADFFIKNKVGTVQMENLESMKRKEDSYFNIRLRGFWPYAEMQNKIEFKLKQYGIEIRKVAPNNTSKTCSKCGHLNNYFNFEYRKKNKFPHFKCEKCNFKENADYNAALNISNPKLKSTKEEPPKKKRKV

SEQ ID NO: 263 - protein, 536 aa, Artificial Sequence; identical to SEQ ID NO: 262
  N/C-terminal NLS + Cas14a1 amino acid sequence

SEQ ID NO: 264 - protein, 1004 aa, Artificial Sequence
  Amino acid sequence (N terminal -Cytidine deaminase)
MPKKKRKVSSETGPVAVDPTLRRRIEPHEFEVFFDPRELRKETCLLYEINWGGRHSIWRHTSQNTNKHVEVNFIEKFTTERYFCPNTRCSITWFLSWSPCGECSRAITEFLSRYPHVTLFIYIARLYHHADPRNRQGLRDLISSGVTIQIMTEQESGYCWRNFVNYSPSNEAHWPRYPHLWVRLYVLELYCIILGLPPCLNILRRKQPQLTFFTIALQSCHYQRLPPHILWATGLKSGGSSGGSSGSETPGTSESATPESSGGSSGGSMAKNTITKTLKLRIVRPYNSAEVEKIVADEKNNREKIALEKNKDKVKEACSKHLKVAAYCTTQVERNACLFCKARKLDDKFYQKLRGQFPDAVFWQEISEIFRQLQKQAAEIYNQSLIELYYEIFIKGKGIANASSVEHYLSDVCYTRAAELFKNAAIASGLRSKIKSNFRLKELKNMKSGLPTTKSDNFPIPLVKQKGGQYTGFEISNHNSDFIIKIPFGRWQVKKEIDKYRPWEKFDFEQVQKSPKPISLLLSTQRRKRNKGWSKDEGTEAEIKKVMNGDYQTSYIEVKRGSKIGEKSAWMLNLSIDVPKIDKGVDPSIIGGIDVGVKSPLVCAINNAFSRYSISDNDLFHFNKKMFARRRILLKKNRHKRAGHGAKNKLKPITILTEKSERFRKKLIERWACEIADFFIKNKVGTVQMENLESMKRKEDSYFNIRLRGFWPYAEMQNKIEFKLKQYGIEIRKVAPNNTSKTCSKCGHLNNYFNFEYRKKNKFPHFKCEKCNFKENADYNAALNISNPKLKSTKEEPSGGSGGSGGSTNLSDIIEKETGKQLVIQESILMLPEEVEEVIGNKPESDILVHTAYDESTDENVMLLTSDAPEYKPWALVIQDSNGENKIKMLSGGSGGSGGSTNLSDIIEKETGKQLVIQESILMLPEEVEEVIGNKPESDILVHTAYDESTDENVMLLTSDAPEYKPWALVIQDSNGENKIKMLSGGSKRTADGSEFEPKKKRKV

SEQ ID NO: 265 - protein, 1003 aa, Artificial Sequence
  Amino acid sequence (C terminal -Cytidine deaminase)
MPKKKRKVAKNTITKTLKLRIVRPYNSAEVEKIVADEKNNREKIALEKNKDKVKEACSKHLKVAAYCTTQVERNACLFCKARKLDDKFYQKLRGQFPDAVFWQEISEIFRQLQKQAAEIYNQSLIELYYEIFIKGKGIANASSVEHYLSDVCYTRAAELFKNAAIASGLRSKIKSNFRLKELKNMKSGLPTTKSDNFPIPLVKQKGGQYTGFEISNHNSDFIIKIPFGRWQVKKEIDKYRPWEKFDFEQVQKSPKPISLLLSTQRRKRNKGWSKDEGTEAEIKKVMNGDYQTSYIEVKRGSKIGEKSAWMLNLSIDVPKIDKGVDPSIIGGIDVGVKSPLVCAINNAFSRYSISDNDLFHFNKKMFARRRILLKKNRHKRAGHGAKNKLKPITILTEKSERFRKKLIERWACEIADFFIKNKVGTVQMENLESMKRKEDSYFNIRLRGFWPYAEMQNKIEFKLKQYGIEIRKVAPNNTSKTCSKCGHLNNYFNFEYRKKNKFPHFKCEKCNFKENADYNAALNISNPKLKSTKEEPSGGSSGGSSGSETPGTSESATPESSGGSSGGSSSETGPVAVDPTLRRRIEPHEFEVFFDPRELRKETCLLYEINWGGRHSIWRHTSQNTNKHVEVNFIEKFTTERYFCPNTRCSITWFLSWSPCGECSRAITEFLSRYPHVTLFIYIARLYHHADPRNRQGLRDLISSGVTIQIMTEQESGYCWRNFVNYSPSNEAHWPRYPHLWVRLYVLELYCIILGLPPCLNILRRKQPQLTFFTIALQSCHYQRLPPHILWATGLKSGGSGGSGGSTNLSDIIEKETGKQLVIQESILMLPEEVEEVIGNKPESDILVHTAYDESTDENVMLLTSDAPEYKPWALVIQDSNGENKIKMLSGGSGGSGGSTNLSDIIEKETGKQLVIQESILMLPEEVEEVIGNKPESDILVHTAYDESTDENVMLLTSDAPEYKPWALVIQDSNGENKIKMLSGGSKRTADGSEFEPKKKRKV

SEQ ID NO: 266 - protein, 941 aa, Artificial Sequence
  DNA sequence (N terminal -Adenine deaminase)
MSEVEFSHEYWMRHALTLAKRAWDEREVPVGAVLVHNNRVIGEGWNRPIGRHDPTAHAEIMALRQGGLVMQNYRLIDATLYVTLEPCVMCAGAMIHSRIGRVVFGARDAKTGAAGSLMDVLHHPGMNHRVEITEGILADECAALLSDFFRMRRQEIKAQKKAQSSTDSGGSSGGSSGSETPGTSESATPESSGGSSGGSSEVEFSHEYWMRHALTLAKRARDEREVPVGAVLVLNNRVIGEGWNRAIGLHDPTAHAEIMALRQGGLVMQNYRLIDATLYVTFEPCVMCAGAMIHSRIGRVVFGVRNAKTGAAGSLMDVLHYPGMNHRVEITEGILADECAALLCYFFRMPRQVFNAQKKAQSSTDSGGSSGGSSGSETPGTSESATPESSGGSSGGSAKNTITKTLKLRIVRPYNSAEVEKIVADEKNNREKIALEKNKDKVKEACSKHLKVAAYCTTQVERNACLFCKARKLDDKFYQKLRGQFPDAVFWQEISEIFRQLQKQAAEIYNQSLIELYYEIFIKGKGIANASSVEHYLSDVCYTRAAELFKNAAIASGLRSKIKSNFRLKELKNMKSGLPTTKSDNFPIPLVKQKGGQYTGFEISNHNSDFIIKIPFGRWQVKKEIDKYRPWEKFDFEQVQKSPKPISLLLSTQRRKRNKGWSKDEGTEAEIKKVMNGDYQTSYIEVKRGSKIGEKSAWMLNLSIDVPKIDKGVDPSIIGGIDVGVKSPLVCAINNAFSRYSISDNDLFHFNKKMFARRRILLKKNRHKRAGHGAKNKLKPITILTEKSERFRKKLIERWACEIADFFIKNKVGTVQMENLESMKRKEDSYFNIRLRGFWPYAEMQNKIEFKLKQYGIEIRKVAPNNTSKTCSKCGHLNNYFNFEYRKKNKFPHFKCEKCNFKENADYNAALNISNPKLKSTKEEPKRPAATKKAGQAKKKK

SEQ ID NO: 267 - protein, 941 aa, Artificial Sequence
  DNA sequence (C terminal -Adenine deaminase)
MAKNTITKTLKLRIVRPYNSAEVEKIVADEKNNREKIALEKNKDKVKEACSKHLKVAAYCTTQVERNACLFCKARKLDDKFYQKLRGQFPDAVFWQEISEIFRQLQKQAAEIYNQSLIELYYEIFIKGKGIANASSVEHYLSDVCYTRAAELFKNAAIASGLRSKIKSNFRLKELKNMKSGLPTTKSDNFPIPLVKQKGGQYTGFEISNHNSDFIIKIPFGRWQVKKEIDKYRPWEKFDFEQVQKSPKPISLLLSTQRRKRNKGWSKDEGTEAEIKKVMNGDYQTSYIEVKRGSKIGEKSAWMLNLSIDVPKIDKGVDPSIIGGIDVGVKSPLVCAINNAFSRYSISDNDLFHFNKKMFARRRILLKKNRHKRAGHGAKNKLKPITILTEKSERFRKKLIERWACEIADFFIKNKVGTVQMENLESMKRKEDSYFNIRLRGFWPYAEMQNKIEFKLKQYGIEIRKVAPNNTSKTCSKCGHLNNYFNFEYRKKNKFPHFKCEKCNFKENADYNAALNISNPKLKSTKEEPSGGSSGGSSGSETPGTSESATPESSGGSSGGSSEVEFSHEYWMRHALTLAKRAWDEREVPVGAVLVHNNRVIGEGWNRPIGRHDPTAHAEIMALRQGGLVMQNYRLIDATLYVTLEPCVMCAGAMIHSRIGRVVFGARDAKTGAAGSLMDVLHHPGMNHRVEITEGILADECAALLSDFFRMRRQEIKAQKKAQSSTDSGGSSGGSSGSETPGTSESATPESSGGSSGGSSEVEFSHEYWMRHALTLAKRARDEREVPVGAVLVLNNRVIGEGWNRAIGLHDPTAHAEIMALRQGGLVMQNYRLIDATLYVTFEPCVMCAGAMIHSRIGRVVFGVRNAKTGAAGSLMDVLHYPGMNHRVEITEGILADECAALLCYFFRMPRQVFNAQKKAQSSTDKRPAATKKAGQAKKKK

SEQ ID NO: 268 - DNA, 1680 bp, Artificial Sequence
  Human codon-optimized Cas14a1 with NLS
atgccaaagaagaagcggaaggtcggtatccacggagtcccagcagccgccaagaacacaattacaaagacactgaagctgaggatcgtgagaccatacaacagcgctgaggtcgagaagattgtggctgatgaaaagaacaacagggaaaagatcgccctcgagaagaacaaggataaggtgaaggaggcctgctctaagcacctgaaagtggccgcctactgcaccacacaggtggagaggaacgcctgtctgttttgtaaagctcggaagctggatgataagttttaccagaagctgcggggccagttccccgatgccgtcttttggcaggagattagcgagatcttcagacagctgcagaagcaggccgccgagatctacaaccagagcctgatcgagctctactacgagatcttcatcaagggcaagggcattgccaacgcctcctccgtggagcactacctgagcgacgtgtgctacacaagagccgccgagctctttaagaacgccgctatcgcttccgggctgaggagcaagattaagagtaacttccggctcaaggagctgaagaacatgaagagcggcctgcccactacaaagagcgacaacttcccaattccactggtgaagcagaaggggggccagtacacagggttcgagatttccaaccacaacagcgactttattattaagatcccctttggcaggtggcaggtcaagaaggagattgacaagtacaggccctgggagaagtttgatttcgagcaggtgcagaagagccccaagcctatttccctgctgctgtccacacagcggcggaagaggaacaaggggtggtctaaggatgaggggaccgaggccgagattaagaaagtgatgaacggcgactaccagacaagctacatcgaggtcaagcggggcagtaagattggcgagaagagcgcctggatgctgaacctgagcattgacgtgccaaagattgataagggcgtggatcccagcatcatcggagggatcgatgtgggggtcaagagccccctcgtgtgcgccatcaacaacgccttcagcaggtacagcatctccgataacgacctgttccactttaacaagaagatgttcgcccggcggaggattttgctcaagaagaaccggcacaagcgggccggacacggggccaagaacaagctcaagcccatcactatcctgaccgagaagagcgagaggttcaggaagaagctcatcgagagatgggcctgcgagatcgccgatttctttattaagaacaaggtcggaacagtgcagatggagaacctcgagagcatgaagaggaaggaggattcctacttcaacattcggctgagggggttctggccctacgctgagatgcagaacaagattgagtttaagctgaagcagtacgggattgagatccggaaggtggcccccaacaacaccagcaagacctgcagcaagtgcgggcacctcaacaactacttcaacttcgagtaccggaagaagaacaagttcccacacttcaagtgcgagaagtgcaactttaaggagaacgccgattacaacgccgccctgaacatcagcaaccctaagctgaagagcactaaggaggagcccaaaaggccggcggccacgaaaaaggccggccaggcaaaaaagaaaaag

SEQ ID NO: 269 - DNA, 3009 bp, Artificial Sequence
  Deaminase fusion Cas14a1
atgccaaagaagaagcggaaagtctcctcagagactgggcctgtcgccgtcgatccaaccctgcgccgccggattgaacctcacgagtttgaagtgttctttgacccccgggagctgagaaaggagacatgcctgctgtacgagatcaactggggaggcaggcactccatctggaggcacacctctcagaacacaaataagcacgtggaggtgaacttcatcgagaagtttaccacagagcggtacttctgccccaataccagatgtagcatcacatggtttctgagctggtccccttgcggagagtgtagcagggccatcaccgagttcctgtccagatatccacacgtgacactgtttatctacatcgccaggctgtatcaccacgcagacccaaggaataggcagggcctgcgcgatctgatcagctccggcgtgaccatccagatcatgacagagcaggagtccggctactgctggcggaacttcgtgaattattctcctagcaacgaggcccactggcctaggtacccacacctgtgggtgcgcctgtacgtgctggagctgtattgcatcatcctgggcctgcccccttgtctgaatatcctgcggagaaagcagccccagctgaccttctttacaatcgccctgcagtcttgtcactatcagaggctgccaccccacatcctgtgggccacaggcctgaagtctggaggatctagcggaggatcctctggcagcgagacaccaggaacaagcgagtcagcaacaccagagagcagtggcggcagcagcggcggcagcgccaagaacacaattacaaagacactgaagctgaggatcgtgagaccatacaacagcgctgaggtcgagaagattgtggctgatgaaaagaacaacagggaaaagatcgccctcgagaagaacaaggataaggtgaaggaggcctgctctaagcacctgaaagtggccgcctactgcaccacacaggtggagaggaacgcctgtctgttttgtaaagctcggaagctggatgataagttttaccagaagctgcggggccagttccccgatgccgtcttttggcaggagattagcgagatcttcagacagctgcagaagcaggccgccgagatctacaaccagagcctgatcgagctctactacgagatcttcatcaagggcaagggcattgccaacgcctcctccgtggagcactacctgagcgacgtgtgctacacaagagccgccgagctctttaagaacgccgctatcgcttccgggctgaggagcaagattaagagtaacttccggctcaaggagctgaagaacatgaagagcggcctgcccactacaaagagcgacaacttcccaattccactggtgaagcagaaggggggccagtacacagggttcgagatttccaaccacaacagcgactttattattaagatcccctttggcaggtggcaggtcaagaaggagattgacaagtacaggccctgggagaagtttgatttcgagcaggtgcagaagagccccaagcctatttccctgctgctgtccacacagcggcggaagaggaacaaggggtggtctaaggatgaggggaccgaggccgagattaagaaagtgatgaacggcgactaccagacaagctacatcgaggtcaagcggggcagtaagattggcgagaagagcgcctggatgctgaacctgagcattgacgtgccaaagattgataagggcgtggatcccagcatcatcggagggatcgatgtgggggtcaagagccccctcgtgtgcgccatcaacaacgccttcagcaggtacagcatctccgataacgacctgttccactttaacaagaagatgttcgcccggcggaggattttgctcaagaagaaccggcacaagcgggccggacacggggccaagaacaagctcaagcccatcactatcctgaccgagaagagcgagaggttcaggaagaagctcatcgagagatgggcctgcgagatcgccgatttctttattaagaacaaggtcggaacagtgcagatggagaacctcgagagcatgaagaggaaggaggattcctacttcaacattcggctgagggggttctggccctacgctgagatgcagaacaagattgagtttaagctgaagcagtacgggattgagatccggaaggtggcccccaacaacaccagcaagacctgcagcaagtgcgggcacctcaacaactacttcaacttcgagtaccggaagaagaacaagttcccacacttcaagtgcgagaagtgcaactttaaggagaacgccgattacaacgccgccctgaacatcagcaaccctaagctgaagagcactaaggaggagcccagcggcgggagcggcgggagcggggggagcactaatctgagcgacatcattgagaaggagactgggaaacagctggtcattcaggagtccatcctgatgctgcctgaggaggtggaggaagtgatcggcaacaagccagagtctgacatcctggtgcacaccgcctacgacgagtccacagatgagaatgtgatgctgctgacctctgacgcccccgagtataagccttgggccctggtcatccaggattctaacggcgagaataagatcaagatgctgagcggaggatccggaggatctggaggcagcaccaacctgtctgacatcatcgagaaggagacaggcaagcagctggtcatccaggagagcatcctgatgctgcccgaagaagtcgaagaagtgatcggaaacaagcctgagagcgatatcctggtccataccgcctacgacgagagtaccgacgaaaatgtgatgctgctgacatccgacgccccagagtataagccctgggctctggtcatccaggattccaacggagagaacaaaatcaaaatgctgtctggcggctcaaaaagaaccgccgacggcagcgaattcgagcccaagaagaagaggaaagtc

SEQ ID NO: 270 - DNA, 1586 bp, Artificial Sequence
  human codon-optimized Cas14a1
atggccaagaacacaattacaaagacactgaagctgaggatcgtgagaccatacaacagcgctgaggtcgagaagattgtggctgatgaaaagaacaacagggaaaagatcgccctcgagaagaacaaggataaggtgaaggaggcctgctctaagcacctgaaagtggccgcctactgcaccacacaggtggagaggaacgcctgtctgttttgtaaagctcggaagctggatgataagttttaccagaagctgcggggccagttccccgatgccgtcttttggcaggagattagcgagatcttcagacagctgcagaagcaggccgccgagatctacaaccagagcctgatcgagctctactacgagatcttcatcaagggcaagggcattgccaacgcctcctccgtggagcactacctgagcgacgtgtgctacacaagagccgccgagctctttaagaacgccgctatcgcttccgggctgaggagcaagattaagagtaacttccggctcaaggagctgaagaacatgaagagcggcctgcccactacaaagagcgacaacttcccaattccactggtgaagcagaaggggggccagtacacagggttcgagatttccaaccacaacagcgactttattattaagatcccctttggcaggtggcaggtcaagaaggagattgacaagtacaggccctgggagaagtttgatttcgagcaggtgcagaagagccccaagcctatttccctgctgctgtccacacagcggcggaagaggaacaaggggtggtctaaggatgaggggaccgaggccgagattaagaaagtgatgaacggcgactaccagacaagctacatcgaggtcaagcggggcagtaagattggcgagaagagcgcctggatgctgaacctgagcattgacgtgccaaagattgataagggcgtggatcccagcatcatcggagggatcgatgtgggggtcaagagccccctcgtgtgcgccatcaacaacgccttcagcaggtacagcatctccgataacgacctgttccactttaacaagaagatgttcgcccggcggaggattttgctcaagaagaaccggcacaagcgggccggacacggggccaagaacaagctcaagcccatcactatcctgaccgagaagagcgagaggttcaggaagaagctcatcgagagatgggcctgcgagatcgccgatttctttattaagaacaaggtcggaacagtgcagatggagaacctcgagagcatgaagaggaaggaggattcctacttcaacattcggctgagggggttctggccctacgctgagatgcagaacaagattgagtttaagctgaagcagtacgggattgagatccggaaggtggcccccaacaacaccagcaagacctgcagcaagtgcgggcacctcaacaactacttcaacttcgagtaccggaagaagaacaagttcccacacttcaagtgcgagaagtgcaactttaaggagaacgccgattacaacgccgccctgaacatcagcaaccctaagctgaagagcactaaggaggagcc

SEQ ID NO: 271 - DNA, 1607 bp, Artificial Sequence
  N-terminal NLS + Cas14a1 amino acid sequence
atgccaaagaagaagcggaaagtcgccaagaacacaattacaaagacactgaagctgaggatcgtgagaccatacaacagcgctgaggtcgagaagattgtggctgatgaaaagaacaacagggaaaagatcgccctcgagaagaacaaggataaggtgaaggaggcctgctctaagcacctgaaagtggccgcctactgcaccacacaggtggagaggaacgcctgtctgttttgtaaagctcggaagctggatgataagttttaccagaagctgcggggccagttccccgatgccgtcttttggcaggagattagcgagatcttcagacagctgcagaagcaggccgccgagatctacaaccagagcctgatcgagctctactacgagatcttcatcaagggcaagggcattgccaacgcctcctccgtggagcactacctgagcgacgtgtgctacacaagagccgccgagctctttaagaacgccgctatcgcttccgggctgaggagcaagattaagagtaacttccggctcaaggagctgaagaacatgaagagcggcctgcccactacaaagagcgacaacttcccaattccactggtgaagcagaaggggggccagtacacagggttcgagatttccaaccacaacagcgactttattattaagatcccctttggcaggtggcaggtcaagaaggagattgacaagtacaggccctgggagaagtttgatttcgagcaggtgcagaagagccccaagcctatttccctgctgctgtccacacagcggcggaagaggaacaaggggtggtctaaggatgaggggaccgaggccgagattaagaaagtgatgaacggcgactaccagacaagctacatcgaggtcaagcggggcagtaagattggcgagaagagcgcctggatgctgaacctgagcattgacgtgccaaagattgataagggcgtggatcccagcatcatcggagggatcgatgtgggggtcaagagccccctcgtgtgcgccatcaacaacgccttcagcaggtacagcatctccgataacgacctgttccactttaacaagaagatgttcgcccggcggaggattttgctcaagaagaaccggcacaagcgggccggacacggggccaagaacaagctcaagcccatcactatcctgaccgagaagagcgagaggttcaggaagaagctcatcgagagatgggcctgcgagatcgccgatttctttattaagaacaaggtcggaacagtgcagatggagaacctcgagagcatgaagaggaaggaggattcctacttcaacattcggctgagggggttctggccctacgctgagatgcagaacaagattgagtttaagctgaagcagtacgggattgagatccggaaggtggcccccaacaacaccagcaagacctgcagcaagtgcgggcacctcaacaactacttcaacttcgagtaccggaagaagaacaagttcccacacttcaagtgcgagaagtgcaactttaaggagaacgccgattacaacgccgccctgaacatcagcaaccctaagctgaagagcactaaggaggagcc

SEQ ID NO: 272 - DNA, 1607 bp, Artificial Sequence
  C-terminal NLS + Cas14a1 amino acid sequence
atggccaagaacacaattacaaagacactgaagctgaggatcgtgagaccatacaacagcgctgaggtcgagaagattgtggctgatgaaaagaacaacagggaaaagatcgccctcgagaagaacaaggataaggtgaaggaggcctgctctaagcacctgaaagtggccgcctactgcaccacacaggtggagaggaacgcctgtctgttttgtaaagctcggaagctggatgataagttttaccagaagctgcggggccagttccccgatgccgtcttttggcaggagattagcgagatcttcagacagctgcagaagcaggccgccgagatctacaaccagagcctgatcgagctctactacgagatcttcatcaagggcaagggcattgccaacgcctcctccgtggagcactacctgagcgacgtgtgctacacaagagccgccgagctctttaagaacgccgctatcgcttccgggctgaggagcaagattaagagtaacttccggctcaaggagctgaagaacatgaagagcggcctgcccactacaaagagcgacaacttcccaattccactggtgaagcagaaggggggccagtacacagggttcgagatttccaaccacaacagcgactttattattaagatcccctttggcaggtggcaggtcaagaaggagattgacaagtacaggccctgggagaagtttgatttcgagcaggtgcagaagagccccaagcctatttccctgctgctgtccacacagcggcggaagaggaacaaggggtggtctaaggatgaggggaccgaggccgagattaagaaagtgatgaacggcgactaccagacaagctacatcgaggtcaagcggggcagtaagattggcgagaagagcgcctggatgctgaacctgagcattgacgtgccaaagattgataagggcgtggatcccagcatcatcggagggatcgatgtgggggtcaagagccccctcgtgtgcgccatcaacaacgccttcagcaggtacagcatctccgataacgacctgttccactttaacaagaagatgttcgcccggcggaggattttgctcaagaagaaccggcacaagcgggccggacacggggccaagaacaagctcaagcccatcactatcctgaccgagaagagcgagaggttcaggaagaagctcatcgagagatgggcctgcgagatcgccgatttctttattaagaacaaggtcggaacagtgcagatggagaacctcgagagcatgaagaggaaggaggattcctacttcaacattcggctgagggggttctggccctacgctgagatgcagaacaagattgagtttaagctgaagcagtacgggattgagatccggaaggtggcccccaacaacaccagcaagacctgcagcaagtgcgggcacctcaacaactacttcaacttcgagtaccggaagaagaacaagttcccacacttcaagtgcgagaagtgcaactttaaggagaacgccgattacaacgccgccctgaacatcagcaaccctaagctgaagagcactaaggaggagccccaaagaagaagcggaaagtc

SEQ ID NO: 273 - DNA, 1628 bp, Artificial Sequence
  N/C-terminal NLS + Cas14a1 amino acid sequence
atgccaaagaagaagcggaaagtcgccaagaacacaattacaaagacactgaagctgaggatcgtgagaccatacaacagcgctgaggtcgagaagattgtggctgatgaaaagaacaacagggaaaagatcgccctcgagaagaacaaggataaggtgaaggaggcctgctctaagcacctgaaagtggccgcctactgcaccacacaggtggagaggaacgcctgtctgttttgtaaagctcggaagctggatgataagttttaccagaagctgcggggccagttccccgatgccgtcttttggcaggagattagcgagatcttcagacagctgcagaagcaggccgccgagatctacaaccagagcctgatcgagctctactacgagatcttcatcaagggcaagggcattgccaacgcctcctccgtggagcactacctgagcgacgtgtgctacacaagagccgccgagctctttaagaacgccgctatcgcttccgggctgaggagcaagattaagagtaacttccggctcaaggagctgaagaacatgaagagcggcctgcccactacaaagagcgacaacttcccaattccactggtgaagcagaaggggggccagtacacagggttcgagatttccaaccacaacagcgactttattattaagatcccctttggcaggtggcaggtcaagaaggagattgacaagtacaggccctgggagaagtttgatttcgagcaggtgcagaagagccccaagcctatttccctgctgctgtccacacagcggcggaagaggaacaaggggtggtctaaggatgaggggaccgaggccgagattaagaaagtgatgaacggcgactaccagacaagctacatcgaggtcaagcggggcagtaagattggcgagaagagcgcctggatgctgaacctgagcattgacgtgccaaagattgataagggcgtggatcccagcatcatcggagggatcgatgtgggggtcaagagccccctcgtgtgcgccatcaacaacgccttcagcaggtacagcatctccgataacgacctgttccactttaacaagaagatgttcgcccggcggaggattttgctcaagaagaaccggcacaagcgggccggacacggggccaagaacaagctcaagcccatcactatcctgaccgagaagagcgagaggttcaggaagaagctcatcgagagatgggcctgcgagatcgccgatttctttattaagaacaaggtcggaacagtgcagatggagaacctcgagagcatgaagaggaaggaggattcctacttcaacattcggctgagggggttctggccctacgctgagatgcagaacaagattgagtttaagctgaagcagtacgggattgagatccggaaggtggcccccaacaacaccagcaagacctgcagcaagtgcgggcacctcaacaactacttcaacttcgagtaccggaagaagaacaagttcccacacttcaagtgcgagaagtgcaactttaaggagaacgccgattacaacgccgccctgaacatcagcaaccctaagctgaagagcactaaggaggagccccaaagaagaagcggaaagtc

SEQ ID NO: 274 - DNA, 3009 bp, Artificial Sequence; identical to SEQ ID NO: 269
  Amino acid sequence (N terminal -Cytidine deaminase)

SEQ ID NO: 275 - DNA, 3009 bp, Artificial Sequence
  Amino acid sequence (C terminal -Cytidine deaminase)
atgccaaagaagaagcggaaagtcgccaagaacacaattacaaagacactgaagctgaggatcgtgagaccatacaacagcgctgaggtcgagaagattgtggctgatgaaaagaacaacagggaaaagatcgccctcgagaagaacaaggataaggtgaaggaggcctgctctaagcacctgaaagtggccgcctactgcaccacacaggtggagaggaacgcctgtctgttttgtaaagctcggaagctggatgataagttttaccagaagctgcggggccagttccccgatgccgtcttttggcaggagattagcgagatcttcagacagctgcagaagcaggccgccgagatctacaaccagagcctgatcgagctctactacgagatcttcatcaagggcaagggcattgccaacgcctcctccgtggagcactacctgagcgacgtgtgctacacaagagccgccgagctctttaagaacgccgctatcgcttccgggctgaggagcaagattaagagtaacttccggctcaaggagctgaagaacatgaagagcggcctgcccactacaaagagcgacaacttcccaattccactggtgaagcagaaggggggccagtacacagggttcgagatttccaaccacaacagcgactttattattaagatcccctttggcaggtggcaggtcaagaaggagattgacaagtacaggccctgggagaagtttgatttcgagcaggtgcagaagagccccaagcctatttccctgctgctgtccacacagcggcggaagaggaacaaggggtggtctaaggatgaggggaccgaggccgagattaagaaagtgatgaacggcgactaccagacaagctacatcgaggtcaagcggggcagtaagattggcgagaagagcgcctggatgctgaacctgagcattgacgtgccaaagattgataagggcgtggatcccagcatcatcggagggatcgatgtgggggtcaagagccccctcgtgtgcgccatcaacaacgccttcagcaggtacagcatctccgataacgacctgttccactttaacaagaagatgttcgcccggcggaggattttgctcaagaagaaccggcacaagcgggccggacacggggccaagaacaagctcaagcccatcactatcctgaccgagaagagcgagaggttcaggaagaagctcatcgagagatgggcctgcgagatcgccgatttctttattaagaacaaggtcggaacagtgcagatggagaacctcgagagcatgaagaggaaggaggattcctacttcaacattcggctgagggggttctggccctacgctgagatgcagaacaagattgagtttaagctgaagcagtacgggattgagatccggaaggtggcccccaacaacaccagcaagacctgcagcaagtgcgggcacctcaacaactacttcaacttcgagtaccggaagaagaacaagttcccacacttcaagtgcgagaagtgcaactttaaggagaacgccgattacaacgccgccctgaacatcagcaaccctaagctgaagagcactaaggaggagccctctggaggatctagcggaggatcctctggcagcgagacaccaggaacaagcgagtcagcaacaccagagagcagtggcggcagcagcggcggcagctcctcagagactgggcctgtcgccgtcgatccaaccctgcgccgccggattgaacctcacgagtttgaagtgttctttgacccccgggagctgagaaaggagacatgcctgctgtacgagatcaactggggaggcaggcactccatctggaggcacacctctcagaacacaaataagcacgtggaggtgaacttcatcgagaagtttaccacagagcggtacttctgccccaataccagatgtagcatcacatggtttctgagctggtccccttgcggagagtgtagcagggccatcaccgagttcctgtccagatatccacacgtgacactgtttatctacatcgccaggctgtatcaccacgcagacccaaggaataggcagggcctgcgcgatctgatcagctccggcgtgaccatccagatcatgacagagcaggagtccggctactgctggcggaacttcgtgaattattctcctagcaacgaggcccactggcctaggtacccacacctgtgggtgcgcctgtacgtgctggagctgtattgcatcatcctgggcctgcccccttgtctgaatatcctgcggagaaagcagccccagctgaccttctttacaatcgccctgcagtcttgtcactatcagaggctgccaccccacatcctgtgggccacaggcctgaagagcggcgggagcggcgggagcggggggagcactaatctgagcgacatcattgagaaggagactgggaaacagctggtcattcaggagtccatcctgatgctgcctgaggaggtggaggaagtgatcggcaacaagccagagtctgacatcctggtgcacaccgcctacgacgagtccacagatgagaatgtgatgctgctgacctctgacgcccccgagtataagccttgggccctggtcatccaggattctaacggcgagaataagatcaagatgctgagcggaggatccggaggatctggaggcagcaccaacctgtctgacatcatcgagaaggagacaggcaagcagctggtcatccaggagagcatcctgatgctgcccgaagaagtcgaagaagtgatcggaaacaagcctgagagcgatatcctggtccataccgcctacgacgagagtaccgacgaaaatgtgatgctgctgacatccgacgccccagagtataagccctgggctctggtcatccaggattccaacggagagaacaaaatcaaaatgctgtctggcggctcaaaaagaaccgccgacggcagcgaattcgagcccaagaagaagaggaaagtc

SEQ ID NO: 276 - DNA, 2823 bp, Artificial Sequence
  DNA sequence (N terminal -Adenine deaminase)
atgtccgaagtcgagttttcccatgagtactggatgagacacgcattgactctcgcaaagagggcttgggatgaacgcgaggtgcccgtgggggcagtactcgtgcataacaatcgcgtaatcggcgaaggttggaataggccgatcggacgccacgaccccactgcacatgcggaaatcatggcccttcgacagggagggcttgtgatgcagaattatcgacttatcgatgcgacgctgtacgtcacgcttgaaccttgcgtaatgtgcgcgggagctatgattcactcccgcattggacgagttgtattcggtgcccgcgacgccaagacgggtgccgcaggttcactgatggacgtgctgcatcacccaggcatgaaccaccgggtagaaatcacagaaggcatattggcggacgaatgtgcggcgctgttgtccgacttttttcgcatgcggaggcaggagatcaaggcccagaaaaaagcacaatcctctactgactctggtggttcttctggtggttctagcggcagcgagactcccgggacctcagagtccgccacacccgaaagttctggtggttcttctggtggttcttccgaagtcgagttttcccatgagtactggatgagacacgcattgactctcgcaaagagggctcgagatgaacgcgaggtgcccgtgggggcagtactcgtgctcaacaatcgcgtaatcggcgaaggttggaatagggcaatcggactccacgaccccactgcacatgcggaaatcatggcccttcgacagggagggcttgtgatgcagaattatcgacttatcgatgcgacgctgtacgtcacgtttgaaccttgcgtaatgtgcgcgggagctatgattcactcccgcattggacgagttgtattcggtgttcgcaacgccaagacgggtgccgcaggttcactgatggacgtgctgcattacccaggcatgaaccaccgggtagaaatcacagaaggcatattggcggacgaatgtgcggcgctgttgtgttacttttttcgcatgcccaggcaggtctttaacgcccagaaaaaagcacaatcctctactgactctggtggttcttctggtggttctagcggcagcgagactcccgggacctcagagtccgccacacccgaaagttctggtggttcttctggtggttctgccaagaacacaattacaaagacactgaagctgaggatcgtgagaccatacaacagcgctgaggtcgagaagattgtggctgatgaaaagaacaacagggaaaagatcgccctcgagaagaacaaggataaggtgaaggaggcctgctctaagcacctgaaagtggccgcctactgcaccacacaggtggagaggaacgcctgtctgttttgtaaagctcggaagctggatgataagttttaccagaagctgcggggccagttccccgatgccgtcttttggcaggagattagcgagatcttcagacagctgcagaagcaggccgccgagatctacaaccagagcctgatcgagctctactacgagatcttcatcaagggcaagggcattgccaacgcctcctccgtggagcactacctgagcgacgtgtgctacacaagagccgccgagctctttaagaacgccgctatcgcttccgggctgaggagcaagattaagagtaacttccggctcaaggagctgaagaacatgaagagcggcctgcccactacaaagagcgacaacttcccaattccactggtgaagcagaaggggggccagtacacagggttcgagatttccaaccacaacagcgactttattattaagatcccctttggcaggtggcaggtcaagaaggagattgacaagtacaggccctgggagaagtttgatttcgagcaggtgcagaagagccccaagcctatttccctgctgctgtccacacagcggcggaagaggaacaaggggtggtctaaggatgaggggaccgaggccgagattaagaaagtgatgaacggcgactaccagacaagctacatcgaggtcaagcggggcagtaagattggcgagaagagcgcctggatgctgaacctgagcattgacgtgccaaagattgataagggcgtggatcccagcatcatcggagggatcgatgtgggggtcaagagccccctcgtgtgcgccatcaacaacgccttcagcaggtacagcatctccgataacgacctgttccactttaacaagaagatgttcgcccggcggaggattttgctcaagaagaaccggcacaagcgggccggacacggggccaagaacaagctcaagcccatcactatcctgaccgagaagagcgagaggttcaggaagaagctcatcgagagatgggcctgcgagatcgccgatttctttattaagaacaaggtcggaacagtgcagatggagaacctcgagagcatgaagaggaaggaggattcctacttcaacattcggctgagggggttctggccctacgctgagatgcagaacaagattgagtttaagctgaagcagtacgggattgagatccggaaggtggcccccaacaacaccagcaagacctgcagcaagtgcgggcacctcaacaactacttcaacttcgagtaccggaagaagaacaagttcccacacttcaagtgcgagaagtgcaactttaaggagaacgccgattacaacgccgccctgaacatcagcaaccctaagctgaagagcactaaggaggagcccaaaaggccggcggccacgaaaaaggccggccaggcaaaaaagaaaaag

SEQ ID NO: 277 - DNA, 2823 bp, Artificial Sequence
  DNA sequence (C terminal -Adenine deaminase)
atggccaagaacacaattacaaagacactgaagctgaggatcgtgagaccatacaacagcgctgaggtcgagaagattgtggctgatgaaaagaacaacagggaaaagatcgccctcgagaagaacaaggataaggtgaaggaggcctgctctaagcacctgaaagtggccgcctactgcaccacacaggtggagaggaacgcctgtctgttttgtaaagctcggaagctggatgataagttttaccagaagctgcggggccagttccccgatgccgtcttttggcaggagattagcgagatcttcagacagctgcagaagcaggccgccgagatctacaaccagagcctgatcgagctctactacgagatcttcatcaagggcaagggcattgccaacgcctcctccgtggagcactacctgagcgacgtgtgctacacaagagccgccgagctctttaagaacgccgctatcgcttccgggctgaggagcaagattaagagtaacttccggctcaaggagctgaagaacatgaagagcggcctgcccactacaaagagcgacaacttcccaattccactggtgaagcagaaggggggccagtacacagggttcgagatttccaaccacaacagcgactttattattaagatcccctttggcaggtggcaggtcaagaaggagattgacaagtacaggccctgggagaagtttgatttcgagcaggtgcagaagagccccaagcctatttccctgctgctgtccacacagcggcggaagaggaacaaggggtggtctaaggatgaggggaccgaggccgagattaagaaagtgatgaacggcgactaccagacaagctacatcgaggtcaagcggggcagtaagattggcgagaagagcgcctggatgctgaacctgagcattgacgtgccaaagattgataagggcgtggatcccagcatcatcggagggatcgatgtgggggtcaagagccccctcgtgtgcgccatcaacaacgccttcagcaggtacagcatctccgataacgacctgttccactttaacaagaagatgttcgcccggcggaggattttgctcaagaagaaccggcacaagcgggccggacacggggccaagaacaagctcaagcccatcactatcctgaccgagaagagcgagaggttcaggaagaagctcatcgagagatgggcctgcgagatcgccgatttctttattaagaacaaggtcggaacagtgcagatggagaacctcgagagcatgaagaggaaggaggattcctacttcaacattcggctgagggggttctggccctacgctgagatgcagaacaagattgagtttaagctgaagcagtacgggattgagatccggaaggtggcccccaacaacaccagcaagacctgcagcaagtgcgggcacctcaacaactacttcaacttcgagtaccggaagaagaacaagttcccacacttcaagtgcgagaagtgcaactttaaggagaacgccgattacaacgccgccctgaacatcagcaaccctaagctgaagagcactaaggaggagccctctggaggatctagcggaggatcctctggcagcgagacaccaggaacaagcgagtcagcaacaccagagagcagtggcggcagcagcggcggcagctccgaagtcgagttttcccatgagtactggatgagacacgcattgactctcgcaaagagggcttgggatgaacgcgaggtgcccgtgggggcagtactcgtgcataacaatcgcgtaatcggcgaaggttggaataggccgatcggacgccacgaccccactgcacatgcggaaatcatggcccttcgacagggagggcttgtgatgcagaattatcgacttatcgatgcgacgctgtacgtcacgcttgaaccttgcgtaatgtgcgcgggagctatgattcactcccgcattggacgagttgtattcggtgcccgcgacgccaagacgggtgccgcaggttcactgatggacgtgctgcatcacccaggcatgaaccaccgggtagaaatcacagaaggcatattggcggacgaatgtgcggcgctgttgtccgacttttttcgcatgcggaggcaggagatcaaggcccagaaaaaagcacaatcctctactgactctggtggttcttctggtggttctagcggcagcgagactcccgggacctcagagtccgccacacccgaaagttcaggtggatcttcaggtggatcttcggaagtggaattttcgcacgagtattggatgaggcacgctttaactctcgctaagagagcacgagacgaacgggaagtgccggttggggctgtcctcgtactcaataatcgagttatcggagaaggctggaacagggcaatcggactccacgatcccacagctcatgccgagataatggcgcttcgacaaggaggcctagtcatgcaaaattatcgtcttattgacgcgaccctctacgtgacctttgagccatgcgttatgtgtgcgggtgcaatgatacattcccggataggacgtgtagtatttggagttcgcaacgcgaagaccggtgcggctggttctctcatggatgtcctgcactaccctgggatgaatcaccgcgttgaaatcactgaaggcattttggccgatgaatgcgcggccctgttatgttacttttttcgcatgcccaggcaggtctttaacgcacagaagaaagcccaatcgtccactgataaaaggccggcggccacgaaaaaggccggccaggcaaaaaagaaaaag

SEQ ID NO: 278 - protein, 7 aa, simian virus 40
PKKKRKV

SEQ ID NO: 279 - protein, 16 aa, mus musculus
KRPAATKKAGQAKKKK

SEQ ID NO: 280 - protein, 9 aa, homo sapiens
PAAKRVKLD

SEQ ID NO: 281 - protein, 11 aa, Homo sapiens
RQRRNELKRSP

SEQ ID NO: 282 - protein, 38 aa, mus musculus
NQSSNFGPMKGGNFGGRSSGPYGGGGQYFAKPRNQGGY

SEQ ID NO: 283 - protein, 42 aa, Homo sapiens
RMRIZFKNKGKDTAELRRRRVEVSVELRKAKKDEQILKRRNV

SEQ ID NO: 284 - protein, 8 aa, Homo sapiens
VSRKRPRP

SEQ ID NO: 285 - protein, 8 aa, homo sapiens
PPKKARED

SEQ ID NO: 286 - protein, 8 aa, homo sapiens
PQPKKKPL

SEQ ID NO: 287 - protein, 12 aa, mus musculus
SALIKKKKKMAP

SEQ ID NO: 288 - protein, 5 aa, Influenza virus
DRLRR

SEQ ID NO: 289 - protein, 7 aa, influenza virus
PKQKKRK

SEQ ID NO: 290 - protein, 10 aa, Hepatitis D virus
RKLKKKIKKL

SEQ ID NO: 291 - protein, 10 aa, mus musculus
REKKKFLKRR

SEQ ID NO: 292 - protein, 20 aa, homo sapiens
KRKGDEVDGVDEVAKKKSKK

SEQ ID NO: 293 - protein, 17 aa, Homo sapiens
RKCLQAGMNLEARKTKK

SEQ ID NO: 294 - RNA, 181 nt, Artificial Sequence
  Comperative Example 1.1.1
cuucacugauaaaguggagaaccgcuucaccaaaagcugucccuuaggggauuagaacuugagugaaggugggcugcuugcaucagccuaaugucgagaagugcuuucuucggaaaguaacccucgaaacaaauucauuugaaagaaugaaggaaugcaaccacacacacagugggcuacc

SEQ ID NO: 295 - RNA, 190 nt, Artificial Sequence
  Comperative Example 1.1.2
cuucacugauaaaguggagaaccgcuucaccaaaagcugucccuuaggggauuagaacuugagugaaggugggcugcuugcaucagccuaaugucgagaagugcuuucuucggaaaguaacccucgaaacaaauucauuugaaagaaugaaggaaugcaaccacacacacagugggcuaccuuuuauuuu

SEQ ID NO: 296 - RNA, 183 nt, Artificial Sequence
  Example 1.1.1
gauaaaguggagaaccgcuucaccaaaagcugucccuuaggggauuagaacuugagugaaggugggcugcuugcaucagccuaaugucgagaagugcuuucuucggaaaguaacccucgaaacaaauucauuugaaagaaugaaggaaugcaaccacacacacagugggcuaccuuuuauuuu

SEQ ID NO: 297 - RNA, 176 nt, Artificial Sequence
  Example 1.1.2
uggagaaccgcuucaccaaaagcugucccuuaggggauuagaacuugagugaaggugggcugcuugcaucagccuaaugucgagaagugcuuucuucggaaaguaacccucgaaacaaauucauuugaaagaaugaaggaaugcaaccacacacacagugggcuaccuuuuauuuu

SEQ ID NO: 298 - RNA, 170 nt, Artificial Sequence
  Example 1.1.3
accgcuucaccaaaagcugucccuuaggggauuagaacuugagugaaggugggcugcuugcaucagccuaaugucgagaagugcuuucuucggaaaguaacccucgaaacaaauucauuugaaagaaugaaggaaugcaaccacacacacagugggcuaccuuuuauuuu

SEQ ID NO: 299 - RNA, 184 nt, Artificial Sequence
  Example 1.1.4
cuucacugauaaaguggagaaccgcuucaccaaaagcuguuuagauuagaacuugagugaaggugggcugcuugcaucagccuaaugucgagaagugcuuucuucggaaaguaacccucgaaacaaauucauuugaaagaaugaaggaaugcaaccacacacacagugggcuaccuuuuauuuu

SEQ ID NO: 300 - RNA, 179 nt, Artificial Sequence
  Example 1.1.5
cuucacugauaaaguggagaaccgcuucaccaaaagcuuuagagaacuugagugaaggugggcugcuugcaucagccuaaugucgagaagugcuuucuucggaaaguaacccucgaaacaaauucauuugaaagaaugaaggaaugcaaccacacacacagugggcuaccuuuuauuuu

SEQ ID NO: 301 - RNA, 169 nt, Artificial Sequence
  Example 1.1.6
cuucacugauaaaguggagaaccgcuucaccaauuaguugagugaaggugggcugcuugcaucagccuaaugucgagaagugcuuucuucggaaaguaacccucgaaacaaauucauuugaaagaaugaaggaaugcaaccacacacacagugggcuaccuuuuauuuu

SEQ ID NO: 302 - RNA, 186 nt, Artificial Sequence
  Example 1.1.7
cuucacugauaaaguggagaaccgcuucaccaaaagcugucccuuaggggauuagaacuugagugaaggugggcugcuugcaucagccuaaugucgagaagugcuuucuucggaaaguaacccucgaaacaaauucaugaaaaugaaggaaugcaaccacacacacagugggcuaccuuuuauuuu

SEQ ID NO: 303 - RNA, 182 nt, Artificial Sequence
  Example 1.1.8
cuucacugauaaaguggagaaccgcuucaccaaaagcugucccuuaggggauuagaacuugagugaaggugggcugcuugcaucagccuaaugucgagaagugcuuucuucggaaaguaacccucgaaacaaauucgaaagaaggaaugcaaccacacacacagugggcuaccuuuuauuuu

SEQ ID NO: 304 - RNA, 176 nt, Artificial Sequence
  Example 1.1.9
cuucacugauaaaguggagaaccgcuucaccaaaagcugucccuuaggggauuagaacuugagugaaggugggcugcuugcaucagccuaaugucgagaagugcuuucuucggaaaguaacccucgaaacaaagaaaggaaugcaaccacacacacagugggcuaccuuuuauuuu

SEQ ID NO: 305 - RNA, 147 nt, Artificial Sequence
  Example 1.1.10
accgcuucaccauuagugagugaaggugggcugcuugcaucagccuaaugucgagaagugcuuucuucggaaaguaacccucgaaacaaauucauuugaaagaaugaaggaaugcaaccacacacacagugggcuaccuuuuauuuu

SEQ ID NO: 306 - RNA, 156 nt, Artificial Sequence
  Example 1.1.11
accgcuucaccaaaagcugucccuuaggggauuagaacuugagugaaggugggcugcuugcaucagccuaaugucgagaagugcuuucuucggaaaguaacccucgaaacaaagaaaggaaugcaaccacacacacagugggcuaccuuuuauuuu

SEQ ID NO: 307 - RNA, 153 nt, Artificial Sequence
  Example 1.1.12
cuucacugauaaaguggagaaccgcuucaccauuagugagugaaggugggcugcuugcaucagccuaaugucgagaagugcuuucuucggaaaguaacccucgaaacaaagaaaggaaugcaaccacacacacagugggcuaccuuuuauuuu

SEQ ID NO: 308 - RNA, 133 nt, Artificial Sequence
  Example 1.1.13
accgcuucaccauuagugagugaaggugggcugcuugcaucagccuaaugucgagaagugcuuucuucggaaaguaacccucgaaacaaagaaaggaaugcaaccacacacacagugggcuaccuuuuauuuu

SEQ ID NO: 309 - RNA, 181 nt, Artificial Sequence
  Comperative Example 1.2.1
cuucacugauaaaguggagaaccgcuucaccaaaagcugucccuuaggggauuagaacuugagugaaggugggcugcuugcaucagccuaaugucgagaagugcuuucuucggaaaguaacccucgaaacaaauucauuugaaagaaugaaggaaugcaaccauccccaggacacacacac

SEQ ID NO: 310 - RNA, 190 nt, Artificial Sequence
  Comperative Example 1.2.2
cuucacugauaaaguggagaaccgcuucaccaaaagcugucccuuaggggauuagaacuugagugaaggugggcugcuugcaucagccuaaugucgagaagugcuuucuucggaaaguaacccucgaaacaaauucauuugaaagaaugaaggaaugcaaccauccccaggacacacacacuuuuauuuu

SEQ ID NO: 311 - RNA, 183 nt, Artificial Sequence
  Example 1.2.1
gauaaaguggagaaccgcuucaccaaaagcugucccuuaggggauuagaacuugagugaaggugggcugcuugcaucagccuaaugucgagaagugcuuucuucggaaaguaacccucgaaacaaauucauuugaaagaaugaaggaaugcaaccauccccaggacacacacacuuuuauuuu

SEQ ID NO: 312 - RNA, 176 nt, Artificial Sequence
  Example 1.2.2
uggagaaccgcuucaccaaaagcugucccuuaggggauuagaacuugagugaaggugggcugcuugcaucagccuaaugucgagaagugcuuucuucggaaaguaacccucgaaacaaauucauuugaaagaaugaaggaaugcaaccauccccaggacacacacacuuuuauuuu

SEQ ID NO: 313 - RNA, 170 nt, Artificial Sequence
  Example 1.2.3
accgcuucaccaaaagcugucccuuaggggauuagaacuugagugaaggugggcugcuugcaucagccuaaugucgagaagugcuuucuucggaaaguaacccucgaaacaaauucauuugaaagaaugaaggaaugcaaccauccccaggacacacacacuuuuauuuu

SEQ ID NO: 314 - RNA, 184 nt, Artificial Sequence
  Example 1.2.4
cuucacugauaaaguggagaaccgcuucaccaaaagcuguuuagauuagaacuugagugaaggugggcugcuugcaucagccuaaugucgagaagugcuuucuucggaaaguaacccucgaaacaaauucauuugaaagaaugaaggaaugcaaccauccccaggacacacacacuuuuauuuu

SEQ ID NO: 315 - RNA, 178 nt, Artificial Sequence
  Example 1.2.5
cuucacugauaaaguggagaaccgcuucaccaaaagcuuagagaacuugagugaaggugggcugcuugcaucagccuaaugucgagaagugcuuucuucggaaaguaacccucgaaacaaauucauuugaaagaaugaaggaaugcaaccauccccaggacacacacacuuuuauuuu

SEQ ID NO: 316 - RNA, 167 nt, Artificial Sequence
  Example 1.2.6
cuucacugauaaaguggagaaccgcuucaccauuagugagugaaggugggcugcuugcaucagccuaaugucgagaagugcuuucuucggaaaguaacccucgaaacaaauucauuugaaagaaugaaggaaugcaaccauccccaggacacacacacuuuuauuuu

SEQ ID NO: 317 - RNA, 186 nt, Artificial Sequence
  Example 1.2.7
cuucacugauaaaguggagaaccgcuucaccaaaagcugucccuuaggggauuagaacuugagugaaggugggcugcuugcaucagccuaaugucgagaagugcuuucuucggaaaguaacccucgaaacaaauucaugaaaaugaaggaaugcaaccauccccaggacacacacacuuuuauuuu

SEQ ID NO: 318 - RNA, 182 nt, Artificial Sequence
  Example 1.2.8
cuucacugauaaaguggagaaccgcuucaccaaaagcugucccuuaggggauuagaacuugagugaaggugggcugcuugcaucagccuaaugucgagaagugcuuucuucggaaaguaacccucgaaacaaauucgaaagaaggaaugcaaccauccccaggacacacacacuuuuauuuu

SEQ ID NO: 319 - RNA, 176 nt, Artificial Sequence
  Example 1.2.9
cuucacugauaaaguggagaaccgcuucaccaaaagcugucccuuaggggauuagaacuugagugaaggugggcugcuugcaucagccuaaugucgagaagugcuuucuucggaaaguaacccucgaaacaaagaaaggaaugcaaccauccccaggacacacacacuuuuauuuu

SEQ ID NO: 320 - RNA, 147 nt, Artificial Sequence
  Example 1.2.10
accgcuucaccauuagugagugaaggugggcugcuugcaucagccuaaugucgagaagugcuuucuucggaaaguaacccucgaaacaaauucauuugaaagaaugaaggaaugcaaccauccccaggacacacacacuuuuauuuu

SEQ ID NO: 321 - RNA, 156 nt, Artificial Sequence
  Example 1.2.11
accgcuucaccaaaagcugucccuuaggggauuagaacuugagugaaggugggcugcuugcaucagccuaaugucgagaagugcuuucuucggaaaguaacccucgaaacaaagaaaggaaugcaaccauccccaggacacacacacuuuuauuuu

SEQ ID NO: 322 - RNA, 153 nt, Artificial Sequence
  Example 1.2.12
cuucacugauaaaguggagaaccgcuucaccauuagugagugaaggugggcugcuugcaucagccuaaugucgagaagugcuuucuucggaaaguaacccucgaaacaaagaaaggaaugcaaccauccccaggacacacacacuuuuauuuu

SEQ ID NO: 323 - RNA, 133 nt, Artificial Sequence
  Example 1.2.13
accgcuucaccauuagugagugaaggugggcugcuugcaucagccuaaugucgagaagugcuuucuucggaaaguaacccucgaaacaaagaaaggaaugcaaccauccccaggacacacacacuuuuauuuu

SEQ ID NO: 324 - RNA, 181 nt, Artificial Sequence
  Comperative Example 1.3.1
cuucacugauaaaguggagaaccgcuucaccaaaagcugucccuuaggggauuagaacuugagugaaggugggcugcuugcaucagccuaaugucgagaagugcuuucuucggaaaguaacccucgaaacaaauucauuugaaagaaugaaggaaugcaacagaacacauaccccugggcc

SEQ ID NO: 325 - RNA, 190 nt, Artificial Sequence
  Comperative Example 1.3.2
cuucacugauaaaguggagaaccgcuucaccaaaagcugucccuuaggggauuagaacuugagugaaggugggcugcuugcaucagccuaaugucgagaagugcuuucuucggaaaguaacccucgaaacaaauucauuugaaagaaugaaggaaugcaacagaacacauaccccugggccuuuuauuuu

SEQ ID NO: 326 - RNA, 183 nt, Artificial Sequence
  Example 1.3.1
gauaaaguggagaaccgcuucaccaaaagcugucccuuaggggauuagaacuugagugaaggugggcugcuugcaucagccuaaugucgagaagugcuuucuucggaaaguaacccucgaaacaaauucauuugaaagaaugaaggaaugcaacagaacacauaccccugggccuuuuauuuu

SEQ ID NO: 327 - RNA, 176 nt, Artificial Sequence
  Example 1.3.2
uggagaaccgcuucaccaaaagcugucccuuaggggauuagaacuugagugaaggugggcugcuugcaucagccuaaugucgagaagugcuuucuucggaaaguaacccucgaaacaaauucauuugaaagaaugaaggaaugcaacagaacacauaccccugggccuuuuauuuu

SEQ ID NO: 328 - RNA, 170 nt, Artificial Sequence
  Example 1.3.3
accgcuucaccaaaagcugucccuuaggggauuagaacuugagugaaggugggcugcuugcaucagccuaaugucgagaagugcuuucuucggaaaguaacccucgaaacaaauucauuugaaagaaugaaggaaugcaacagaacacauaccccugggccuuuuauuuu

SEQ ID NO: 329 - RNA, 184 nt, Artificial Sequence
  Example 1.3.4
cuucacugauaaaguggagaaccgcuucaccaaaagcuguuuagauuagaacuugagugaaggugggcugcuugcaucagccuaaugucgagaagugcuuucuucggaaaguaacccucgaaacaaauucauuugaaagaaugaaggaaugcaacagaacacauaccccugggccuuuuauuuu

SEQ ID NO: 330 - RNA, 179 nt, Artificial Sequence
  Example 1.3.5
cuucacugauaaaguggagaaccgcuucaccaaaagcuuuagagaacuugagugaaggugggcugcuugcaucagccuaaugucgagaagugcuuucuucggaaaguaacccucgaaacaaauucauuugaaagaaugaaggaaugcaacagaacacauaccccugggccuuuuauuuu

SEQ ID NO: 331 - RNA, 169 nt, Artificial Sequence
  Example 1.3.6
cuucacugauaaaguggagaaccgcuucaccaauuaguugagugaaggugggcugcuugcaucagccuaaugucgagaagugcuuucuucggaaaguaacccucgaaacaaauucauuugaaagaaugaaggaaugcaacagaacacauaccccugggccuuuuauuuu

SEQ ID NO: 332 - RNA, 186 nt, Artificial Sequence
  Example 1.3.7
cuucacugauaaaguggagaaccgcuucaccaaaagcugucccuuaggggauuagaacuugagugaaggugggcugcuugcaucagccuaaugucgagaagugcuuucuucggaaaguaacccucgaaacaaauucaugaaaaugaaggaaugcaacagaacacauaccccugggccuuuuauuuu

SEQ ID NO: 333 - RNA, 182 nt, Artificial Sequence
  Example 1.3.8
cuucacugauaaaguggagaaccgcuucaccaaaagcugucccuuaggggauuagaacuugagugaaggugggcugcuugcaucagccuaaugucgagaagugcuuucuucggaaaguaacccucgaaacaaauucgaaagaaggaaugcaacagaacacauaccccugggccuuuuauuuu

SEQ ID NO: 334 - RNA, 176 nt, Artificial Sequence
  Example 1.3.9
cuucacugauaaaguggagaaccgcuucaccaaaagcugucccuuaggggauuagaacuugagugaaggugggcugcuugcaucagccuaaugucgagaagugcuuucuucggaaaguaacccucgaaacaaagaaaggaaugcaacagaacacauaccccugggccuuuuauuuu

SEQ ID NO: 335 - RNA, 147 nt, Artificial Sequence
  Example 1.3.10
accgcuucaccauuagugagugaaggugggcugcuugcaucagccuaaugucgagaagugcuuucuucggaaaguaacccucgaaacaaauucauuugaaagaaugaaggaaugcaacagaacacauaccccugggccuuuuauuuu

SEQ ID NO: 336 - RNA, 156 nt, Artificial Sequence
  Example 1.3.11
accgcuucaccaaaagcugucccuuaggggauuagaacuugagugaaggugggcugcuugcaucagccuaaugucgagaagugcuuucuucggaaaguaacccucgaaacaaagaaaggaaugcaacagaacacauaccccugggccuuuuauuuu

SEQ ID NO: 337 - RNA, 153 nt, Artificial Sequence
  Example 1.3.12
cuucacugauaaaguggagaaccgcuucaccauuagugagugaaggugggcugcuugcaucagccuaaugucgagaagugcuuucuucggaaaguaacccucgaaacaaagaaaggaaugcaacagaacacauaccccugggccuuuuauuuu

SEQ ID NO: 338 - RNA, 133 nt, Artificial Sequence
  Example 1.3.13
accgcuucaccauuagugagugaaggugggcugcuugcaucagccuaaugucgagaagugcuuucuucggaaaguaacccucgaaacaaagaaaggaaugcaacagaacacauaccccugggccuuuuauuuu

SEQ ID NO: 339 - DNA, 20 bp, Artificial Sequence
  Protospacer sequence for targeting DY2
cacacacacagtgggctacc

SEQ ID NO: 340 - DNA, 20 bp, Artificial Sequence
  Protospacer sequence for targeting DY10
catccccaggacacacacac

SEQ ID NO: 341 - DNA, 20 bp, Artificial Sequence
  Protospacer sequence for targeting Intergenic-22
agaacacatacccctgggcc

SEQ ID NO: 342 - RNA, 23 nt, Artificial Sequence
  modified second region
ccgcuucacuuaggugaaggugg

SEQ ID NO: 343 - RNA, 11 nt, Artificial Sequence
  modified second region
ccguuaggugg

SEQ ID NO: 344 - RNA, 13 nt, Artificial Sequence
  modified second region
ccgcuuagggugg

SEQ ID NO: 345 - RNA, 15 nt, Artificial Sequence
  modified second region
ccgcuuuagaggugg

SEQ ID NO: 346 - RNA, 17 nt, Artificial Sequence
  modified second region
ccgcuuuuagaaggugg

SEQ ID NO: 347 - RNA, 19 nt, Artificial Sequence
  modified second region
ccgcuucuuaggaaggugg

SEQ ID NO: 348 - RNA, 21 nt, Artificial Sequence
  modified second region
ccgcuucauuagugaaggugg

SEQ ID NO: 349 - RNA, 23 nt, Artificial Sequence
  modified second region
ccgcuucacuuaggugaaggugg

SEQ ID NO: 350 - RNA, 24 nt, Artificial Sequence
  modified second region
ccgcuucacuuagagugaaggugg

SEQ ID NO: 351 - RNA, 26 nt, Artificial Sequence
  modified second region
ccgcuucaccuuaggagugaaggugg

SEQ ID NO: 352 - RNA, 28 nt, Artificial Sequence
  modified second region
ccgcuucaccauuagugagugaaggugg

SEQ ID NO: 353 - RNA, 30 nt, Artificial Sequence; identical to SEQ ID NO: 40
  modified second region

SEQ ID NO: 354 - RNA, 32 nt, Artificial Sequence; identical to SEQ ID NO: 41
  modified second region

SEQ ID NO: 355 - RNA, 34 nt, Artificial Sequence; identical to SEQ ID NO: 42
  modified second region

SEQ ID NO: 356 - RNA, 36 nt, Artificial Sequence; identical to SEQ ID NO: 43
  modified second region

SEQ ID NO: 357 - RNA, 38 nt, Artificial Sequence; identical to SEQ ID NO: 44
  modified second region

SEQ ID NO: 358 - RNA, 40 nt, Artificial Sequence; identical to SEQ ID NO: 45
  modified second region

SEQ ID NO: 359 - RNA, 42 nt, Artificial Sequence; identical to SEQ ID NO: 47
  modified second region

SEQ ID NO: 360 - RNA, 43 nt, Artificial Sequence; identical to SEQ ID NO: 46
  modified second region

SEQ ID NO: 361 - RNA, 45 nt, Artificial Sequence; identical to SEQ ID NO: 48
  modified second region

SEQ ID NO: 362 - RNA, 47 nt, Artificial Sequence; identical to SEQ ID NO: 49
  modified second region

SEQ ID NO: 363 - RNA, 10 nt, Artificial Sequence
  modified second region, upper part (5' to UUAG)
ccgcuuuuag

SEQ ID NO: 364 - RNA, 11 nt, Artificial Sequence
  modified second region, upper part (5' to UUAG)
ccgcuucuuag

SEQ ID NO: 365 - RNA, 12 nt, Artificial Sequence
  modified second region, upper part (5' to UUAG)
ccgcuucauuag

SEQ ID NO: 366 - RNA, 13 nt, Artificial Sequence
  modified second region, upper part (5' to UUAG)
ccgcuucacuuag

SEQ ID NO: 367 - RNA, 14 nt, Artificial Sequence
  modified second region, upper part (5' to UUAG)
ccgcuucaccuuag

SEQ ID NO: 368 - RNA, 15 nt, Artificial Sequence
  modified second region, upper part (5' to UUAG)
ccgcuucaccauuag

SEQ ID NO: 369 - RNA, 16 nt, Artificial Sequence
  modified second region, upper part (5' to UUAG)
ccgcuucaccaauuag

SEQ ID NO: 370 - RNA, 17 nt, Artificial Sequence
  modified second region, upper part (5' to UUAG)
ccgcuucaccaaauuag

SEQ ID NO: 371 - RNA, 18 nt, Artificial Sequence
  modified second region, upper part (5' to UUAG)
ccgcuucaccaaaauuag

SEQ ID NO: 372 - RNA, 19 nt, Artificial Sequence
  modified second region, upper part (5' to UUAG)
ccgcuucaccaaaaguuag

SEQ ID NO: 373 - RNA, 20 nt, Artificial Sequence
  modified second region, upper part (5' to UUAG)
ccgcuucaccaaaagcuuag

SEQ ID NO: 374 - RNA, 21 nt, Artificial Sequence
  modified second region, upper part (5' to UUAG)
ccgcuucaccaaaagcuuuag

SEQ ID NO: 375 - RNA, 22 nt, Artificial Sequence
  modified second region, upper part (5' to UUAG)
ccgcuucaccaaaagcuguuag

SEQ ID NO: 376 - RNA, 23 nt, Artificial Sequence
  modified second region, upper part (5' to UUAG)
ccgcuucaccaaaagcuguuuag

SEQ ID NO: 377 - RNA, 24 nt, Artificial Sequence
  modified second region, upper part (5' to UUAG)
ccgcuucaccaaaagcugucuuag

SEQ ID NO: 378 - RNA, 25 nt, Artificial Sequence
  modified second region, upper part (5' to UUAG)
ccgcuucaccaaaagcuguccuuag

SEQ ID NO: 379 - RNA, 119 nt, Artificial Sequence
  engineered tracrRNA(mature form, the first region is deleted)
ccgcuucaccaaaagcugucccuuaggggauuagaacuugagugaaggugggcugcuugcaucagccuaaugucgagaagugcuuucuucggaaaguaacccucgaaacaaauucauuu

SEQ ID NO: 380 - RNA, 89 nt, Artificial Sequence
  engineered tracrRNA(mature form, the second region is deleted)
cuucacugauaaaguggagaagcugcuugcaucagccuaaugucgagaagugcuuucuucggaaaguaacccucgaaacaaauucauuu

SEQ ID NO: 381 - RNA, 90 nt, Artificial Sequence
  engineered tracrRNA(mature form, having modified second region)
cuucacugauaaaguggagaaggcugcuugcaucagccuaaugucgagaagugcuuucuucggaaaguaacccucgaaacaaauucauuu

SEQ ID NO: 382 - RNA, 94 nt, Artificial Sequence
  engineered tracrRNA(mature form, having modified second region)
cuucacugauaaaguggagaauuagggcugcuugcaucagccuaaugucgagaagugcuuucuucggaaaguaacccucgaaacaaauucauuu

SEQ ID NO: 383 - RNA, 96 nt, Artificial Sequence
  engineered tracrRNA(mature form, having modified second region)
cuucacugauaaaguggagaacuuaggggcugcuugcaucagccuaaugucgagaagugcuuucuucggaaaguaacccucgaaacaaauucauuu

SEQ ID NO: 384 - RNA, 97 nt, Artificial Sequence
  engineered tracrRNA(mature form, having modified second region)
cuucacugauaaaguggagaacuuagugggcugcuugcaucagccuaaugucgagaagugcuuucuucggaaaguaacccucgaaacaaauucauuu

SEQ ID NO: 385 - RNA, 99 nt, Artificial Sequence
  engineered tracrRNA(mature form, having modified second region)
cuucacugauaaaguggagaaccuuaggugggcugcuugcaucagccuaaugucgagaagugcuuucuucggaaaguaacccucgaaacaaauucauuu

SEQ ID NO: 386 - RNA, 100 nt, Artificial Sequence
  engineered tracrRNA(mature form, having modified second region)
cuucacugauaaaguggagaaccguuaggugggcugcuugcaucagccuaaugucgagaagugcuuucuucggaaaguaacccucgaaacaaauucauuu

SEQ ID NO: 387 - RNA, 102 nt, Artificial Sequence
  engineered tracrRNA(mature form, having modified second region)
cuucacugauaaaguggagaaccgcuuagggugggcugcuugcaucagccuaaugucgagaagugcuuucuucggaaaguaacccucgaaacaaauucauuu

SEQ ID NO: 388 - RNA, 104 nt, Artificial Sequence
  engineered tracrRNA(mature form, having modified second region)
cuucacugauaaaguggagaaccgcuuuagaggugggcugcuugcaucagccuaaugucgagaagugcuuucuucggaaaguaacccucgaaacaaauucauuu

SEQ ID NO: 389 - RNA, 106 nt, Artificial Sequence
  engineered tracrRNA(mature form, having modified second region)
cuucacugauaaaguggagaaccgcuuuuagaaggugggcugcuugcaucagccuaaugucgagaagugcuuucuucggaaaguaacccucgaaacaaauucauuu

SEQ ID NO: 390 - RNA, 108 nt, Artificial Sequence
  engineered tracrRNA(mature form, having modified second region)
cuucacugauaaaguggagaaccgcuucuuaggaaggugggcugcuugcaucagccuaaugucgagaagugcuuucuucggaaaguaacccucgaaacaaauucauuu

SEQ ID NO: 391 - RNA, 110 nt, Artificial Sequence
  engineered tracrRNA(mature form, having modified second region)
cuucacugauaaaguggagaaccgcuucauuagugaaggugggcugcuugcaucagccuaaugucgagaagugcuuucuucggaaaguaacccucgaaacaaauucauuu

SEQ ID NO: 392 - RNA, 112 nt, Artificial Sequence
  engineered tracrRNA(mature form, having modified second region)
cuucacugauaaaguggagaaccgcuucacuuaggugaaggugggcugcuugcaucagccuaaugucgagaagugcuuucuucggaaaguaacccucgaaacaaauucauuu

SEQ ID NO: 393 - RNA, 113 nt, Artificial Sequence
  engineered tracrRNA(mature form, having modified second region)
cuucacugauaaaguggagaaccgcuucacuuagagugaaggugggcugcuugcaucagccuaaugucgagaagugcuuucuucggaaaguaacccucgaaacaaauucauuu

SEQ ID NO: 394 - RNA, 115 nt, Artificial Sequence
  engineered tracrRNA(mature form, having modified second region)
cuucacugauaaaguggagaaccgcuucaccuuaggagugaaggugggcugcuugcaucagccuaaugucgagaagugcuuucuucggaaaguaacccucgaaacaaauucauuu

SEQ ID NO: 395 - RNA, 117 nt, Artificial Sequence; identical to SEQ ID NO: 139
  engineered tracrRNA(mature form, having modified second region)

SEQ ID NO: 396 - RNA, 119 nt, Artificial Sequence; identical to SEQ ID NO: 140
  engineered tracrRNA(mature form, having modified second region)

SEQ ID NO: 397 - RNA, 121 nt, Artificial Sequence
  engineered tracrRNA(mature form, having modified second region)
cuucacugauaaaguggagaaccgcuucaccaaauuagcuugagugaaggugggcugcuugcaucagccuaaugucgagaagugcuuucuucggaaaguaacccucgaaacaaauucauuu

SEQ ID NO: 398 - RNA, 123 nt, Artificial Sequence
  engineered tracrRNA(mature form, having modified second region)
cuucacugauaaaguggagaaccgcuucaccaaaauuagacuugagugaaggugggcugcuugcaucagccuaaugucgagaagugcuuucuucggaaaguaacccucgaaacaaauucauuu

SEQ ID NO: 399 - RNA, 125 nt, Artificial Sequence; identical to SEQ ID NO: 142
  engineered tracrRNA(mature form, having modified second region)

SEQ ID NO: 400 - RNA, 127 nt, Artificial Sequence; identical to SEQ ID NO: 143
  engineered tracrRNA(mature form, having modified second region)

SEQ ID NO: 401 - RNA, 129 nt, Artificial Sequence; identical to SEQ ID NO: 144
  engineered tracrRNA(mature form, having modified second region)

SEQ ID NO: 402 - RNA, 131 nt, Artificial Sequence; identical to SEQ ID NO: 146
  engineered tracrRNA(mature form, having modified second region)

SEQ ID NO: 403 - RNA, 132 nt, Artificial Sequence; identical to SEQ ID NO: 145
  engineered tracrRNA(mature form, having modified second region)

SEQ ID NO: 404 - RNA, 134 nt, Artificial Sequence; identical to SEQ ID NO: 147
  engineered tracrRNA(mature form, having modified second region)

SEQ ID NO: 405 - RNA, 136 nt, Artificial Sequence; identical to SEQ ID NO: 148
  engineered tracrRNA(mature form, having modified second region)

SEQ ID NO: 406 - RNA, 138 nt, Artificial Sequence; identical to SEQ ID NO: 149
  engineered tracrRNA(mature form, having modified second region)

SEQ ID NO: 407 - RNA, 110 nt, Artificial Sequence
  engineered scaffold(mature form, the second region is deleted)
cuucacugauaaaguggagaagcugcuugcaucagccuaaugucgagaagugcuuucuucggaaaguaacccucgaaacaaauucauuugaaagaaugaaggaaugcaac

SEQ ID NO: 408 - RNA, 111 nt, Artificial Sequence
  engineered scaffold(mature form, having modified second region)
cuucacugauaaaguggagaaggcugcuugcaucagccuaaugucgagaagugcuuucuucggaaaguaacccucgaaacaaauucauuugaaagaaugaaggaaugcaac

SEQ ID NO: 409 - RNA, 115 nt, Artificial Sequence
  engineered scaffold(mature form, having modified second region)
cuucacugauaaaguggagaauuagggcugcuugcaucagccuaaugucgagaagugcuuucuucggaaaguaacccucgaaacaaauucauuugaaagaaugaaggaaugcaac

SEQ ID NO: 410 - RNA, 117 nt, Artificial Sequence
  engineered scaffold(mature form, having modified second region)
cuucacugauaaaguggagaacuuaggggcugcuugcaucagccuaaugucgagaagugcuuucuucggaaaguaacccucgaaacaaauucauuugaaagaaugaaggaaugcaac

SEQ ID NO: 411 - RNA, 118 nt, Artificial Sequence
  engineered scaffold(mature form, having modified second region)
cuucacugauaaaguggagaacuuagugggcugcuugcaucagccuaaugucgagaagugcuuucuucggaaaguaacccucgaaacaaauucauuugaaagaaugaaggaaugcaac

SEQ ID NO: 412 - RNA, 120 nt, Artificial Sequence
  engineered scaffold(mature form, having modified second region)
cuucacugauaaaguggagaaccuuaggugggcugcuugcaucagccuaaugucgagaagugcuuucuucggaaaguaacccucgaaacaaauucauuugaaagaaugaaggaaugcaac

SEQ ID NO: 413 - RNA, 121 nt, Artificial Sequence
  engineered scaffold(mature form, having modified second region)
cuucacugauaaaguggagaaccguuaggugggcugcuugcaucagccuaaugucgagaagugcuuucuucggaaaguaacccucgaaacaaauucauuugaaagaaugaaggaaugcaac

SEQ ID NO: 414 - RNA, 123 nt, Artificial Sequence
  engineered scaffold(mature form, having modified second region)
cuucacugauaaaguggagaaccgcuuagggugggcugcuugcaucagccuaaugucgagaagugcuuucuucggaaaguaacccucgaaacaaauucauuugaaagaaugaaggaaugcaac

SEQ ID NO: 415 - RNA, 125 nt, Artificial Sequence
  engineered scaffold(mature form, having modified second region)
cuucacugauaaaguggagaaccgcuuuagaggugggcugcuugcaucagccuaaugucgagaagugcuuucuucggaaaguaacccucgaaacaaauucauuugaaagaaugaaggaaugcaac

SEQ ID NO: 416 - RNA, 127 nt, Artificial Sequence
  engineered scaffold(mature form, having modified second region)
cuucacugauaaaguggagaaccgcuuuuagaaggugggcugcuugcaucagccuaaugucgagaagugcuuucuucggaaaguaacccucgaaacaaauucauuugaaagaaugaaggaaugcaac

SEQ ID NO: 417 - RNA, 129 nt, Artificial Sequence
  engineered scaffold(mature form, having modified second region)
cuucacugauaaaguggagaaccgcuucuuaggaaggugggcugcuugcaucagccuaaugucgagaagugcuuucuucggaaaguaacccucgaaacaaauucauuugaaagaaugaaggaaugcaac

SEQ ID NO: 418 - RNA, 131 nt, Artificial Sequence
  engineered scaffold(mature form, having modified second region)
cuucacugauaaaguggagaaccgcuucauuagugaaggugggcugcuugcaucagccuaaugucgagaagugcuuucuucggaaaguaacccucgaaacaaauucauuugaaagaaugaaggaaugcaac

SEQ ID NO: 419 - RNA, 133 nt, Artificial Sequence
  engineered scaffold(mature form, having modified second region)
cuucacugauaaaguggagaaccgcuucacuuaggugaaggugggcugcuugcaucagccuaaugucgagaagugcuuucuucggaaaguaacccucgaaacaaauucauuugaaagaaugaaggaaugcaac

SEQ ID NO: 420 - RNA, 134 nt, Artificial Sequence
  engineered scaffold(mature form, having modified second region)
cuucacugauaaaguggagaaccgcuucacuuagagugaaggugggcugcuugcaucagccuaaugucgagaagugcuuucuucggaaaguaacccucgaaacaaauucauuugaaagaaugaaggaaugcaac

SEQ ID NO: 421 - RNA, 136 nt, Artificial Sequence
  engineered scaffold(mature form, having modified second region)
cuucacugauaaaguggagaaccgcuucaccuuaggagugaaggugggcugcuugcaucagccuaaugucgagaagugcuuucuucggaaaguaacccucgaaacaaauucauuugaaagaaugaaggaaugcaac

SEQ ID NO: 422 - RNA, 138 nt, Artificial Sequence; identical to SEQ ID NO: 188
  engineered scaffold(mature form, having modified second region)

SEQ ID NO: 423 - RNA, 140 nt, Artificial Sequence; identical to SEQ ID NO: 189
  engineered scaffold(mature form, having modified second region)

SEQ ID NO: 424 - RNA, 142 nt, Artificial Sequence; identical to SEQ ID NO: 190
  engineered scaffold(mature form, having modified second region)

SEQ ID NO: 425 - RNA, 144 nt, Artificial Sequence; identical to SEQ ID NO: 191
  engineered scaffold(mature form, having modified second region)

SEQ ID NO: 426 - RNA, 146 nt, Artificial Sequence; identical to SEQ ID NO: 192
  engineered scaffold(mature form, having modified second region)

SEQ ID NO: 427 - RNA, 148 nt, Artificial Sequence; identical to SEQ ID NO: 193
  engineered scaffold(mature form, having modified second region)

SEQ ID NO: 428 - RNA, 150 nt, Artificial Sequence; identical to SEQ ID NO: 194
  engineered scaffold(mature form, having modified second region)

SEQ ID NO: 429 - RNA, 152 nt, Artificial Sequence; identical to SEQ ID NO: 195
  engineered scaffold(mature form, having modified second region)

SEQ ID NO: 430 - RNA, 153 nt, Artificial Sequence; identical to SEQ ID NO: 196
  engineered scaffold(mature form, having modified second region)

SEQ ID NO: 431 - RNA, 155 nt, Artificial Sequence; identical to SEQ ID NO: 197
  engineered scaffold(mature form, having modified second region)

SEQ ID NO: 432 - RNA, 157 nt, Artificial Sequence; identical to SEQ ID NO: 198
  engineered scaffold(mature form, having modified second region)

SEQ ID NO: 433 - RNA, 159 nt, Artificial Sequence; identical to SEQ ID NO: 199
  engineered scaffold(mature form, having modified second region)

SEQ ID NO: 434 - RNA, 55 nt, Artificial Sequence
  modified third region
gcugcuugcaucagccuaaugucgagaagugcuuucuucggaaaguaacccucga

SEQ ID NO: 435 - RNA, 53 nt, Artificial Sequence
  modified third region
gcugcuugcaucagccuaaugucgagaagugcuuuuucgaaaguaacccucga

SEQ ID NO: 436 - RNA, 51 nt, Artificial Sequence
  modified third region
gcugcuugcaucagccuaaugucgagaagugcuuuucgaaguaacccucga

SEQ ID NO: 437 - RNA, 51 nt, Artificial Sequence
  modified third region
gcugcuugcaucagccuaaugucgagaagugcucuucggaguaacccucga

SEQ ID NO: 438 - RNA, 49 nt, Artificial Sequence
  modified third region
gcugcuugcaucagccuaaugucgagaagugcuuucgaguaacccucga

SEQ ID NO: 439 - RNA, 47 nt, Artificial Sequence
  modified third region
gcugcuugcaucagccuaaugucgagaagugcuucgguaacccucga

SEQ ID NO: 440 - RNA, 45 nt, Artificial Sequence
  modified third region
gcugcuugcaucagccuaaugucgagaaguguucguaacccucga

SEQ ID NO: 441 - RNA, 43 nt, Artificial Sequence
  modified third region
gcugcuugcaucagccuaaugucgagaaguuucgaacccucga

SEQ ID NO: 442 - RNA, 41 nt, Artificial Sequence
  modified third region
gcugcuugcaucagccuaaugucgagaaguucgacccucga

SEQ ID NO: 443 - RNA, 40 nt, Artificial Sequence
  modified third region
gcugcuugcaucagccuaaugucgagaaguucgcccucga

SEQ ID NO: 444 - RNA, 39 nt, Artificial Sequence
  modified third region
gcugcuugcaucagccuaaugucgagaauucgcccucga

SEQ ID NO: 445 - RNA, 38 nt, Artificial Sequence
  modified third region
gcugcuugcaucagccuaaugucgagaauucgccucga

SEQ ID NO: 446 - RNA, 37 nt, Artificial Sequence
  modified third region
gcugcuugcaucagccuaaugucgagauucgccucga

SEQ ID NO: 447 - RNA, 35 nt, Artificial Sequence
  modified third region
gcugcuugcaucagccuaaugucgaguucgcucga

SEQ ID NO: 448 - RNA, 138 nt, Artificial Sequence
  engineered tracrRNA(mature form, having modified third region)
cuucacugauaaaguggagaaccgcuucaccaaaagcugucccuuaggggauuagaacuugagugaaggugggcugcuugcaucagccuaaugucgagaagugcuuuuucgaaaguaacccucgaaacaaauucauuu

SEQ ID NO: 449 - RNA, 136 nt, Artificial Sequence
  engineered tracrRNA(mature form, having modified third region)
cuucacugauaaaguggagaaccgcuucaccaaaagcugucccuuaggggauuagaacuugagugaaggugggcugcuugcaucagccuaaugucgagaagugcuuuucgaaguaacccucgaaacaaauucauuu

SEQ ID NO: 450 - RNA, 136 nt, Artificial Sequence
  engineered tracrRNA(mature form, having modified third region)
cuucacugauaaaguggagaaccgcuucaccaaaagcugucccuuaggggauuagaacuugagugaaggugggcugcuugcaucagccuaaugucgagaagugcucuucggaguaacccucgaaacaaauucauuu

SEQ ID NO: 451 - RNA, 134 nt, Artificial Sequence
  engineered tracrRNA(mature form, having modified third region)
cuucacugauaaaguggagaaccgcuucaccaaaagcugucccuuaggggauuagaacuugagugaaggugggcugcuugcaucagccuaaugucgagaagugcuuucgaguaacccucgaaacaaauucauuu

SEQ ID NO: 452 - RNA, 132 nt, Artificial Sequence
  engineered tracrRNA(mature form, having modified third region)
cuucacugauaaaguggagaaccgcuucaccaaaagcugucccuuaggggauuagaacuugagugaaggugggcugcuugcaucagccuaaugucgagaagugcuucgguaacccucgaaacaaauucauuu

SEQ ID NO: 453 - RNA, 130 nt, Artificial Sequence
  engineered tracrRNA(mature form, having modified third region)
cuucacugauaaaguggagaaccgcuucaccaaaagcugucccuuaggggauuagaacuugagugaaggugggcugcuugcaucagccuaaugucgagaaguguucguaacccucgaaacaaauucauuu

SEQ ID NO: 454 - RNA, 128 nt, Artificial Sequence
  engineered tracrRNA(mature form, having modified third region)
cuucacugauaaaguggagaaccgcuucaccaaaagcugucccuuaggggauuagaacuugagugaaggugggcugcuugcaucagccuaaugucgagaaguuucgaacccucgaaacaaauucauuu

SEQ ID NO: 455 - RNA, 126 nt, Artificial Sequence
  engineered tracrRNA(mature form, having modified third region)
cuucacugauaaaguggagaaccgcuucaccaaaagcugucccuuaggggauuagaacuugagugaaggugggcugcuugcaucagccuaaugucgagaaguucgacccucgaaacaaauucauuu

SEQ ID NO: 456 - RNA, 125 nt, Artificial Sequence
  engineered tracrRNA(mature form, having modified third region)
cuucacugauaaaguggagaaccgcuucaccaaaagcugucccuuaggggauuagaacuugagugaaggugggcugcuugcaucagccuaaugucgagaaguucgcccucgaaacaaauucauuu

SEQ ID NO: 457 - RNA, 124 nt, Artificial Sequence
  engineered tracrRNA(mature form, having modified third region)
cuucacugauaaaguggagaaccgcuucaccaaaagcugucccuuaggggauuagaacuugagugaaggugggcugcuugcaucagccuaaugucgagaauucgcccucgaaacaaauucauuu

SEQ ID NO: 458 - RNA, 123 nt, Artificial Sequence
  engineered tracrRNA(mature form, having modified third region)
cuucacugauaaaguggagaaccgcuucaccaaaagcugucccuuaggggauuagaacuugagugaaggugggcugcuugcaucagccuaaugucgagaauucgccucgaaacaaauucauuu

SEQ ID NO: 459 - RNA, 122 nt, Artificial Sequence
  engineered tracrRNA(mature form, having modified third region)
cuucacugauaaaguggagaaccgcuucaccaaaagcugucccuuaggggauuagaacuugagugaaggugggcugcuugcaucagccuaaugucgagauucgccucgaaacaaauucauuu

SEQ ID NO: 460 - RNA, 120 nt, Artificial Sequence
  engineered tracrRNA(mature form, having modified third region)
cuucacugauaaaguggagaaccgcuucaccaaaagcugucccuuaggggauuagaacuugagugaaggugggcugcuugcaucagccuaaugucgaguucgcucgaaacaaauucauuu

SEQ ID NO: 461 - RNA, 161 nt, Artificial Sequence; identical to SEQ ID NO: 7
  engineered scaffold(mature form, having modified third region)

SEQ ID NO: 462 - RNA, 159 nt, Artificial Sequence
  engineered scaffold(mature form, having modified third region)
cuucacugauaaaguggagaaccgcuucaccaaaagcugucccuuaggggauuagaacuugagugaaggugggcugcuugcaucagccuaaugucgagaagugcuuuuucgaaaguaacccucgaaacaaauucauuugaaagaaugaaggaaugcaac

SEQ ID NO: 463 - RNA, 157 nt, Artificial Sequence
  engineered scaffold(mature form, having modified third region)
cuucacugauaaaguggagaaccgcuucaccaaaagcugucccuuaggggauuagaacuugagugaaggugggcugcuugcaucagccuaaugucgagaagugcuuuucgaaguaacccucgaaacaaauucauuugaaagaaugaaggaaugcaac

SEQ ID NO: 464 - RNA, 157 nt, Artificial Sequence
  engineered scaffold(mature form, having modified third region)
cuucacugauaaaguggagaaccgcuucaccaaaagcugucccuuaggggauuagaacuugagugaaggugggcugcuugcaucagccuaaugucgagaagugcucuucggaguaacccucgaaacaaauucauuugaaagaaugaaggaaugcaac

SEQ ID NO: 465 - RNA, 155 nt, Artificial Sequence
  engineered scaffold(mature form, having modified third region)
cuucacugauaaaguggagaaccgcuucaccaaaagcugucccuuaggggauuagaacuugagugaaggugggcugcuugcaucagccuaaugucgagaagugcuuucgaguaacccucgaaacaaauucauuugaaagaaugaaggaaugcaac

SEQ ID NO: 466 - RNA, 153 nt, Artificial Sequence
  engineered scaffold(mature form, having modified third region)
cuucacugauaaaguggagaaccgcuucaccaaaagcugucccuuaggggauuagaacuugagugaaggugggcugcuugcaucagccuaaugucgagaagugcuucgguaacccucgaaacaaauucauuugaaagaaugaaggaaugcaac

SEQ ID NO: 467 - RNA, 151 nt, Artificial Sequence
  engineered scaffold(mature form, having modified third region)
cuucacugauaaaguggagaaccgcuucaccaaaagcugucccuuaggggauuagaacuugagugaaggugggcugcuugcaucagccuaaugucgagaaguguucguaacccucgaaacaaauucauuugaaagaaugaaggaaugcaac

SEQ ID NO: 468 - RNA, 149 nt, Artificial Sequence
  engineered scaffold(mature form, having modified third region)
cuucacugauaaaguggagaaccgcuucaccaaaagcugucccuuaggggauuagaacuugagugaaggugggcugcuugcaucagccuaaugucgagaaguuucgaacccucgaaacaaauucauuugaaagaaugaaggaaugcaac

SEQ ID NO: 469 - RNA, 147 nt, Artificial Sequence
  engineered scaffold(mature form, having modified third region)
cuucacugauaaaguggagaaccgcuucaccaaaagcugucccuuaggggauuagaacuugagugaaggugggcugcuugcaucagccuaaugucgagaaguucgacccucgaaacaaauucauuugaaagaaugaaggaaugcaac

SEQ ID NO: 470 - RNA, 146 nt, Artificial Sequence
  engineered scaffold(mature form, having modified third region)
cuucacugauaaaguggagaaccgcuucaccaaaagcugucccuuaggggauuagaacuugagugaaggugggcugcuugcaucagccuaaugucgagaaguucgcccucgaaacaaauucauuugaaagaaugaaggaaugcaac

SEQ ID NO: 471 - RNA, 145 nt, Artificial Sequence
  engineered scaffold(mature form, having modified third region)
cuucacugauaaaguggagaaccgcuucaccaaaagcugucccuuaggggauuagaacuugagugaaggugggcugcuugcaucagccuaaugucgagaauucgcccucgaaacaaauucauuugaaagaaugaaggaaugcaac

SEQ ID NO: 472 - RNA, 144 nt, Artificial Sequence
  engineered scaffold(mature form, having modified third region)
cuucacugauaaaguggagaaccgcuucaccaaaagcugucccuuaggggauuagaacuugagugaaggugggcugcuugcaucagccuaaugucgagaauucgccucgaaacaaauucauuugaaagaaugaaggaaugcaac

SEQ ID NO: 473 - RNA, 143 nt, Artificial Sequence
  engineered scaffold(mature form, having modified third region)
cuucacugauaaaguggagaaccgcuucaccaaaagcugucccuuaggggauuagaacuugagugaaggugggcugcuugcaucagccuaaugucgagauucgccucgaaacaaauucauuugaaagaaugaaggaaugcaac

SEQ ID NO: 474 - RNA, 141 nt, Artificial Sequence
  engineered scaffold(mature form, having modified third region)
cuucacugauaaaguggagaaccgcuucaccaaaagcugucccuuaggggauuagaacuugagugaaggugggcugcuugcaucagccuaaugucgaguucgcucgaaacaaauucauuugaaagaaugaaggaaugcaac

SEQ ID NO: 475 - RNA, 26 nt, Artificial Sequence
  476%intermediate sequence of modified third region
gcugcuugcaucagccuaaugucgag

SEQ ID NO: 476 - RNA, 10 nt, Artificial Sequence
  intermediate sequence of modified third region
aaguucgacc

SEQ ID NO: 477 - RNA, 12 nt, Artificial Sequence
  intermediate sequence of modified third region
aaguuucgaacc

SEQ ID NO: 478 - RNA, 14 nt, Artificial Sequence
  intermediate sequence of modified third region
aaguguucguaacc

SEQ ID NO: 479 - RNA, 16 nt, Artificial Sequence
  intermediate sequence of modified third region
aagugcuucgguaacc

SEQ ID NO: 480 - RNA, 18 nt, Artificial Sequence
  intermediate sequence of modified third region
aagugcuuucgaguaacc

SEQ ID NO: 481 - RNA, 20 nt, Artificial Sequence
  intermediate sequence of modified third region
aagugcucuucggaguaacc

SEQ ID NO: 482 - RNA, 20 nt, Artificial Sequence
  intermediate sequence of modified third region
aagugcuuuucgaaguaacc

SEQ ID NO: 483 - RNA, 22 nt, Artificial Sequence
  intermediate sequence of modified third region
aagugcuuuuucgaaaguaacc

SEQ ID NO: 484 - RNA, 24 nt, Artificial Sequence
  intermediate sequence of modified third region
aagugcuuucuucggaaaguaacc

SEQ ID NO: 485 - RNA, 10 nt, Artificial Sequence
  deleted part of modified third region, upper stream
aagugcuuuc

SEQ ID NO: 486 - RNA, 10 nt, Artificial Sequence
  deleted part of modified third region, lower stream
gaaaguaacc

SEQ ID NO: 487 - RNA, 140 nt, Artificial Sequence
  engineered scaffold(mature form, the first region is deleted)
ccgcuucaccaaaagcugucccuuaggggauuagaacuugagugaaggugggcugcuugcaucagccuaaugucgagaagugcuuucuucggaaaguaacccucgaaacaaauucauuugaaagaaugaaggaaugcaac

SEQ ID NO: 488 - RNA, 125 nt, Artificial Sequence
  Example 2.1.1
accgcuucauuaggaaggugggcugcuugcaucagccuaaugucgagaagugcuuucuucggaaaguaacccucgaaacaaagaaaggaaugcaaccacacacacagugggcuaccuuuuauuuu

SEQ ID NO: 489 - RNA, 126 nt, Artificial Sequence
  Example 2.1.2
accgcuucauuagugaaggugggcugcuugcaucagccuaaugucgagaagugcuuucuucggaaaguaacccucgaaacaaagaaaggaaugcaaccacacacacagugggcuaccuuuuauuuu

SEQ ID NO: 490 - RNA, 128 nt, Artificial Sequence
  Example 2.1.3
accgcuucacuuaggugaaggugggcugcuugcaucagccuaaugucgagaagugcuuucuucggaaaguaacccucgaaacaaagaaaggaaugcaaccacacacacagugggcuaccuuuuauuuu

SEQ ID NO: 491 - RNA, 129 nt, Artificial Sequence
  Example 2.1.4
accgcuucacuuagagugaaggugggcugcuugcaucagccuaaugucgagaagugcuuucuucggaaaguaacccucgaaacaaagaaaggaaugcaaccacacacacagugggcuaccuuuuauuuu

SEQ ID NO: 492 - RNA, 131 nt, Artificial Sequence
  Example 2.1.5
accgcuucaccuuaggagugaaggugggcugcuugcaucagccuaaugucgagaagugcuuucuucggaaaguaacccucgaaacaaagaaaggaaugcaaccacacacacagugggcuaccuuuuauuuu

SEQ ID NO: 493 - RNA, 135 nt, Artificial Sequence
  Example 2.1.6
accgcuucaccaauuaguugagugaaggugggcugcuugcaucagccuaaugucgagaagugcuuucuucggaaaguaacccucgaaacaaagaaaggaaugcaaccacacacacagugggcuaccuuuuauuuu

SEQ ID NO: 494 - RNA, 137 nt, Artificial Sequence
  Example 2.1.7
accgcuucaccaaauuagcuugagugaaggugggcugcuugcaucagccuaaugucgagaagugcuuucuucggaaaguaacccucgaaacaaagaaaggaaugcaaccacacacacagugggcuaccuuuuauuuu

SEQ ID NO: 495 - RNA, 139 nt, Artificial Sequence
  Example 2.1.8
accgcuucaccaaaauuagacuugagugaaggugggcugcuugcaucagccuaaugucgagaagugcuuucuucggaaaguaacccucgaaacaaagaaaggaaugcaaccacacacacagugggcuaccuuuuauuuu

SEQ ID NO: 496 - RNA, 141 nt, Artificial Sequence
  Example 2.1.9
accgcuucaccaaaaguuagaacuugagugaaggugggcugcuugcaucagccuaaugucgagaagugcuuucuucggaaaguaacccucgaaacaaagaaaggaaugcaaccacacacacagugggcuaccuuuuauuuu

SEQ ID NO: 497 - RNA, 143 nt, Artificial Sequence
  Example 2.1.10
accgcuucaccaaaagcuuaggaacuugagugaaggugggcugcuugcaucagccuaaugucgagaagugcuuucuucggaaaguaacccucgaaacaaagaaaggaaugcaaccacacacacagugggcuaccuuuuauuuu

SEQ ID NO: 498 - RNA, 145 nt, Artificial Sequence
  Example 2.1.11
accgcuucaccaaaagcuuuagagaacuugagugaaggugggcugcuugcaucagccuaaugucgagaagugcuuucuucggaaaguaacccucgaaacaaagaaaggaaugcaaccacacacacagugggcuaccuuuuauuuu

SEQ ID NO: 499 - RNA, 147 nt, Artificial Sequence
  Example 2.1.12
accgcuucaccaaaagcuuuaguuagaacuugagugaaggugggcugcuugcaucagccuaaugucgagaagugcuuucuucggaaaguaacccucgaaacaaagaaaggaaugcaaccacacacacagugggcuaccuuuuauuuu

SEQ ID NO: 500 - RNA, 150 nt, Artificial Sequence
  Example 2.1.13
accgcuucaccaaaagcuguuuagauuagaacuugagugaaggugggcugcuugcaucagccuaaugucgagaagugcuuucuucggaaaguaacccucgaaacaaagaaaggaaugcaaccacacacacagugggcuaccuuuuauuuu

SEQ ID NO: 501 - RNA, 152 nt, Artificial Sequence
  Example 2.1.14
accgcuucaccaaaagcugucuuaggauuagaacuugagugaaggugggcugcuugcaucagccuaaugucgagaagugcuuucuucggaaaguaacccucgaaacaaagaaaggaaugcaaccacacacacagugggcuaccuuuuauuuu

SEQ ID NO: 502 - RNA, 156 nt, Artificial Sequence; identical to SEQ ID NO: 306
  Example 2.1.15

SEQ ID NO: 503 - RNA, 125 nt, Artificial Sequence
  Example 2.2.1
accgcuucauuaggaaggugggcugcuugcaucagccuaaugucgagaagugcuuucuucggaaaguaacccucgaaacaaagaaaggaaugcaaccauccccaggacacacacacuuuuauuuu

SEQ ID NO: 504 - RNA, 126 nt, Artificial Sequence
  Example 2.2.2
accgcuucauuagugaaggugggcugcuugcaucagccuaaugucgagaagugcuuucuucggaaaguaacccucgaaacaaagaaaggaaugcaaccauccccaggacacacacacuuuuauuuu

SEQ ID NO: 505 - RNA, 128 nt, Artificial Sequence
  Example 2.2.3
accgcuucacuuaggugaaggugggcugcuugcaucagccuaaugucgagaagugcuuucuucggaaaguaacccucgaaacaaagaaaggaaugcaaccauccccaggacacacacacuuuuauuuu

SEQ ID NO: 506 - RNA, 129 nt, Artificial Sequence
  Example 2.2.4
accgcuucacuuagagugaaggugggcugcuugcaucagccuaaugucgagaagugcuuucuucggaaaguaacccucgaaacaaagaaaggaaugcaaccauccccaggacacacacacuuuuauuuu

SEQ ID NO: 507 - RNA, 131 nt, Artificial Sequence
  Example 2.2.5
accgcuucaccuuaggagugaaggugggcugcuugcaucagccuaaugucgagaagugcuuucuucggaaaguaacccucgaaacaaagaaaggaaugcaaccauccccaggacacacacacuuuuauuuu

SEQ ID NO: 508 - RNA, 135 nt, Artificial Sequence
  Example 2.2.6
accgcuucaccaauuaguugagugaaggugggcugcuugcaucagccuaaugucgagaagugcuuucuucggaaaguaacccucgaaacaaagaaaggaaugcaaccauccccaggacacacacacuuuuauuuu

SEQ ID NO: 509 - RNA, 137 nt, Artificial Sequence
  Example 2.2.7
accgcuucaccaaauuagcuugagugaaggugggcugcuugcaucagccuaaugucgagaagugcuuucuucggaaaguaacccucgaaacaaagaaaggaaugcaaccauccccaggacacacacacuuuuauuuu

SEQ ID NO: 510 - RNA, 139 nt, Artificial Sequence
  Example 2.2.8
accgcuucaccaaaauuagacuugagugaaggugggcugcuugcaucagccuaaugucgagaagugcuuucuucggaaaguaacccucgaaacaaagaaaggaaugcaaccauccccaggacacacacacuuuuauuuu

SEQ ID NO: 511 - RNA, 141 nt, Artificial Sequence
  Example 2.2.9
accgcuucaccaaaaguuagaacuugagugaaggugggcugcuugcaucagccuaaugucgagaagugcuuucuucggaaaguaacccucgaaacaaagaaaggaaugcaaccauccccaggacacacacacuuuuauuuu

SEQ ID NO: 512 - RNA, 143 nt, Artificial Sequence
  Example 2.2.10
accgcuucaccaaaagcuuaggaacuugagugaaggugggcugcuugcaucagccuaaugucgagaagugcuuucuucggaaaguaacccucgaaacaaagaaaggaaugcaaccauccccaggacacacacacuuuuauuuu

SEQ ID NO: 513 - RNA, 145 nt, Artificial Sequence
  Example 2.2.11
accgcuucaccaaaagcuuuagagaacuugagugaaggugggcugcuugcaucagccuaaugucgagaagugcuuucuucggaaaguaacccucgaaacaaagaaaggaaugcaaccauccccaggacacacacacuuuuauuuu

SEQ ID NO: 514 - RNA, 147 nt, Artificial Sequence
  Example 2.2.12
accgcuucaccaaaagcuuuaguuagaacuugagugaaggugggcugcuugcaucagccuaaugucgagaagugcuuucuucggaaaguaacccucgaaacaaagaaaggaaugcaaccauccccaggacacacacacuuuuauuuu

SEQ ID NO: 515 - RNA, 150 nt, Artificial Sequence
  Example 2.2.13
accgcuucaccaaaagcuguuuagauuagaacuugagugaaggugggcugcuugcaucagccuaaugucgagaagugcuuucuucggaaaguaacccucgaaacaaagaaaggaaugcaaccauccccaggacacacacacuuuuauuuu

SEQ ID NO: 516 - RNA, 152 nt, Artificial Sequence
  Example 2.2.14
accgcuucaccaaaagcugucuuaggauuagaacuugagugaaggugggcugcuugcaucagccuaaugucgagaagugcuuucuucggaaaguaacccucgaaacaaagaaaggaaugcaaccauccccaggacacacacacuuuuauuuu

SEQ ID NO: 517 - RNA, 156 nt, Artificial Sequence; identical to SEQ ID NO: 321
  Example 2.2.15

SEQ ID NO: 518 - RNA, 122 nt, Artificial Sequence
  Example 3.1.1
accgcuuuuagaaggugggcugcuugcaucagccuaaugucgagaagugcuuucuucggaaaguaacccucgaaacaaagaaaggaaugcaaccacacacacagugggcuaccuuuuauuuu

SEQ ID NO: 519 - RNA, 120 nt, Artificial Sequence
  Example 3.1.2
accgcuuuagaggugggcugcuugcaucagccuaaugucgagaagugcuuucuucggaaaguaacccucgaaacaaagaaaggaaugcaaccacacacacagugggcuaccuuuuauuuu

SEQ ID NO: 520 - RNA, 119 nt, Artificial Sequence
  Example 3.1.3
accgcuuaguggugggcugcuugcaucagccuaaugucgagaagugcuuucuucggaaaguaacccucgaaacaaagaaaggaaugcaaccacacacacagugggcuaccuuuuauuuu

SEQ ID NO: 521 - RNA, 116 nt, Artificial Sequence
  Example 3.1.4
accguuaggugggcugcuugcaucagccuaaugucgagaagugcuuucuucggaaaguaacccucgaaacaaagaaaggaaugcaaccacacacacagugggcuaccuuuuauuuu

SEQ ID NO: 522 - RNA, 115 nt, Artificial Sequence
  Example 3.1.5
accuuaggugggcugcuugcaucagccuaaugucgagaagugcuuucuucggaaaguaacccucgaaacaaagaaaggaaugcaaccacacacacagugggcuaccuuuuauuuu

SEQ ID NO: 523 - RNA, 113 nt, Artificial Sequence
  Example 3.1.6
acuuagugggcugcuugcaucagccuaaugucgagaagugcuuucuucggaaaguaacccucgaaacaaagaaaggaaugcaaccacacacacagugggcuaccuuuuauuuu

SEQ ID NO: 524 - RNA, 112 nt, Artificial Sequence
  Example 3.1.7
acuuaggggcugcuugcaucagccuaaugucgagaagugcuuucuucggaaaguaacccucgaaacaaagaaaggaaugcaaccacacacacagugggcuaccuuuuauuuu

SEQ ID NO: 525 - RNA, 110 nt, Artificial Sequence
  Example 3.1.8
auuagggcugcuugcaucagccuaaugucgagaagugcuuucuucggaaaguaacccucgaaacaaagaaaggaaugcaaccacacacacagugggcuaccuuuuauuuu

SEQ ID NO: 526 - RNA, 106 nt, Artificial Sequence
  Example 3.1.9
aggcugcuugcaucagccuaaugucgagaagugcuuucuucggaaaguaacccucgaaacaaagaaaggaaugcaaccacacacacagugggcuaccuuuuauuuu

SEQ ID NO: 527 - RNA, 104 nt, Artificial Sequence
  Example 3.1.10
gcugcuugcaucagccuaaugucgagaagugcuuucuucggaaaguaacccucgaaacaaagaaaggaaugcaaccacacacacagugggcuaccuuuuauuuu

SEQ ID NO: 528 - RNA, 129 nt, Artificial Sequence; identical to SEQ ID NO: 491
  Example 3.1.11

SEQ ID NO: 529 - RNA, 156 nt, Artificial Sequence; identical to SEQ ID NO: 306
  Example 3.1.12

SEQ ID NO: 530 - RNA, 122 nt, Artificial Sequence
  Example 3.2.1
accgcuuuuagaaggugggcugcuugcaucagccuaaugucgagaagugcuuucuucggaaaguaacccucgaaacaaagaaaggaaugcaaccauccccaggacacacacacuuuuauuuu

SEQ ID NO: 531 - RNA, 120 nt, Artificial Sequence
  Example 3.2.2
accgcuuuagaggugggcugcuugcaucagccuaaugucgagaagugcuuucuucggaaaguaacccucgaaacaaagaaaggaaugcaaccauccccaggacacacacacuuuuauuuu

SEQ ID NO: 532 - RNA, 119 nt, Artificial Sequence
  Example 3.2.3
accgcuuaguggugggcugcuugcaucagccuaaugucgagaagugcuuucuucggaaaguaacccucgaaacaaagaaaggaaugcaaccauccccaggacacacacacuuuuauuuu

SEQ ID NO: 533 - RNA, 116 nt, Artificial Sequence
  Example 3.2.4
accguuaggugggcugcuugcaucagccuaaugucgagaagugcuuucuucggaaaguaacccucgaaacaaagaaaggaaugcaaccauccccaggacacacacacuuuuauuuu

SEQ ID NO: 534 - RNA, 115 nt, Artificial Sequence
  Example 3.2.5
accuuaggugggcugcuugcaucagccuaaugucgagaagugcuuucuucggaaaguaacccucgaaacaaagaaaggaaugcaaccauccccaggacacacacacuuuuauuuu

SEQ ID NO: 535 - RNA, 113 nt, Artificial Sequence
  Example 3.2.6
acuuagugggcugcuugcaucagccuaaugucgagaagugcuuucuucggaaaguaacccucgaaacaaagaaaggaaugcaaccauccccaggacacacacacuuuuauuuu

SEQ ID NO: 536 - RNA, 112 nt, Artificial Sequence
  Example 3.2.7
acuuaggggcugcuugcaucagccuaaugucgagaagugcuuucuucggaaaguaacccucgaaacaaagaaaggaaugcaaccauccccaggacacacacacuuuuauuuu

SEQ ID NO: 537 - RNA, 110 nt, Artificial Sequence
  Example 3.2.8
auuagggcugcuugcaucagccuaaugucgagaagugcuuucuucggaaaguaacccucgaaacaaagaaaggaaugcaaccauccccaggacacacacacuuuuauuuu

SEQ ID NO: 538 - RNA, 106 nt, Artificial Sequence
  Example 3.2.9
aggcugcuugcaucagccuaaugucgagaagugcuuucuucggaaaguaacccucgaaacaaagaaaggaaugcaaccauccccaggacacacacacuuuuauuuu

SEQ ID NO: 539 - RNA, 104 nt, Artificial Sequence
  Example 3.2.10
gcugcuugcaucagccuaaugucgagaagugcuuucuucggaaaguaacccucgaaacaaagaaaggaaugcaaccauccccaggacacacacacuuuuauuuu

SEQ ID NO: 540 - RNA, 129 nt, Artificial Sequence; identical to SEQ ID NO: 506
  Example 3.2.11

SEQ ID NO: 541 - RNA, 156 nt, Artificial Sequence; identical to SEQ ID NO: 321
  Example 3.2.12

SEQ ID NO: 542 - DNA, 20 bp, Artificial Sequence
  protospacer sequence for targeting FUS
gtgggtaggtccagtttggg

SEQ ID NO: 543 - DNA, 20 bp, Artificial Sequence
  protospacer sequence for targeting GAK
cagagtcccgggaacaagcc

SEQ ID NO: 544 - DNA, 20 bp, Artificial Sequence
  protospacer sequence for targeting MLH
agggaatgaaagtgaagatg

SEQ ID NO: 545 - RNA, 129 nt, Artificial Sequence
  Example 4.4.1
accgcuucaccauuagugagugaaggugggcugcuugcaucagccuaaugucgagaagugcucuucggaguaacccucgaaacaaagaaaggaaugcaacguggguagguccaguuuggguuuuauuuu

SEQ ID NO: 546 - RNA, 123 nt, Artificial Sequence
  Example 4.4.2
accgcuucaccauuagugagugaaggugggcugcuugcaucagccuaaugucgagaaguguucguaacccucgaaacaaagaaaggaaugcaacguggguagguccaguuuggguuuuauuuu

SEQ ID NO: 547 - RNA, 118 nt, Artificial Sequence
  Example 4.4.3
accgcuucaccauuagugagugaaggugggcugcuugcaucagccuaaugucgagaaguucgcccucgaaacaaagaaaggaaugcaacguggguagguccaguuuggguuuuauuuu

SEQ ID NO: 548 - RNA, 113 nt, Artificial Sequence
  Example 4.4.4
accgcuucaccauuagugagugaaggugggcugcuugcaucagccuaaugucgaguucgcucgaaacaaagaaaggaaugcaacguggguagguccaguuuggguuuuauuuu

SEQ ID NO: 549 - RNA, 129 nt, Artificial Sequence
  Example 4.5.1
accgcuucaccauuagugagugaaggugggcugcuugcaucagccuaaugucgagaagugcucuucggaguaacccucgaaacaaagaaaggaaugcaaccagagucccgggaacaagccuuuuauuuu

SEQ ID NO: 550 - RNA, 123 nt, Artificial Sequence
  Example 4.5.2
accgcuucaccauuagugagugaaggugggcugcuugcaucagccuaaugucgagaaguguucguaacccucgaaacaaagaaaggaaugcaaccagagucccgggaacaagccuuuuauuuu

SEQ ID NO: 551 - RNA, 129 nt, Artificial Sequence
  Example 4.6.1
accgcuucaccauuagugagugaaggugggcugcuugcaucagccuaaugucgagaagugcucuucggaguaacccucgaaacaaagaaaggaaugcaacagggaaugaaagugaagauguuuuauuuu

SEQ ID NO: 552 - DNA, 20 bp, Artificial Sequence
  protospacer sequence for targeting AHRR
ccttaataaagtataacttc

SEQ ID NO: 553 - DNA, 20 bp, Artificial Sequence
  protospacer sequence for targeting APEX1
aagaaggaatggtagttgag

SEQ ID NO: 554 - DNA, 20 bp, Artificial Sequence
  protospacer sequence for targeting BCL2L13
atttccaagtcaaccttatg

SEQ ID NO: 555 - DNA, 20 bp, Artificial Sequence
  protospacer sequence for targeting CARS
caacagcctcaccaggaaca

SEQ ID NO: 556 - DNA, 20 bp, Artificial Sequence
  protospacer sequence for targeting CCDC127
ggcaagggtcttgatgcatc

SEQ ID NO: 557 - DNA, 20 bp, Artificial Sequence
  protospacer sequence for targeting CLIC4
ccctggctacctcccctacc

SEQ ID NO: 558 - DNA, 20 bp, Artificial Sequence
  protospacer sequence for targeting COL8A1-1
gattcattctcagtgccatg

SEQ ID NO: 559 - DNA, 20 bp, Artificial Sequence
  protospacer sequence for targeting COL8A1-2
aggcaattgcaaccactgaa

SEQ ID NO: 560 - DNA, 20 bp, Artificial Sequence
  protospacer sequence for targeting EMX1
tactttgtcctccggttctg

SEQ ID NO: 561 - DNA, 20 bp, Artificial Sequence
  protospacer sequence for targeting FANCF-1
ggttctctctatagccattg

SEQ ID NO: 562 - DNA, 20 bp, Artificial Sequence
  protospacer sequence for targeting FANCF-2
actttagtgactagccgcca

SEQ ID NO: 563 - DNA, 20 bp, Artificial Sequence
  protospacer sequence for targeting FUS-1
gtgggtaggtccagtttggg

SEQ ID NO: 564 - DNA, 20 bp, Artificial Sequence
  protospacer sequence for targeting FUS-2
acaaagaaaccagcagtggc

SEQ ID NO: 565 - DNA, 20 bp, Artificial Sequence
  protospacer sequence for targeting GAB4
cctggtggctgagaccaggg

SEQ ID NO: 566 - DNA, 20 bp, Artificial Sequence
  protospacer sequence for targeting GAK
cagagtcccgggaacaagcc

SEQ ID NO: 567 - DNA, 20 bp, Artificial Sequence
  protospacer sequence for targeting HBB
ccaaagtgatgggccagcac

SEQ ID NO: 568 - DNA, 20 bp, Artificial Sequence
  protospacer sequence for targeting INIP
agagcagcgattgtaaggag

SEQ ID NO: 569 - DNA, 20 bp, Artificial Sequence
  protospacer sequence for targeting intergenic-01
gaaatatgactggaagtaaa

SEQ ID NO: 570 - DNA, 20 bp, Artificial Sequence
  protospacer sequence for targeting intergenic-02
cttccagtcatatttctaaa

SEQ ID NO: 571 - DNA, 20 bp, Artificial Sequence
  protospacer sequence for targeting intergenic-03
cccttattacaatcctgtgg

SEQ ID NO: 572 - DNA, 20 bp, Artificial Sequence
  protospacer sequence for targeting intergenic-04
cccccacaggattgtaataa

SEQ ID NO: 573 - DNA, 20 bp, Artificial Sequence
  protospacer sequence for targeting intergenic-05
atctccataacaatctttgg

SEQ ID NO: 574 - DNA, 20 bp, Artificial Sequence
  protospacer sequence for targeting intergenic-06
ctatccccattttacagatg

SEQ ID NO: 575 - DNA, 20 bp, Artificial Sequence
  protospacer sequence for targeting intergenic-07
ctgagatttgcgaagagtta

SEQ ID NO: 576 - DNA, 20 bp, Artificial Sequence
  protospacer sequence for targeting intergenic-08
attaaatagagtcttttgaa

SEQ ID NO: 577 - DNA, 20 bp, Artificial Sequence
  protospacer sequence for targeting intergenic-09
atattaattgcaagtttggg

SEQ ID NO: 578 - DNA, 20 bp, Artificial Sequence
  protospacer sequence for targeting intergenic-10
ggccaagtgcgaagtcagag

SEQ ID NO: 579 - DNA, 20 bp, Artificial Sequence
  protospacer sequence for targeting intergenic-11
ggggtgaacacccaagatcc

SEQ ID NO: 580 - DNA, 20 bp, Artificial Sequence
  protospacer sequence for targeting intergenic-12
gggtgggctcctggcagggc

SEQ ID NO: 581 - DNA, 20 bp, Artificial Sequence
  protospacer sequence for targeting intergenic-13
agaagcatgcaaaaccggca

SEQ ID NO: 582 - DNA, 20 bp, Artificial Sequence
  protospacer sequence for targeting intergenic-14
aagaggggaggttgactttg

SEQ ID NO: 583 - DNA, 20 bp, Artificial Sequence
  protospacer sequence for targeting intergenic-15
gtcaaataaagaaaaatacg

SEQ ID NO: 584 - DNA, 20 bp, Artificial Sequence
  protospacer sequence for targeting intergenic-16
atgcatctcagtggttaaca

SEQ ID NO: 585 - DNA, 20 bp, Artificial Sequence
  protospacer sequence for targeting intergenic-17
catacagggctctgtaccca

SEQ ID NO: 586 - DNA, 20 bp, Artificial Sequence
  protospacer sequence for targeting intergenic-18
caaagacactcaccctgttg

SEQ ID NO: 587 - DNA, 20 bp, Artificial Sequence
  protospacer sequence for targeting intergenic-19
agaacacatacccctgggcc

SEQ ID NO: 588 - DNA, 20 bp, Artificial Sequence
  protospacer sequence for targeting intergenic-20
ataataaaagtatttcctca

SEQ ID NO: 589 - DNA, 20 bp, Artificial Sequence
  protospacer sequence for targeting intergenic-21
agccgtggtcagtgagaggc

SEQ ID NO: 590 - DNA, 20 bp, Artificial Sequence
  protospacer sequence for targeting intergenic-22
gagctcattagcttggggag

SEQ ID NO: 591 - DNA, 20 bp, Artificial Sequence
  protospacer sequence for targeting intergenic-23
gaaaataactaaacttccca

SEQ ID NO: 592 - DNA, 20 bp, Artificial Sequence
  protospacer sequence for targeting intergenic-24
aattctttaagtaatttaag

SEQ ID NO: 593 - DNA, 20 bp, Artificial Sequence
  protospacer sequence for targeting intergenic-25
cttagtagtctcagaaccaa

SEQ ID NO: 594 - DNA, 20 bp, Artificial Sequence
  protospacer sequence for targeting intergenic-26
aaaggagcacaagtacaaac

SEQ ID NO: 595 - DNA, 20 bp, Artificial Sequence
  protospacer sequence for targeting intergenic-27
aatgatgcagtaatcgtgta

SEQ ID NO: 596 - DNA, 20 bp, Artificial Sequence
  protospacer sequence for targeting intergenic-28
ataaaaggaactatttacaa

SEQ ID NO: 597 - DNA, 20 bp, Artificial Sequence
  protospacer sequence for targeting KLHL29
gagagaccgctcaggctgga

SEQ ID NO: 598 - DNA, 20 bp, Artificial Sequence
  protospacer sequence for targeting LINC01551-1
attttgaagtgaccgtacga

SEQ ID NO: 599 - DNA, 20 bp, Artificial Sequence
  protospacer sequence for targeting LINC01551-2
ataatacactctttacactg

SEQ ID NO: 600 - DNA, 20 bp, Artificial Sequence
  protospacer sequence for targeting LOC100128398-1
aagagttattgtcaatagaa

SEQ ID NO: 601 - DNA, 20 bp, Artificial Sequence
  protospacer sequence for targeting LOC100128398-2
caaagaaatgtactgcctta

SEQ ID NO: 602 - DNA, 20 bp, Artificial Sequence
  protospacer sequence for targeting LOC100130876
aaataaccgtcggtttctta

SEQ ID NO: 603 - DNA, 20 bp, Artificial Sequence
  protospacer sequence for targeting LOC101926886
caaacaaaataattggctca

SEQ ID NO: 604 - DNA, 20 bp, Artificial Sequence
  protospacer sequence for targeting LOC105369597
gccatggtgaaggtgaaatc

SEQ ID NO: 605 - DNA, 20 bp, Artificial Sequence
  protospacer sequence for targeting LOC105370393-1
gcagtacacctgagggaaca

SEQ ID NO: 606 - DNA, 20 bp, Artificial Sequence
  protospacer sequence for targeting LOC105370393-2
aagaaagctacaggaaagca

SEQ ID NO: 607 - DNA, 20 bp, Artificial Sequence
  protospacer sequence for targeting LOC105374431
ctttaaaatgaggtactagg

SEQ ID NO: 608 - DNA, 20 bp, Artificial Sequence
  protospacer sequence for targeting LOC105375122
ccaaccaggtaccctgtgcc

SEQ ID NO: 609 - DNA, 20 bp, Artificial Sequence
  protospacer sequence for targeting LOC105378763
attgaaacatatacgtggta

SEQ ID NO: 610 - DNA, 20 bp, Artificial Sequence
  protospacer sequence for targeting LOC107984132
ggaaagcgcagaaaagtaaa

SEQ ID NO: 611 - DNA, 20 bp, Artificial Sequence
  protospacer sequence for targeting MLH1-1
agggaatgaaagtgaagatg

SEQ ID NO: 612 - DNA, 20 bp, Artificial Sequence
  protospacer sequence for targeting MLH1-2
gatcaatttacatcaaacta

SEQ ID NO: 613 - DNA, 20 bp, Artificial Sequence
  protospacer sequence for targeting MRPL39
atttcacaggactttgttaa

SEQ ID NO: 614 - DNA, 20 bp, Artificial Sequence
  protospacer sequence for targeting NEK10-1
agacaagctgtcttccttca

SEQ ID NO: 615 - DNA, 20 bp, Artificial Sequence
  protospacer sequence for targeting NEK10-2
atctgaagatcattgaaaca

SEQ ID NO: 616 - DNA, 20 bp, Artificial Sequence
  protospacer sequence for targeting NLGN1
gtctaatagaaatatagtac

SEQ ID NO: 617 - DNA, 20 bp, Artificial Sequence
  protospacer sequence for targeting NLRC4-1
gagggagacacaagttgata

SEQ ID NO: 618 - DNA, 20 bp, Artificial Sequence
  protospacer sequence for targeting NLRC4-2
gtctcagtcttccttgtggg

SEQ ID NO: 619 - DNA, 20 bp, Artificial Sequence
  protospacer sequence for targeting NUDT16-1
ggggtagaggtactctacag

SEQ ID NO: 620 - DNA, 20 bp, Artificial Sequence
  protospacer sequence for targeting NUDT16-2
ggggtagaggtagtctacag

SEQ ID NO: 621 - DNA, 20 bp, Artificial Sequence
  protospacer sequence for targeting OR4K17
acaagttcagaatcacctta

SEQ ID NO: 622 - DNA, 20 bp, Artificial Sequence
  protospacer sequence for targeting OSBPL5
gcattaaggccagcgctggg

SEQ ID NO: 623 - DNA, 20 bp, Artificial Sequence
  protospacer sequence for targeting P2RX5-TAX1BP3
cacataggccattcagaaac

SEQ ID NO: 624 - DNA, 20 bp, Artificial Sequence
  protospacer sequence for targeting POLRMT-1
gaaactgccccaaaaccggc

SEQ ID NO: 625 - DNA, 20 bp, Artificial Sequence
  protospacer sequence for targeting POLRMT-2
aggactatgtgtggccagtg

SEQ ID NO: 626 - DNA, 20 bp, Artificial Sequence
  protospacer sequence for targeting PWAR5
aacaaatcactgactaacca

SEQ ID NO: 627 - DNA, 20 bp, Artificial Sequence
  protospacer sequence for targeting RMST
ataatgccttttaggtgata

SEQ ID NO: 628 - DNA, 20 bp, Artificial Sequence
  protospacer sequence for targeting RPH3AL-1
attttcaaaacagccctatg

SEQ ID NO: 629 - DNA, 20 bp, Artificial Sequence
  protospacer sequence for targeting RPH3AL-2
cacaagggatctgagacttg

SEQ ID NO: 630 - DNA, 20 bp, Artificial Sequence
  protospacer sequence for targeting RSPO4-1
actcatacatcacctcctcc

SEQ ID NO: 631 - DNA, 20 bp, Artificial Sequence
  protospacer sequence for targeting RSPO4-2
aaggaaaggcttcctggagg

SEQ ID NO: 632 - DNA, 20 bp, Artificial Sequence
  protospacer sequence for targeting RSRP1-1
atataggatttagaaaccaa

SEQ ID NO: 633 - DNA, 20 bp, Artificial Sequence
  protospacer sequence for targeting RSRP1-2
gctctaatgtaagtatatcc

SEQ ID NO: 634 - DNA, 20 bp, Artificial Sequence
  protospacer sequence for targeting TYW1B
gatccgatgcaattttggga

SEQ ID NO: 635 - DNA, 20 bp, Artificial Sequence
  protospacer sequence for targeting UNCX
cctgaactcgggactcgacc

SEQ ID NO: 636 - DNA, 20 bp, Artificial Sequence
  protospacer sequence for targeting WNK1
gaacccagtgaaaaatacca

SEQ ID NO: 637 - DNA, 20 bp, Artificial Sequence
  protospacer sequence for targeting ZMYM2
gtaggctgctgttggacaga

SEQ ID NO: 638 - DNA, 20 bp, Artificial Sequence
  protospacer sequence for targeting ZNF10-1
aataagtcttaccacgtgtc

SEQ ID NO: 639 - DNA, 20 bp, Artificial Sequence
  protospacer sequence for targeting ZNF10-2
attcccacaataaccctatg

SEQ ID NO: 640 - RNA, 218 nt, Artificial Sequence
  Canonical Cas12f
cuucacugauaaaguggagaaccgcuucaccaaaagcugucccuuaggggauuagaacuugagugaaggugggcugcuugcaucagccuaaugucgagaagugcuuucuucggaaaguaacccucgaaacaaauucauuuuuccucuccaauucugcacaaguugcagaacccgaauagacgaaugaaggaaugcaacnnnnnnnnnnnnnnnnnnnn

SEQ ID NO: 641 - RNA, 218 nt, Artificial Sequence
  Canonical Cas12f targeting Intergenic22
cuucacugauaaaguggagaaccgcuucaccaaaagcugucccuuaggggauuagaacuugagugaaggugggcugcuugcaucagccuaaugucgagaagugcuuucuucggaaaguaacccucgaaacaaauucauuuuuccucuccaauucugcacaaguugcagaacccgaauagacgaaugaaggaaugcaacagaacacauaccccugggcc

SEQ ID NO: 642 - RNA, 10 nt, Artificial Sequence
  Linker variants for MF sgRNA
uucgaaagaa

SEQ ID NO: 643 - RNA, 12 nt, Artificial Sequence
  Linker variants for MF sgRNA
uucagaaaugaa

SEQ ID NO: 644 - RNA, 14 nt, Artificial Sequence
  Linker variants for MF sgRNA
uucaugaaaaugaa

SEQ ID NO: 645 - RNA, 16 nt, Artificial Sequence
  Linker variants for MF sgRNA
uucauugaaaaaugaa

SEQ ID NO: 646 - RNA, 11 nt, Artificial Sequence
  U-rich tail sequence
uuuruuuruuu

SEQ ID NO: 647 - RNA, 10 nt, Artificial Sequence
  U-rich tail sequence
uuuuruuuuu

SEQ ID NO: 648 - RNA, 11 nt, Artificial Sequence
  U-rich tail sequence
uuuuruuuuuu

SEQ ID NO: 649 - RNA, 129 nt, Artificial Sequence
  MS2/3/4/5
accgcuucacuuagagugaaggugggcugcuugcaucagccuaaugucgagaagugcuuucuucggaaaguaacccucgaaacaaagaaaggaaugcaacagaacacauaccccugggccuuuuauuuu